European Patent Specification EP 3 606 570 B1, published November 27, 2024. Title: COLLAGEN PEPTIDE-BASED MEDICAMENT COMPOSITIONS AND DEVICES AND METHODS OF PRODUCTION AND USE THEREOF. Applicant: SUSTAIN HOLDINGS, LLC. Application PCT/US2018/026180. The sequence listing filed with the application follows.

SEQUENCE LISTING (398 sequences)

SEQ ID NO: 1 - protein, 21 aa, Artificial Sequence
  Description of Artificial Sequence: Synthetic peptide
PPGPPGPPGPPGPPGPPGPPG

SEQ ID NO: 2 - protein, 21 aa, Artificial Sequence
  Description of Artificial Sequence: Synthetic peptide
  MOD_RES (1)..(1): 4S-hydroxyproline
  MOD_RES (4)..(4): 4S-hydroxyproline
  MOD_RES (7)..(7): 4S-hydroxyproline
  MOD_RES (10)..(10): 4S-hydroxyproline
  MOD_RES (13)..(13): 4S-hydroxyproline
  MOD_RES (16)..(16): 4S-hydroxyproline
  MOD_RES (19)..(19): 4S-hydroxyproline
PPGPPGPPGPPGPPGPPGPPG

SEQ ID NO: 3 - protein, 21 aa, Artificial Sequence
  Description of Artificial Sequence: Synthetic peptide
  MOD_RES (2)..(2): 4S-hydroxyproline
  MOD_RES (5)..(5): 4S-hydroxyproline
  MOD_RES (8)..(8): 4S-hydroxyproline
  MOD_RES (11)..(11): 4S-hydroxyproline
  MOD_RES (14)..(14): 4S-hydroxyproline
  MOD_RES (17)..(17): 4S-hydroxyproline
  MOD_RES (20)..(20): 4S-hydroxyproline
PPGPPGPPGPPGPPGPPGPPG

SEQ ID NO: 4 - protein, 21 aa, Artificial Sequence
  Description of Artificial Sequence: Synthetic peptide
  MOD_RES (1)..(1): Fluoroproline
  MOD_RES (4)..(4): Fluoroproline
  MOD_RES (7)..(7): Fluoroproline
  MOD_RES (10)..(10): Fluoroproline
  MOD_RES (13)..(13): Fluoroproline
  MOD_RES (16)..(16): Fluoroproline
  MOD_RES (19)..(19): Fluoroproline
PPGPPGPPGPPGPPGPPGPPG

SEQ ID NO: 5 - protein, 21 aa, Artificial Sequence
  Description of Artificial Sequence: Synthetic peptide
  MOD_RES (2)..(2): Fluoroproline
  MOD_RES (5)..(5): Fluoroproline
  MOD_RES (8)..(8): Fluoroproline
  MOD_RES (11)..(11): Fluoroproline
  MOD_RES (14)..(14): Fluoroproline
  MOD_RES (17)..(17): Fluoroproline
  MOD_RES (20)..(20): Fluoroproline
PPGPPGPPGPPGPPGPPGPPG

SEQ ID NO: 6 - protein, 21 aa, Artificial Sequence
  Description of Artificial Sequence: Synthetic peptide
  MOD_RES (1)..(1): Fluoroproline
  MOD_RES (2)..(2): Hydroxyproline
  MOD_RES (4)..(4): Fluoroproline
  MOD_RES (5)..(5): Hydroxyproline
  MOD_RES (7)..(7): Fluoroproline
  MOD_RES (8)..(8): Hydroxyproline
  MOD_RES (10)..(10): Fluoroproline
  MOD_RES (11)..(11): Hydroxyproline
  MOD_RES (13)..(13): Fluoroproline
  MOD_RES (14)..(14): Hydroxyproline
  MOD_RES (16)..(16): Fluoroproline
  MOD_RES (17)..(17): Hydroxyproline
  MOD_RES (19)..(19): Fluoroproline
  MOD_RES (20)..(20): Hydroxyproline
PPGPPGPPGPPGPPGPPGPPG

SEQ ID NO: 7 - protein, 21 aa, Artificial Sequence
  Description of Artificial Sequence: Synthetic peptide
  MOD_RES (1)..(1): Chloroproline
  MOD_RES (4)..(4): Chloroproline
  MOD_RES (7)..(7): Chloroproline
  MOD_RES (10)..(10): Chloroproline
  MOD_RES (13)..(13): Chloroproline
  MOD_RES (16)..(16): Chloroproline
  MOD_RES (19)..(19): Chloroproline
PPGPPGPPGPPGPPGPPGPPG

SEQ ID NO: 8 - protein, 21 aa, Artificial Sequence
  Description of Artificial Sequence: Synthetic peptide
  MOD_RES (2)..(2): Chloroproline
  MOD_RES (5)..(5): Chloroproline
  MOD_RES (8)..(8): Chloroproline
  MOD_RES (11)..(11): Chloroproline
  MOD_RES (14)..(14): Chloroproline
  MOD_RES (17)..(17): Chloroproline
  MOD_RES (20)..(20): Chloroproline
PPGPPGPPGPPGPPGPPGPPG

SEQ ID NO: 9 - protein, 21 aa, Artificial Sequence
  Description of Artificial Sequence: Synthetic peptide
  MOD_RES (1)..(1): Chloroproline
  MOD_RES (2)..(2): Hydroxyproline
  MOD_RES (4)..(4): Chloroproline
  MOD_RES (5)..(5): Hydroxyproline
  MOD_RES (7)..(7): Chloroproline
  MOD_RES (8)..(8): Hydroxyproline
  MOD_RES (10)..(10): Chloroproline
  MOD_RES (11)..(11): Hydroxyproline
  MOD_RES (13)..(13): Chloroproline
  MOD_RES (14)..(14): Hydroxyproline
  MOD_RES (16)..(16): Chloroproline
  MOD_RES (17)..(17): Hydroxyproline
  MOD_RES (19)..(19): Chloroproline
  MOD_RES (20)..(20): Hydroxyproline
PPGPPGPPGPPGPPGPPGPPG

SEQ ID NO: 10 - protein, 21 aa, Artificial Sequence
  Description of Artificial Sequence: Synthetic peptide
PPGPPGCPGPPGPPGPPGPPG

SEQ ID NO: 11 - protein, 21 aa, Artificial Sequence
  Description of Artificial Sequence: Synthetic peptide
  MOD_RES (1)..(1): Hydroxyproline
  MOD_RES (4)..(4): Hydroxyproline
  MOD_RES (10)..(10): Hydroxyproline
  MOD_RES (13)..(13): Hydroxyproline
  MOD_RES (16)..(16): Hydroxyproline
  MOD_RES (19)..(19): Hydroxyproline
PPGPPGCPGPPGPPGPPGPPG

SEQ ID NO: 12 - protein, 21 aa, Artificial Sequence
  Description of Artificial Sequence: Synthetic peptide
  MOD_RES (2)..(2): Hydroxyproline
  MOD_RES (5)..(5): Hydroxyproline
  MOD_RES (11)..(11): Hydroxyproline
  MOD_RES (14)..(14): Hydroxyproline
  MOD_RES (17)..(17): Hydroxyproline
  MOD_RES (20)..(20): Hydroxyproline
PPGPPGPCGPPGPPGPPGPPG

SEQ ID NO: 13 - protein, 21 aa, Artificial Sequence
  Description of Artificial Sequence: Synthetic peptide
  MOD_RES (2)..(2): Fluoroproline
  MOD_RES (5)..(5): Fluoroproline
  MOD_RES (11)..(11): Fluoroproline
  MOD_RES (14)..(14): Fluoroproline
  MOD_RES (17)..(17): Fluoroproline
  MOD_RES (20)..(20): Fluoroproline
PPGPPGPCGPPGPPGPPGPPG

SEQ ID NO: 14 - protein, 21 aa, Artificial Sequence
  Description of Artificial Sequence: Synthetic peptide
  MOD_RES (2)..(2): Chloroproline
  MOD_RES (5)..(5): Chloroproline
  MOD_RES (11)..(11): Chloroproline
  MOD_RES (14)..(14): Chloroproline
  MOD_RES (17)..(17): Chloroproline
  MOD_RES (20)..(20): Chloroproline
PPGPPGPCGPPGPPGPPGPPG

SEQ ID NO: 15 - protein, 21 aa, Artificial Sequence
  Description of Artificial Sequence: Synthetic peptide
CPGPPGPPGPPGPPGPPGPPG

SEQ ID NO: 16 - protein, 21 aa, Artificial Sequence
  Description of Artificial Sequence: Synthetic peptide
PCGPPGPPGPPGPPGPPGPPG

SEQ ID NO: 17 - protein, 21 aa, Artificial Sequence
  Description of Artificial Sequence: Synthetic peptide
PPGCPGPPGPPGPPGPPGPPG

SEQ ID NO: 18 - protein, 21 aa, Artificial Sequence
  Description of Artificial Sequence: Synthetic peptide
PPGPCGPPGPPGPPGPPGPPG

SEQ ID NO: 19 - protein, 21 aa, Artificial Sequence
  Description of Artificial Sequence: Synthetic peptide
PPGPPGPCGPPGPPGPPGPPG

SEQ ID NO: 20 - protein, 21 aa, Artificial Sequence
  Description of Artificial Sequence: Synthetic peptide
PPGPPGPPGCPGPPGPPGPPG

SEQ ID NO: 21 - protein, 21 aa, Artificial Sequence
  Description of Artificial Sequence: Synthetic peptide
PPGPPGPPGPCGPPGPPGPPG

SEQ ID NO: 22 - protein, 21 aa, Artificial Sequence
  Description of Artificial Sequence: Synthetic peptide
PPGPPGPPGPPGCPGPPGPPG

SEQ ID NO: 23 - protein, 21 aa, Artificial Sequence
  Description of Artificial Sequence: Synthetic peptide
PPGPPGPPGPPGPCGPPGPPG

SEQ ID NO: 24 - protein, 21 aa, Artificial Sequence
  Description of Artificial Sequence: Synthetic peptide
PPGPPGPPGPPGPPGCPGPPG

SEQ ID NO: 25 - protein, 21 aa, Artificial Sequence
  Description of Artificial Sequence: Synthetic peptide
PPGPPGPPGPPGPPGPCGCPG

SEQ ID NO: 26 - protein, 21 aa, Artificial Sequence
  Description of Artificial Sequence: Synthetic peptide
PPGPPGPPGPPGPPGPPGCPG

SEQ ID NO: 27 - protein, 21 aa, Artificial Sequence
  Description of Artificial Sequence: Synthetic peptide
PPGPPGPPGPPGPPGPPGPCG

SEQ ID NO: 28 - protein, 21 aa, Artificial Sequence
  Description of Artificial Sequence: Synthetic peptide
  MOD_RES (4)..(4): Hydroxyproline
  MOD_RES (7)..(7): Hydroxyproline
  MOD_RES (10)..(10): Hydroxyproline
  MOD_RES (13)..(13): Hydroxyproline
  MOD_RES (16)..(16): Hydroxyproline
  MOD_RES (19)..(19): Hydroxyproline
CPGPPGPPGPPGPPGPPGPPG

SEQ ID NO: 29 - protein, 21 aa, Artificial Sequence
  Description of Artificial Sequence: Synthetic peptide
  MOD_RES (1)..(1): Hydroxyproline
  MOD_RES (4)..(4): Hydroxyproline
  MOD_RES (7)..(7): Hydroxyproline
  MOD_RES (10)..(10): Hydroxyproline
  MOD_RES (13)..(13): Hydroxyproline
  MOD_RES (16)..(16): Hydroxyproline
  MOD_RES (19)..(19): Hydroxyproline
PCGPPGPPGPPGPPGPPGPPG

SEQ ID NO: 30 - protein, 21 aa, Artificial Sequence
  Description of Artificial Sequence: Synthetic peptide
  MOD_RES (1)..(1): Hydroxyproline
  MOD_RES (7)..(7): Hydroxyproline
  MOD_RES (10)..(10): Hydroxyproline
  MOD_RES (13)..(13): Hydroxyproline
  MOD_RES (16)..(16): Hydroxyproline
  MOD_RES (19)..(19): Hydroxyproline
PPGCPGPPGPPGPPGPPGPPG

SEQ ID NO: 31 - protein, 21 aa, Artificial Sequence
  Description of Artificial Sequence: Synthetic peptide
  MOD_RES (1)..(1): Hydroxyproline
  MOD_RES (4)..(4): Hydroxyproline
  MOD_RES (7)..(7): Hydroxyproline
  MOD_RES (10)..(10): Hydroxyproline
  MOD_RES (13)..(13): Hydroxyproline
  MOD_RES (16)..(16): Hydroxyproline
  MOD_RES (19)..(19): Hydroxyproline
PPGPCGPPGPPGPPGPPGPPG

SEQ ID NO: 32 - protein, 21 aa, Artificial Sequence
  Description of Artificial Sequence: Synthetic peptide
  MOD_RES (1)..(1): Hydroxyproline
  MOD_RES (4)..(4): Hydroxyproline
  MOD_RES (7)..(7): Hydroxyproline
  MOD_RES (10)..(10): Hydroxyproline
  MOD_RES (13)..(13): Hydroxyproline
  MOD_RES (16)..(16): Hydroxyproline
  MOD_RES (19)..(19): Hydroxyproline
PPGPPGPCGPPGPPGPPGPPG

SEQ ID NO: 33 - protein, 21 aa, Artificial Sequence
  Description of Artificial Sequence: Synthetic peptide
  MOD_RES (1)..(1): Hydroxyproline
  MOD_RES (4)..(4): Hydroxyproline
  MOD_RES (7)..(7): Hydroxyproline
  MOD_RES (13)..(13): Hydroxyproline
  MOD_RES (16)..(16): Hydroxyproline
  MOD_RES (19)..(19): Hydroxyproline
PPGPPGPPGCPGPPGPPGPPG

SEQ ID NO: 34 - protein, 21 aa, Artificial Sequence
  Description of Artificial Sequence: Synthetic peptide
  MOD_RES (1)..(1): Hydroxyproline
  MOD_RES (4)..(4): Hydroxyproline
  MOD_RES (7)..(7): Hydroxyproline
  MOD_RES (10)..(10): Hydroxyproline
  MOD_RES (13)..(13): Hydroxyproline
  MOD_RES (16)..(16): Hydroxyproline
  MOD_RES (19)..(19): Hydroxyproline
PPGPPGPPGPCGPPGPPGPPG

SEQ ID NO: 35 - protein, 21 aa, Artificial Sequence
  Description of Artificial Sequence: Synthetic peptide
  MOD_RES (1)..(1): Hydroxyproline
  MOD_RES (4)..(4): Hydroxyproline
  MOD_RES (7)..(7): Hydroxyproline
  MOD_RES (10)..(10): Hydroxyproline
  MOD_RES (16)..(16): Hydroxyproline
  MOD_RES (19)..(19): Hydroxyproline
PPGPPGPPGPPGCPGPPGPPG

SEQ ID NO: 36 - protein, 21 aa, Artificial Sequence
  Description of Artificial Sequence: Synthetic peptide
  MOD_RES (1)..(1): Hydroxyproline
  MOD_RES (4)..(4): Hydroxyproline
  MOD_RES (7)..(7): Hydroxyproline
  MOD_RES (10)..(10): Hydroxyproline
  MOD_RES (13)..(13): Hydroxyproline
  MOD_RES (16)..(16): Hydroxyproline
  MOD_RES (19)..(19): Hydroxyproline
PPGPPGPPGPPGPCGPPGPPG

SEQ ID NO: 37 - protein, 21 aa, Artificial Sequence
  Description of Artificial Sequence: Synthetic peptide
  MOD_RES (1)..(1): Hydroxyproline
  MOD_RES (4)..(4): Hydroxyproline
  MOD_RES (7)..(7): Hydroxyproline
  MOD_RES (10)..(10): Hydroxyproline
  MOD_RES (13)..(13): Hydroxyproline
  MOD_RES (19)..(19): Hydroxyproline
PPGPPGPPGPPGPPGCPGPPG

SEQ ID NO: 38 - protein, 21 aa, Artificial Sequence
  Description of Artificial Sequence: Synthetic peptide
  MOD_RES (1)..(1): Hydroxyproline
  MOD_RES (4)..(4): Hydroxyproline
  MOD_RES (7)..(7): Hydroxyproline
  MOD_RES (10)..(10): Hydroxyproline
  MOD_RES (13)..(13): Hydroxyproline
  MOD_RES (16)..(16): Hydroxyproline
  MOD_RES (19)..(19): Hydroxyproline
PPGPPGPPGPPGPPGPCGPPG

SEQ ID NO: 39 - protein, 21 aa, Artificial Sequence
  Description of Artificial Sequence: Synthetic peptide
  MOD_RES (1)..(1): Hydroxyproline
  MOD_RES (4)..(4): Hydroxyproline
  MOD_RES (7)..(7): Hydroxyproline
  MOD_RES (10)..(10): Hydroxyproline
  MOD_RES (13)..(13): Hydroxyproline
  MOD_RES (16)..(16): Hydroxyproline
PPGPPGPPGPPGPPGPPGCPG

SEQ ID NO: 40 - protein, 21 aa, Artificial Sequence
  Description of Artificial Sequence: Synthetic peptide
  MOD_RES (1)..(1): Hydroxyproline
  MOD_RES (4)..(4): Hydroxyproline
  MOD_RES (7)..(7): Hydroxyproline
  MOD_RES (10)..(10): Hydroxyproline
  MOD_RES (13)..(13): Hydroxyproline
  MOD_RES (16)..(16): Hydroxyproline
  MOD_RES (19)..(19): Hydroxyproline
PPGPPGPPGPPGPPGPPGPCG

SEQ ID NO: 41 - protein, 21 aa, Artificial Sequence
  Description of Artificial Sequence: Synthetic peptide
  MOD_RES (2)..(2): Hydroxyproline
  MOD_RES (5)..(5): Hydroxyproline
  MOD_RES (8)..(8): Hydroxyproline
  MOD_RES (11)..(11): Hydroxyproline
  MOD_RES (14)..(14): Hydroxyproline
  MOD_RES (17)..(17): Hydroxyproline
  MOD_RES (20)..(20): Hydroxyproline
CPGPPGPPGPPGPPGPPGPPG

SEQ ID NO: 42 - protein, 21 aa, Artificial Sequence
  Description of Artificial Sequence: Synthetic peptide
  MOD_RES (5)..(5): Hydroxyproline
  MOD_RES (8)..(8): Hydroxyproline
  MOD_RES (11)..(11): Hydroxyproline
  MOD_RES (14)..(14): Hydroxyproline
  MOD_RES (17)..(17): Hydroxyproline
  MOD_RES (20)..(20): Hydroxyproline
PCGPPGPPGPPGPPGPPGPPG

SEQ ID NO: 43 - protein, 21 aa, Artificial Sequence
  Description of Artificial Sequence: Synthetic peptide
  MOD_RES (2)..(2): Hydroxyproline
  MOD_RES (5)..(5): Hydroxyproline
  MOD_RES (8)..(8): Hydroxyproline
  MOD_RES (11)..(11): Hydroxyproline
  MOD_RES (14)..(14): Hydroxyproline
  MOD_RES (17)..(17): Hydroxyproline
  MOD_RES (20)..(20): Hydroxyproline
PPGCPGPPGPPGPPGPPGPPG

SEQ ID NO: 44 - protein, 21 aa, Artificial Sequence
  Description of Artificial Sequence: Synthetic peptide
  MOD_RES (2)..(2): Hydroxyproline
  MOD_RES (8)..(8): Hydroxyproline
  MOD_RES (11)..(11): Hydroxyproline
  MOD_RES (14)..(14): Hydroxyproline
  MOD_RES (17)..(17): Hydroxyproline
  MOD_RES (20)..(20): Hydroxyproline
PPGPCGPPGPPGPPGPPGPPG

SEQ ID NO: 45 - protein, 21 aa, Artificial Sequence
  Description of Artificial Sequence: Synthetic peptide
  MOD_RES (2)..(2): Hydroxyproline
  MOD_RES (5)..(5): Hydroxyproline
  MOD_RES (8)..(8): Hydroxyproline
  MOD_RES (11)..(11): Hydroxyproline
  MOD_RES (14)..(14): Hydroxyproline
  MOD_RES (17)..(17): Hydroxyproline
  MOD_RES (20)..(20): Hydroxyproline
PPGPPGCPGPPGPPGPPGPPG

SEQ ID NO: 46 - protein, 21 aa, Artificial Sequence
  Description of Artificial Sequence: Synthetic peptide
  MOD_RES (2)..(2): Hydroxyproline
  MOD_RES (5)..(5): Hydroxyproline
  MOD_RES (8)..(8): Hydroxyproline
  MOD_RES (11)..(11): Hydroxyproline
  MOD_RES (14)..(14): Hydroxyproline
  MOD_RES (17)..(17): Hydroxyproline
  MOD_RES (20)..(20): Hydroxyproline
PPGPPGPPGCPGPPGPPGPPG

SEQ ID NO: 47 - protein, 21 aa, Artificial Sequence
  Description of Artificial Sequence: Synthetic peptide
  MOD_RES (2)..(2): Hydroxyproline
  MOD_RES (5)..(5): Hydroxyproline
  MOD_RES (8)..(8): Hydroxyproline
  MOD_RES (14)..(14): Hydroxyproline
  MOD_RES (17)..(17): Hydroxyproline
  MOD_RES (20)..(20): Hydroxyproline
PPGPPGPPGPCGPPGPPGPPG

SEQ ID NO: 48 - protein, 21 aa, Artificial Sequence
  Description of Artificial Sequence: Synthetic peptide
  MOD_RES (2)..(2): Hydroxyproline
  MOD_RES (5)..(5): Hydroxyproline
  MOD_RES (8)..(8): Hydroxyproline
  MOD_RES (11)..(11): Hydroxyproline
  MOD_RES (14)..(14): Hydroxyproline
  MOD_RES (17)..(17): Hydroxyproline
  MOD_RES (20)..(20): Hydroxyproline
PPGPPGPPGPPGCPGPPGPPG

SEQ ID NO: 49 - protein, 21 aa, Artificial Sequence
  Description of Artificial Sequence: Synthetic peptide
  MOD_RES (2)..(2): Hydroxyproline
  MOD_RES (5)..(5): Hydroxyproline
  MOD_RES (8)..(8): Hydroxyproline
  MOD_RES (11)..(11): Hydroxyproline
  MOD_RES (17)..(17): Hydroxyproline
  MOD_RES (20)..(20): Hydroxyproline
PPGPPGPPGPPGPCGPPGPPG

SEQ ID NO: 50 - protein, 21 aa, Artificial Sequence
  Description of Artificial Sequence: Synthetic peptide
  MOD_RES (2)..(2): Hydroxyproline
  MOD_RES (5)..(5): Hydroxyproline
  MOD_RES (8)..(8): Hydroxyproline
  MOD_RES (11)..(11): Hydroxyproline
  MOD_RES (14)..(14): Hydroxyproline
  MOD_RES (17)..(17): Hydroxyproline
  MOD_RES (20)..(20): Hydroxyproline
PPGPPGPPGPPGPPGCPGPPG

SEQ ID NO: 51 - protein, 21 aa, Artificial Sequence
  Description of Artificial Sequence: Synthetic peptide
  MOD_RES (2)..(2): Hydroxyproline
  MOD_RES (5)..(5): Hydroxyproline
  MOD_RES (8)..(8): Hydroxyproline
  MOD_RES (11)..(11): Hydroxyproline
  MOD_RES (14)..(14): Hydroxyproline
  MOD_RES (20)..(20): Hydroxyproline
PPGPPGPPGPPGPPGPCGPPG

SEQ ID NO: 52 - protein, 21 aa, Artificial Sequence
  Description of Artificial Sequence: Synthetic peptide
  MOD_RES (2)..(2): Hydroxyproline
  MOD_RES (5)..(5): Hydroxyproline
  MOD_RES (8)..(8): Hydroxyproline
  MOD_RES (11)..(11): Hydroxyproline
  MOD_RES (14)..(14): Hydroxyproline
  MOD_RES (17)..(17): Hydroxyproline
  MOD_RES (20)..(20): Hydroxyproline
PPGPPGPPGPPGPPGPPGCPG

SEQ ID NO: 53 - protein, 21 aa, Artificial Sequence
  Description of Artificial Sequence: Synthetic peptide
  MOD_RES (2)..(2): Hydroxyproline
  MOD_RES (5)..(5): Hydroxyproline
  MOD_RES (8)..(8): Hydroxyproline
  MOD_RES (11)..(11): Hydroxyproline
  MOD_RES (14)..(14): Hydroxyproline
  MOD_RES (17)..(17): Hydroxyproline
PPGPPGPPGPPGPPGPPGPCG

SEQ ID NO: 54 - protein, 21 aa, Artificial Sequence
  Description of Artificial Sequence: Synthetic peptide
  MOD_RES (2)..(2): Fluoroproline
  MOD_RES (5)..(5): Fluoroproline
  MOD_RES (8)..(8): Fluoroproline
  MOD_RES (11)..(11): Fluoroproline
  MOD_RES (14)..(14): Fluoroproline
  MOD_RES (17)..(17): Fluoroproline
  MOD_RES (20)..(20): Fluoroproline
CPGPPGPPGPPGPPGPPGPPG

SEQ ID NO: 55 - protein, 21 aa, Artificial Sequence
  Description of Artificial Sequence: Synthetic peptide
  MOD_RES (5)..(5): Fluoroproline
  MOD_RES (8)..(8): Fluoroproline
  MOD_RES (11)..(11): Fluoroproline
  MOD_RES (14)..(14): Fluoroproline
  MOD_RES (17)..(17): Fluoroproline
  MOD_RES (20)..(20): Fluoroproline
PCGPPGPPGPPGPPGPPGPPG

SEQ ID NO: 56 - protein, 21 aa, Artificial Sequence
  Description of Artificial Sequence: Synthetic peptide
  MOD_RES (2)..(2): Fluoroproline
  MOD_RES (5)..(5): Fluoroproline
  MOD_RES (8)..(8): Fluoroproline
  MOD_RES (11)..(11): Fluoroproline
  MOD_RES (14)..(14): Fluoroproline
  MOD_RES (17)..(17): Fluoroproline
  MOD_RES (20)..(20): Fluoroproline
PPGCPGPPGPPGPPGPPGPPG

SEQ ID NO: 57 - protein, 21 aa, Artificial Sequence
  Description of Artificial Sequence: Synthetic peptide
  MOD_RES (2)..(2): Fluoroproline
  MOD_RES (8)..(8): Fluoroproline
  MOD_RES (11)..(11): Fluoroproline
  MOD_RES (14)..(14): Fluoroproline
  MOD_RES (17)..(17): Fluoroproline
  MOD_RES (20)..(20): Fluoroproline
PPGPCGPPGPPGPPGPPGPPG

SEQ ID NO: 58 - protein, 21 aa, Artificial Sequence
  Description of Artificial Sequence: Synthetic peptide
  MOD_RES (2)..(2): Fluoroproline
  MOD_RES (5)..(5): Fluoroproline
  MOD_RES (8)..(8): Fluoroproline
  MOD_RES (11)..(11): Fluoroproline
  MOD_RES (14)..(14): Fluoroproline
  MOD_RES (17)..(17): Fluoroproline
  MOD_RES (20)..(20): Fluoroproline
PPGPPGCPGPPGPPGPPGPPG

SEQ ID NO: 59 - protein, 21 aa, Artificial Sequence
  Description of Artificial Sequence: Synthetic peptide
  MOD_RES (2)..(2): Fluoroproline
  MOD_RES (5)..(5): Fluoroproline
  MOD_RES (8)..(8): Fluoroproline
  MOD_RES (11)..(11): Fluoroproline
  MOD_RES (14)..(14): Fluoroproline
  MOD_RES (17)..(17): Fluoroproline
  MOD_RES (20)..(20): Fluoroproline
PPGPPGPPGCPGPPGPPGPPG

SEQ ID NO: 60 - protein, 21 aa, Artificial Sequence
  Description of Artificial Sequence: Synthetic peptide
  MOD_RES (2)..(2): Fluoroproline
  MOD_RES (5)..(5): Fluoroproline
  MOD_RES (8)..(8): Fluoroproline
  MOD_RES (14)..(14): Fluoroproline
  MOD_RES (17)..(17): Fluoroproline
  MOD_RES (20)..(20): Fluoroproline
PPGPPGPPGPCGPPGPPGPPG

SEQ ID NO: 61 - protein, 21 aa, Artificial Sequence
  Description of Artificial Sequence: Synthetic peptide
  MOD_RES (2)..(2): Fluoroproline
  MOD_RES (5)..(5): Fluoroproline
  MOD_RES (8)..(8): Fluoroproline
  MOD_RES (11)..(11): Fluoroproline
  MOD_RES (14)..(14): Fluoroproline
  MOD_RES (17)..(17): Fluoroproline
  MOD_RES (20)..(20): Fluoroproline
PPGPPGPPGPPGCPGPPGPPG

SEQ ID NO: 62 - protein, 21 aa, Artificial Sequence
  Description of Artificial Sequence: Synthetic peptide
  MOD_RES (2)..(2): Fluoroproline
  MOD_RES (5)..(5): Fluoroproline
  MOD_RES (8)..(8): Fluoroproline
  MOD_RES (11)..(11): Fluoroproline
  MOD_RES (17)..(17): Fluoroproline
  MOD_RES (20)..(20): Fluoroproline
PPGPPGPPGPPGPCGPPGPPG

SEQ ID NO: 63 - protein, 21 aa, Artificial Sequence
  Description of Artificial Sequence: Synthetic peptide
  MOD_RES (2)..(2): Fluoroproline
  MOD_RES (5)..(5): Fluoroproline
  MOD_RES (8)..(8): Fluoroproline
  MOD_RES (11)..(11): Fluoroproline
  MOD_RES (14)..(14): Fluoroproline
  MOD_RES (17)..(17): Fluoroproline
  MOD_RES (20)..(20): Fluoroproline
PPGPPGPPGPPGPPGCPGPPG

SEQ ID NO: 64 - protein, 21 aa, Artificial Sequence
  Description of Artificial Sequence: Synthetic peptide
  MOD_RES (2)..(2): Fluoroproline
  MOD_RES (5)..(5): Fluoroproline
  MOD_RES (8)..(8): Fluoroproline
  MOD_RES (11)..(11): Fluoroproline
  MOD_RES (14)..(14): Fluoroproline
  MOD_RES (20)..(20): Fluoroproline
PPGPPGPPGPPGPPGPCGPPG

SEQ ID NO: 65 - protein, 21 aa, Artificial Sequence
  Description of Artificial Sequence: Synthetic peptide
  MOD_RES (2)..(2): Fluoroproline
  MOD_RES (5)..(5): Fluoroproline
  MOD_RES (8)..(8): Fluoroproline
  MOD_RES (11)..(11): Fluoroproline
  MOD_RES (14)..(14): Fluoroproline
  MOD_RES (17)..(17): Fluoroproline
  MOD_RES (20)..(20): Fluoroproline
PPGPPGPPGPPGPPGPPGCPG

SEQ ID NO: 66 - protein, 21 aa, Artificial Sequence
  Description of Artificial Sequence: Synthetic peptide
  MOD_RES (2)..(2): Fluoroproline
  MOD_RES (5)..(5): Fluoroproline
  MOD_RES (8)..(8): Fluoroproline
  MOD_RES (11)..(11): Fluoroproline
  MOD_RES (14)..(14): Fluoroproline
  MOD_RES (17)..(17): Fluoroproline
PPGPPGPPGPPGPPGPPGPCG

SEQ ID NO: 67 - protein, 21 aa, Artificial Sequence
  Description of Artificial Sequence: Synthetic peptide
  MOD_RES (2)..(2): Fluoroproline
  MOD_RES (5)..(5): Fluoroproline
  MOD_RES (8)..(8): Fluoroproline
  MOD_RES (11)..(11): Fluoroproline
  MOD_RES (14)..(14): Fluoroproline
  MOD_RES (17)..(17): Fluoroproline
  MOD_RES (20)..(20): Fluoroproline
CPGPPGPPGPPGPPGPPGPPG

SEQ ID NO: 68 - protein, 21 aa, Artificial Sequence
  Description of Artificial Sequence: Synthetic peptide
  MOD_RES (5)..(5): Fluoroproline
  MOD_RES (8)..(8): Fluoroproline
  MOD_RES (11)..(11): Fluoroproline
  MOD_RES (14)..(14): Fluoroproline
  MOD_RES (17)..(17): Fluoroproline
  MOD_RES (20)..(20): Fluoroproline
PCGPPGPPGPPGPPGPPGPPG

SEQ ID NO: 69 - protein, 21 aa, Artificial Sequence
  Description of Artificial Sequence: Synthetic peptide
  MOD_RES (2)..(2): Fluoroproline
  MOD_RES (5)..(5): Fluoroproline
  MOD_RES (8)..(8): Fluoroproline
  MOD_RES (11)..(11): Fluoroproline
  MOD_RES (14)..(14): Fluoroproline
  MOD_RES (17)..(17): Fluoroproline
  MOD_RES (20)..(20): Fluoroproline
PPGCPGPPGPPGPPGPPGPPG

SEQ ID NO: 70 - protein, 21 aa, Artificial Sequence
  Description of Artificial Sequence: Synthetic peptide
  MOD_RES (2)..(2): Fluoroproline
  MOD_RES (8)..(8): Fluoroproline
  MOD_RES (11)..(11): Fluoroproline
  MOD_RES (14)..(14): Fluoroproline
  MOD_RES (17)..(17): Fluoroproline
  MOD_RES (20)..(20): Fluoroproline
PPGPCGPPGPPGPPGPPGPPG

SEQ ID NO: 71 - protein, 21 aa, Artificial Sequence
  Description of Artificial Sequence: Synthetic peptide
  MOD_RES (2)..(2): Fluoroproline
  MOD_RES (5)..(5): Fluoroproline
  MOD_RES (8)..(8): Fluoroproline
  MOD_RES (11)..(11): Fluoroproline
  MOD_RES (14)..(14): Fluoroproline
  MOD_RES (17)..(17): Fluoroproline
  MOD_RES (20)..(20): Fluoroproline
PPGPPGCPGPPGPPGPPGPPG

SEQ ID NO: 72 - protein, 21 aa, Artificial Sequence
  Description of Artificial Sequence: Synthetic peptide
  MOD_RES (2)..(2): Fluoroproline
  MOD_RES (5)..(5): Fluoroproline
  MOD_RES (11)..(11): Fluoroproline
  MOD_RES (14)..(14): Fluoroproline
  MOD_RES (17)..(17): Fluoroproline
  MOD_RES (20)..(20): Fluoroproline
PPGPPGPCGPPGPPGPPGPPG

SEQ ID NO: 73 - protein, 21 aa, Artificial Sequence
  Description of Artificial Sequence: Synthetic peptide
  MOD_RES (2)..(2): Fluoroproline
  MOD_RES (5)..(5): Fluoroproline
  MOD_RES (8)..(8): Fluoroproline
  MOD_RES (11)..(11): Fluoroproline
  MOD_RES (14)..(14): Fluoroproline
  MOD_RES (17)..(17): Fluoroproline
  MOD_RES (20)..(20): Fluoroproline
PPGPPGPPGCPGPPGPPGPPG

SEQ ID NO: 74 - protein, 21 aa, Artificial Sequence
  Description of Artificial Sequence: Synthetic peptide
  MOD_RES (2)..(2): Fluoroproline
  MOD_RES (5)..(5): Fluoroproline
  MOD_RES (8)..(8): Fluoroproline
  MOD_RES (14)..(14): Fluoroproline
  MOD_RES (17)..(17): Fluoroproline
  MOD_RES (20)..(20): Fluoroproline
PPGPPGPPGPCGPPGPPGPPG

SEQ ID NO: 75 - protein, 21 aa, Artificial Sequence
  Description of Artificial Sequence: Synthetic peptide
  MOD_RES (2)..(2): Fluoroproline
  MOD_RES (5)..(5): Fluoroproline
  MOD_RES (8)..(8): Fluoroproline
  MOD_RES (11)..(11): Fluoroproline
  MOD_RES (14)..(14): Fluoroproline
  MOD_RES (17)..(17): Fluoroproline
  MOD_RES (20)..(20): Fluoroproline
PPGPPGPPGPPGCPGPPGPPG

SEQ ID NO: 76 - protein, 21 aa, Artificial Sequence
  Description of Artificial Sequence: Synthetic peptide
  MOD_RES (2)..(2): Fluoroproline
  MOD_RES (5)..(5): Fluoroproline
  MOD_RES (8)..(8): Fluoroproline
  MOD_RES (11)..(11): Fluoroproline
  MOD_RES (17)..(17): Fluoroproline
  MOD_RES (20)..(20): Fluoroproline
PPGPPGPPGPPGPCGPPGPPG

SEQ ID NO: 77 - protein, 21 aa, Artificial Sequence
  Description of Artificial Sequence: Synthetic peptide
  MOD_RES (2)..(2): Fluoroproline
  MOD_RES (5)..(5): Fluoroproline
  MOD_RES (8)..(8): Fluoroproline
  MOD_RES (11)..(11): Fluoroproline
  MOD_RES (14)..(14): Fluoroproline
  MOD_RES (17)..(17): Fluoroproline
  MOD_RES (20)..(20): Fluoroproline
PPGPPGPPGPPGPPGCPGPPG

SEQ ID NO: 78 - protein, 21 aa, Artificial Sequence
  Description of Artificial Sequence: Synthetic peptide
  MOD_RES (2)..(2): Fluoroproline
  MOD_RES (5)..(5): Fluoroproline
  MOD_RES (8)..(8): Fluoroproline
  MOD_RES (11)..(11): Fluoroproline
  MOD_RES (14)..(14): Fluoroproline
  MOD_RES (20)..(20): Fluoroproline
PPGPPGPPGPPGPPGPCGPPG

SEQ ID NO: 79 - protein, 21 aa, Artificial Sequence
  Description of Artificial Sequence: Synthetic peptide
  MOD_RES (2)..(2): Fluoroproline
  MOD_RES (5)..(5): Fluoroproline
  MOD_RES (8)..(8): Fluoroproline
  MOD_RES (11)..(11): Fluoroproline
  MOD_RES (14)..(14): Fluoroproline
  MOD_RES (17)..(17): Fluoroproline
  MOD_RES (20)..(20): Fluoroproline
PPGPPGPPGPPGPPGPPGCPG

SEQ ID NO: 80 - protein, 21 aa, Artificial Sequence
  Description of Artificial Sequence: Synthetic peptide
  MOD_RES (2)..(2): Fluoroproline
  MOD_RES (5)..(5): Fluoroproline
  MOD_RES (8)..(8): Fluoroproline
  MOD_RES (11)..(11): Fluoroproline
  MOD_RES (14)..(14): Fluoroproline
  MOD_RES (17)..(17): Fluoroproline
PPGPPGPPGPPGPPGPPGPCG

SEQ ID NO: 81 - protein, 21 aa, Artificial Sequence
  Description of Artificial Sequence: Synthetic peptide
  MOD_RES (2)..(2): Hydroxyproline
  MOD_RES (4)..(4): Fluoroproline
  MOD_RES (5)..(5): Hydroxyproline
  MOD_RES (7)..(7): Fluoroproline
  MOD_RES (8)..(8): Hydroxyproline
  MOD_RES (10)..(10): Fluoroproline
  MOD_RES (11)..(11): Hydroxyproline
  MOD_RES (13)..(13): Fluoroproline
  MOD_RES (14)..(14): Hydroxyproline
  MOD_RES (16)..(16): Fluoroproline
  MOD_RES (17)..(17): Hydroxyproline
  MOD_RES (19)..(19): Fluoroproline
  MOD_RES (20)..(20): Hydroxyproline
CPGPPGPPGPPGPPGPPGPPG

SEQ ID NO: 82 - protein, 21 aa, Artificial Sequence
  Description of Artificial Sequence: Synthetic peptide
  MOD_RES (1)..(1): Fluoroproline
  MOD_RES (4)..(4): Fluoroproline
  MOD_RES (5)..(5): Hydroxyproline
  MOD_RES (7)..(7): Fluoroproline
  MOD_RES (8)..(8): Hydroxyproline
  MOD_RES (10)..(10): Fluoroproline
  MOD_RES (11)..(11): Hydroxyproline
  MOD_RES (13)..(13): Fluoroproline
  MOD_RES (14)..(14): Hydroxyproline
  MOD_RES (16)..(16): Fluoroproline
  MOD_RES (17)..(17): Hydroxyproline
  MOD_RES (19)..(19): Fluoroproline
  MOD_RES (20)..(20): Hydroxyproline
PCGPPGPPGPPGPPGPPGPPG

SEQ ID NO: 83 - protein, 21 aa, Artificial Sequence
  Description of Artificial Sequence: Synthetic peptide
  MOD_RES (1)..(1): Fluoroproline
  MOD_RES (2)..(2): Hydroxyproline
  MOD_RES (5)..(5): Hydroxyproline
  MOD_RES (7)..(7): Fluoroproline
  MOD_RES (8)..(8): Hydroxyproline
  MOD_RES (10)..(10): Fluoroproline
  MOD_RES (11)..(11): Hydroxyproline
  MOD_RES (13)..(13): Fluoroproline
  MOD_RES (14)..(14): Hydroxyproline
  MOD_RES (16)..(16): Fluoroproline
  MOD_RES (17)..(17): Hydroxyproline
  MOD_RES (19)..(19): Fluoroproline
  MOD_RES (20)..(20): Hydroxyproline
PPGCPGPPGPPGPPGPPGPPG

SEQ ID NO: 84 - protein, 21 aa, Artificial Sequence
  Description of Artificial Sequence: Synthetic peptide
  MOD_RES (1)..(1): Fluoroproline
  MOD_RES (2)..(2): Hydroxyproline
  MOD_RES (4)..(4): Fluoroproline
  MOD_RES (7)..(7): Fluoroproline
  MOD_RES (8)..(8): Hydroxyproline
  MOD_RES (10)..(10): Fluoroproline
  MOD_RES (11)..(11): Hydroxyproline
  MOD_RES (13)..(13): Fluoroproline
  MOD_RES (14)..(14): Hydroxyproline
  MOD_RES (16)..(16): Fluoroproline
  MOD_RES (17)..(17): Hydroxyproline
  MOD_RES (19)..(19): Fluoroproline
  MOD_RES (20)..(20): Hydroxyproline
PPGPCGPPGPPGPPGPPGPPG

SEQ ID NO: 85 - protein, 21 aa, Artificial Sequence
  Description of Artificial Sequence: Synthetic peptide
  MOD_RES (1)..(1): Fluoroproline
  MOD_RES (2)..(2): Hydroxyproline
  MOD_RES (4)..(4): Fluoroproline
  MOD_RES (5)..(5): Hydroxyproline
  MOD_RES (8)..(8): Hydroxyproline
  MOD_RES (10)..(10): Fluoroproline
  MOD_RES (11)..(11): Hydroxyproline
  MOD_RES (13)..(13): Fluoroproline
  MOD_RES (14)..(14): Hydroxyproline
  MOD_RES (16)..(16): Fluoroproline
  MOD_RES (17)..(17): Hydroxyproline
  MOD_RES (19)..(19): Fluoroproline
  MOD_RES (20)..(20): Hydroxyproline
PPGPPGCPGPPGPPGPPGPPG

SEQ ID NO: 86 - protein, 21 aa, Artificial Sequence
  Description of Artificial Sequence: Synthetic peptide
  MOD_RES (1)..(1): Fluoroproline
  MOD_RES (2)..(2): Hydroxyproline
  MOD_RES (4)..(4): Fluoroproline
  MOD_RES (5)..(5): Hydroxyproline
  MOD_RES (7)..(7): Fluoroproline
  MOD_RES (10)..(10): Fluoroproline
  MOD_RES (11)..(11): Hydroxyproline
  MOD_RES (13)..(13): Fluoroproline
  MOD_RES (14)..(14): Hydroxyproline
  MOD_RES (16)..(16): Fluoroproline
  MOD_RES (17)..(17): Hydroxyproline
  MOD_RES (19)..(19): Fluoroproline
  MOD_RES (20)..(20): Hydroxyproline
PPGPPGPCGPPGPPGPPGPPG

SEQ ID NO: 87 - protein, 21 aa, Artificial Sequence
  Description of Artificial Sequence: Synthetic peptide
  MOD_RES (1)..(1): Fluoroproline
  MOD_RES (2)..(2): Hydroxyproline
  MOD_RES (4)..(4): Fluoroproline
  MOD_RES (5)..(5): Hydroxyproline
  MOD_RES (7)..(7): Fluoroproline
  MOD_RES (8)..(8): Hydroxyproline
  MOD_RES (11)..(11): Hydroxyproline
  MOD_RES (13)..(13): Fluoroproline
  MOD_RES (14)..(14): Hydroxyproline
  MOD_RES (16)..(16): Fluoroproline
  MOD_RES (17)..(17): Hydroxyproline
  MOD_RES (19)..(19): Fluoroproline
  MOD_RES (20)..(20): Hydroxyproline
PPGPPGPPGCPGPPGPPGPPG

SEQ ID NO: 88 - protein, 21 aa, Artificial Sequence
  Description of Artificial Sequence: Synthetic peptide
  MOD_RES (1)..(1): Fluoroproline
  MOD_RES (2)..(2): Hydroxyproline
  MOD_RES (4)..(4): Fluoroproline
  MOD_RES (5)..(5): Hydroxyproline
  MOD_RES (7)..(7): Fluoroproline
  MOD_RES (8)..(8): Hydroxyproline
  MOD_RES (10)..(10): Fluoroproline
  MOD_RES (13)..(13): Fluoroproline
  MOD_RES (14)..(14): Hydroxyproline
  MOD_RES (16)..(16): Fluoroproline
  MOD_RES (17)..(17): Hydroxyproline
  MOD_RES (19)..(19): Fluoroproline
  MOD_RES (20)..(20): Hydroxyproline
PPGPPGPPGPCGPPGPPGPPG

SEQ ID NO: 89 - protein, 21 aa, Artificial Sequence
  Description of Artificial Sequence: Synthetic peptide
  MOD_RES (1)..(1): Fluoroproline
  MOD_RES (2)..(2): Hydroxyproline
  MOD_RES (4)..(4): Fluoroproline
  MOD_RES (5)..(5): Hydroxyproline
  MOD_RES (7)..(7): Fluoroproline
  MOD_RES (8)..(8): Hydroxyproline
  MOD_RES (10)..(10): Fluoroproline
  MOD_RES (11)..(11): Hydroxyproline
  MOD_RES (14)..(14): Hydroxyproline
  MOD_RES (16)..(16): Fluoroproline
  MOD_RES (17)..(17): Hydroxyproline
  MOD_RES (19)..(19): Fluoroproline
  MOD_RES (20)..(20): Hydroxyproline
PPGPPGPPGPPGCPGPPGPPG

SEQ ID NO: 90 - protein, 21 aa, Artificial Sequence
  Description of Artificial Sequence: Synthetic peptide
  MOD_RES (1)..(1): Fluoroproline
  MOD_RES (2)..(2): Hydroxyproline
  MOD_RES (4)..(4): Fluoroproline
  MOD_RES (5)..(5): Hydroxyproline
  MOD_RES (7)..(7): Fluoroproline
  MOD_RES (8)..(8): Hydroxyproline
  MOD_RES (10)..(10): Fluoroproline
  MOD_RES (11)..(11): Hydroxyproline
  MOD_RES (13)..(13): Fluoroproline
  MOD_RES (16)..(16): Fluoroproline
  MOD_RES (17)..(17): Hydroxyproline
  MOD_RES (19)..(19): Fluoroproline
  MOD_RES (20)..(20): Hydroxyproline
PPGPPGPPGPPGPCGPPGPPG

SEQ ID NO: 91 - protein, 21 aa, Artificial Sequence
  Description of Artificial Sequence: Synthetic peptide
  MOD_RES (1)..(1): Fluoroproline
  MOD_RES (2)..(2): Hydroxyproline
  MOD_RES (4)..(4): Fluoroproline
  MOD_RES (5)..(5): Hydroxyproline
  MOD_RES (7)..(7): Fluoroproline
  MOD_RES (8)..(8): Hydroxyproline
  MOD_RES (10)..(10): Fluoroproline
  MOD_RES (11)..(11): Hydroxyproline
  MOD_RES (13)..(13): Fluoroproline
  MOD_RES (14)..(14): Hydroxyproline
  MOD_RES (17)..(17): Hydroxyproline
  MOD_RES (19)..(19): Fluoroproline
  MOD_RES (20)..(20): Hydroxyproline
PPGPPGPPGPPGPPGCPGPPG

SEQ ID NO: 92 - protein, 21 aa, Artificial Sequence
  Description of Artificial Sequence: Synthetic peptide
  MOD_RES (1)..(1): Fluoroproline
  MOD_RES (2)..(2): Hydroxyproline
  MOD_RES (4)..(4): Fluoroproline
  MOD_RES (5)..(5): Hydroxyproline
  MOD_RES (7)..(7): Fluoroproline
  MOD_RES (8)..(8): Hydroxyproline
  MOD_RES (10)..(10): Fluoroproline
  MOD_RES (11)..(11): Hydroxyproline
  MOD_RES (13)..(13): Fluoroproline
  MOD_RES (14)..(14): Hydroxyproline
  MOD_RES (16)..(16): Fluoroproline
  MOD_RES (19)..(19): Fluoroproline
  MOD_RES (20)..(20): Hydroxyproline
PPGPPGPPGPPGPPGPCGPPG

SEQ ID NO: 93 - protein, 21 aa, Artificial Sequence
  Description of Artificial Sequence: Synthetic peptide
  MOD_RES (1)..(1): Fluoroproline
  MOD_RES (2)..(2): Hydroxyproline
  MOD_RES (4)..(4): Fluoroproline
  MOD_RES (5)..(5): Hydroxyproline
  MOD_RES (7)..(7): Fluoroproline
  MOD_RES (8)..(8): Hydroxyproline
  MOD_RES (10)..(10): Fluoroproline
  MOD_RES (11)..(11): Hydroxyproline
  MOD_RES (13)..(13): Fluoroproline
  MOD_RES (14)..(14): Hydroxyproline
  MOD_RES (16)..(16): Fluoroproline
  MOD_RES (17)..(17): Hydroxyproline
  MOD_RES (20)..(20): Hydroxyproline
PPGPPGPPGPPGPPGPPGCPG

SEQ ID NO: 94 - protein, 21 aa, Artificial Sequence
  Description of Artificial Sequence: Synthetic peptide
  MOD_RES (1)..(1): Fluoroproline
  MOD_RES (2)..(2): Hydroxyproline
  MOD_RES (4)..(4): Fluoroproline
  MOD_RES (5)..(5): Hydroxyproline
  MOD_RES (7)..(7): Fluoroproline
  MOD_RES (8)..(8): Hydroxyproline
  MOD_RES (10)..(10): Fluoroproline
  MOD_RES (11)..(11): Hydroxyproline
  MOD_RES (13)..(13): Fluoroproline
  MOD_RES (14)..(14): Hydroxyproline
  MOD_RES (16)..(16): Fluoroproline
  MOD_RES (17)..(17): Hydroxyproline
  MOD_RES (19)..(19): Fluoroproline
PPGPPGPPGPPGPPGPPGPCG

SEQ ID NO: 95 - protein, 21 aa, Artificial Sequence
  Description of Artificial Sequence: Synthetic peptide
  MOD_RES (2)..(2): Chloroproline
  MOD_RES (5)..(5): Chloroproline
  MOD_RES (8)..(8): Chloroproline
  MOD_RES (11)..(11): Chloroproline
  MOD_RES (14)..(14): Chloroproline
  MOD_RES (17)..(17): Chloroproline
  MOD_RES (20)..(20): Chloroproline
CPGPPGPPGPPGPPGPPGPPG

SEQ ID NO: 96 - protein, 21 aa, Artificial Sequence
  Description of Artificial Sequence: Synthetic peptide
  MOD_RES (5)..(5): Chloroproline
  MOD_RES (8)..(8): Chloroproline
  MOD_RES (11)..(11): Chloroproline
  MOD_RES (14)..(14): Chloroproline
  MOD_RES (17)..(17): Chloroproline
  MOD_RES (20)..(20): Chloroproline
PCGPPGPPGPPGPPGPPGPPG

SEQ ID NO: 97 - protein, 21 aa, Artificial Sequence
  Description of Artificial Sequence: Synthetic peptide
  MOD_RES (2)..(2): Chloroproline
  MOD_RES (5)..(5): Chloroproline
  MOD_RES (8)..(8): Chloroproline
  MOD_RES (11)..(11): Chloroproline
  MOD_RES (14)..(14): Chloroproline
  MOD_RES (17)..(17): Chloroproline
  MOD_RES (20)..(20): Chloroproline
PPGCPGPPGPPGPPGPPGPPG

SEQ ID NO: 98 - protein, 21 aa, Artificial Sequence
  Description of Artificial Sequence: Synthetic peptide
  MOD_RES (2)..(2): Chloroproline
  MOD_RES (8)..(8): Chloroproline
  MOD_RES (11)..(11): Chloroproline
  MOD_RES (14)..(14): Chloroproline
  MOD_RES (17)..(17): Chloroproline
  MOD_RES (20)..(20): Chloroproline
PPGPCGPPGPPGPPGPPGPPG

SEQ ID NO: 99 - protein, 21 aa, Artificial Sequence
  Description of Artificial Sequence: Synthetic peptide
  MOD_RES (2)..(2): Chloroproline
  MOD_RES (5)..(5): Chloroproline
  MOD_RES (8)..(8): Chloroproline
  MOD_RES (11)..(11): Chloroproline
  MOD_RES (14)..(14): Chloroproline
  MOD_RES (17)..(17): Chloroproline
  MOD_RES (20)..(20): Chloroproline
PPGPPGCPGPPGPPGPPGPPG

SEQ ID NO: 100 - protein, 21 aa, Artificial Sequence
  Description of Artificial Sequence: Synthetic peptide
  MOD_RES (2)..(2): Chloroproline
  MOD_RES (5)..(5): Chloroproline
  MOD_RES (8)..(8): Chloroproline
  MOD_RES (11)..(11): Chloroproline
  MOD_RES (14)..(14): Chloroproline
  MOD_RES (17)..(17): Chloroproline
  MOD_RES (20)..(20): Chloroproline
PPGPPGPPGCPGPPGPPGPPG

SEQ ID NO: 101 - protein, 21 aa, Artificial Sequence
  Description of Artificial Sequence: Synthetic peptide
  MOD_RES (2)..(2): Chloroproline
  MOD_RES (5)..(5): Chloroproline
  MOD_RES (8)..(8): Chloroproline
  MOD_RES (14)..(14): Chloroproline
  MOD_RES (17)..(17): Chloroproline
  MOD_RES (20)..(20): Chloroproline
PPGPPGPPGPCGPPGPPGPPG

SEQ ID NO: 102 - protein, 21 aa, Artificial Sequence
  Description of Artificial Sequence: Synthetic peptide
  MOD_RES (2)..(2): Chloroproline
  MOD_RES (5)..(5): Chloroproline
  MOD_RES (8)..(8): Chloroproline
  MOD_RES (11)..(11): Chloroproline
  MOD_RES (14)..(14): Chloroproline
  MOD_RES (17)..(17): Chloroproline
  MOD_RES (20)..(20): Chloroproline
PPGPPGPPGPPGCPGPPGPPG

SEQ ID NO: 103 - protein, 21 aa, Artificial Sequence
  Description of Artificial Sequence: Synthetic peptide
  MOD_RES (2)..(2): Chloroproline
  MOD_RES (5)..(5): Chloroproline
  MOD_RES (8)..(8): Chloroproline
  MOD_RES (11)..(11): Chloroproline
  MOD_RES (17)..(17): Chloroproline
  MOD_RES (20)..(20): Chloroproline
PPGPPGPPGPPGPCGPPGPPG

SEQ ID NO: 104 - protein, 21 aa, Artificial Sequence
  Description of Artificial Sequence: Synthetic peptide
  MOD_RES (2)..(2): Chloroproline
  MOD_RES (5)..(5): Chloroproline
  MOD_RES (8)..(8): Chloroproline
  MOD_RES (11)..(11): Chloroproline
  MOD_RES (14)..(14): Chloroproline
  MOD_RES (17)..(17): Chloroproline
  MOD_RES (20)..(20): Chloroproline
PPGPPGPPGPPGPPGCPGPPG

SEQ ID NO: 105 - protein, 21 aa, Artificial Sequence
  Description of Artificial Sequence: Synthetic peptide
  MOD_RES (2)..(2): Chloroproline
  MOD_RES (5)..(5): Chloroproline
  MOD_RES (8)..(8): Chloroproline
  MOD_RES (11)..(11): Chloroproline
  MOD_RES (14)..(14): Chloroproline
  MOD_RES (20)..(20): Chloroproline
PPGPPGPPGPPGPPGPCGPPG

SEQ ID NO: 106 - protein, 21 aa, Artificial Sequence
  Description of Artificial Sequence: Synthetic peptide
  MOD_RES (2)..(2): Chloroproline
  MOD_RES (5)..(5): Chloroproline
  MOD_RES (8)..(8): Chloroproline
  MOD_RES (11)..(11): Chloroproline
  MOD_RES (14)..(14): Chloroproline
  MOD_RES (17)..(17): Chloroproline
  MOD_RES (20)..(20): Chloroproline
PPGPPGPPGPPGPPGPPGCPG

SEQ ID NO: 107 - protein, 21 aa, Artificial Sequence
  Description of Artificial Sequence: Synthetic peptide
  MOD_RES (2)..(2): Chloroproline
  MOD_RES (5)..(5): Chloroproline
  MOD_RES (8)..(8): Chloroproline
  MOD_RES (11)..(11): Chloroproline
  MOD_RES (14)..(14): Chloroproline
  MOD_RES (17)..(17): Chloroproline
PPGPPGPPGPPGPPGPPGPCG

SEQ ID NO: 108 - protein, 21 aa, Artificial Sequence
  Description of Artificial Sequence: Synthetic peptide
  MOD_RES (2)..(2): Chloroproline
  MOD_RES (5)..(5): Chloroproline
  MOD_RES (8)..(8): Chloroproline
  MOD_RES (11)..(11): Chloroproline
  MOD_RES (14)..(14): Chloroproline
  MOD_RES (17)..(17): Chloroproline
  MOD_RES (20)..(20): Chloroproline
CPGPPGPPGPPGPPGPPGPPG

SEQ ID NO: 109 - protein, 21 aa, Artificial Sequence
  Description of Artificial Sequence: Synthetic peptide
  MOD_RES (5)..(5): Chloroproline
  MOD_RES (8)..(8): Chloroproline
  MOD_RES (11)..(11): Chloroproline
  MOD_RES (14)..(14): Chloroproline
  MOD_RES (17)..(17): Chloroproline
  MOD_RES (20)..(20): Chloroproline
PCGPPGPPGPPGPPGPPGPPG

SEQ ID NO: 110 - protein, 21 aa, Artificial Sequence
  Description of Artificial Sequence: Synthetic peptide
  MOD_RES (2)..(2): Chloroproline
  MOD_RES (5)..(5): Chloroproline
  MOD_RES (8)..(8): Chloroproline
  MOD_RES (11)..(11): Chloroproline
  MOD_RES (14)..(14): Chloroproline
  MOD_RES (17)..(17): Chloroproline
  MOD_RES (20)..(20): Chloroproline
PPGCPGPPGPPGPPGPPGPPG

SEQ ID NO: 111 - protein, 21 aa, Artificial Sequence
  Description of Artificial Sequence: Synthetic peptide
  MOD_RES (2)..(2): Chloroproline
  MOD_RES (8)..(8): Chloroproline
  MOD_RES (11)..(11): Chloroproline
  MOD_RES (14)..(14): Chloroproline
  MOD_RES (17)..(17): Chloroproline
  MOD_RES (20)..(20): Chloroproline
PPGPCGPPGPPGPPGPPGPPG

SEQ ID NO: 112 - protein, 21 aa, Artificial Sequence
  Description of Artificial Sequence: Synthetic peptide
  MOD_RES (2)..(2): Chloroproline
  MOD_RES (5)..(5): Chloroproline
  MOD_RES (8)..(8): Chloroproline
  MOD_RES (11)..(11): Chloroproline
  MOD_RES (14)..(14): Chloroproline
  MOD_RES (17)..(17): Chloroproline
  MOD_RES (20)..(20): Chloroproline
PPGPPGCPGPPGPPGPPGPPG

SEQ ID NO: 113 - protein, 21 aa, Artificial Sequence
  Description of Artificial Sequence: Synthetic peptide
  MOD_RES (2)..(2): Chloroproline
  MOD_RES (5)..(5): Chloroproline
  MOD_RES (11)..(11): Chloroproline
  MOD_RES (14)..(14): Chloroproline
  MOD_RES (17)..(17): Chloroproline
  MOD_RES (20)..(20): Chloroproline
PPGPPGPCGPPGPPGPPGPPG

SEQ ID NO: 114 - protein, 21 aa, Artificial Sequence
  Description of Artificial Sequence: Synthetic peptide
  MOD_RES (2)..(2): Chloroproline
  MOD_RES (5)..(5): Chloroproline
  MOD_RES (8)..(8): Chloroproline
  MOD_RES (11)..(11): Chloroproline
  MOD_RES (14)..(14): Chloroproline
  MOD_RES (17)..(17): Chloroproline
  MOD_RES (20)..(20): Chloroproline
PPGPPGPPGCPGPPGPPGPPG

SEQ ID NO: 115 - protein, 21 aa, Artificial Sequence
  Description of Artificial Sequence: Synthetic peptide
  MOD_RES (2)..(2): Chloroproline
  MOD_RES (5)..(5): Chloroproline
  MOD_RES (8)..(8): Chloroproline
  MOD_RES (14)..(14): Chloroproline
  MOD_RES (17)..(17): Chloroproline
  MOD_RES (20)..(20): Chloroproline
PPGPPGPPGPCGPPGPPGPPG

SEQ ID NO: 116 - protein, 21 aa, Artificial Sequence
  Description of Artificial Sequence: Synthetic peptide
  MOD_RES (2)..(2): Chloroproline
  MOD_RES (5)..(5): Chloroproline
  MOD_RES (8)..(8): Chloroproline
  MOD_RES (11)..(11): Chloroproline
  MOD_RES (14)..(14): Chloroproline
  MOD_RES (17)..(17): Chloroproline
  MOD_RES (20)..(20): Chloroproline
PPGPPGPPGPPGCPGPPGPPG

SEQ ID NO: 117 - protein, 21 aa, Artificial Sequence
  Description of Artificial Sequence: Synthetic peptide
  MOD_RES (2)..(2): Chloroproline
  MOD_RES (5)..(5): Chloroproline
  MOD_RES (8)..(8): Chloroproline
  MOD_RES (11)..(11): Chloroproline
  MOD_RES (17)..(17): Chloroproline
  MOD_RES (20)..(20): Chloroproline
PPGPPGPPGPPGPCGPPGPPG

SEQ ID NO: 118 - protein, 21 aa, Artificial Sequence
  Description of Artificial Sequence: Synthetic peptide
  MOD_RES (2)..(2): Chloroproline
  MOD_RES (5)..(5): Chloroproline
  MOD_RES (8)..(8): Chloroproline
  MOD_RES (11)..(11): Chloroproline
  MOD_RES (14)..(14): Chloroproline
  MOD_RES (17)..(17): Chloroproline
  MOD_RES (20)..(20): Chloroproline
PPGPPGPPGPPGPPGCPGPPG

SEQ ID NO: 119 - protein, 21 aa, Artificial Sequence
  Description of Artificial Sequence: Synthetic peptide
  MOD_RES (2)..(2): Chloroproline
  MOD_RES (5)..(5): Chloroproline
  MOD_RES (8)..(8): Chloroproline
  MOD_RES (11)..(11): Chloroproline
  MOD_RES (14)..(14): Chloroproline
  MOD_RES (20)..(20): Chloroproline
PPGPPGPPGPPGPPGPCGPPG

SEQ ID NO: 120 - protein, 21 aa, Artificial Sequence
  Description of Artificial Sequence: Synthetic peptide
  MOD_RES (2)..(2): Chloroproline
  MOD_RES (5)..(5): Chloroproline
  MOD_RES (8)..(8): Chloroproline
  MOD_RES (11)..(11): Chloroproline
  MOD_RES (14)..(14): Chloroproline
  MOD_RES (17)..(17): Chloroproline
  MOD_RES (20)..(20): Chloroproline
PPGPPGPPGPPGPPGPPGCPG

SEQ ID NO: 121 - protein, 21 aa, Artificial Sequence
  Description of Artificial Sequence: Synthetic peptide
  MOD_RES (2)..(2): Chloroproline
  MOD_RES (5)..(5): Chloroproline
  MOD_RES (8)..(8): Chloroproline
  MOD_RES (11)..(11): Chloroproline
  MOD_RES (14)..(14): Chloroproline
  MOD_RES (17)..(17): Chloroproline
PPGPPGPPGPPGPPGPPGPCG

SEQ ID NO: 122 - protein, 21 aa, Artificial Sequence
  Description of Artificial Sequence: Synthetic peptide
  MOD_RES (2)..(2): Hydroxyproline
  MOD_RES (4)..(4): Chloroproline
  MOD_RES (5)..(5): Hydroxyproline
  MOD_RES (7)..(7): Chloroproline
  MOD_RES (8)..(8): Hydroxyproline
  MOD_RES (10)..(10): Chloroproline
  MOD_RES (11)..(11): Hydroxyproline
  MOD_RES (13)..(13): Chloroproline
  MOD_RES (14)..(14): Hydroxyproline
  MOD_RES (16)..(16): Chloroproline
  MOD_RES (17)..(17): Hydroxyproline
  MOD_RES (19)..(19): Chloroproline
  MOD_RES (20)..(20): Hydroxyproline
CPGPPGPPGPPGPPGPPGPPG

SEQ ID NO: 123 - protein, 21 aa, Artificial Sequence
  Description of Artificial Sequence: Synthetic peptide
  MOD_RES (1)..(1): Chloroproline
  MOD_RES (4)..(4): Chloroproline
  MOD_RES (5)..(5): Hydroxyproline
  MOD_RES (7)..(7): Chloroproline
  MOD_RES (8)..(8): Hydroxyproline
  MOD_RES (10)..(10): Chloroproline
  MOD_RES (11)..(11): Hydroxyproline
  MOD_RES (13)..(13): Chloroproline
  MOD_RES (14)..(14): Hydroxyproline
  MOD_RES (16)..(16): Chloroproline
  MOD_RES (17)..(17): Hydroxyproline
  MOD_RES (19)..(19): Chloroproline
  MOD_RES (20)..(20): Hydroxyproline
PCGPPGPPGPPGPPGPPGPPG

SEQ ID NO: 124 - protein, 21 aa, Artificial Sequence
  Description of Artificial Sequence: Synthetic peptide
  MOD_RES (1)..(1): Chloroproline
  MOD_RES (2)..(2): Hydroxyproline
  MOD_RES (5)..(5): Hydroxyproline
  MOD_RES (7)..(7): Chloroproline
  MOD_RES (8)..(8): Hydroxyproline
  MOD_RES (10)..(10): Chloroproline
  MOD_RES (11)..(11): Hydroxyproline
  MOD_RES (13)..(13): Chloroproline
  MOD_RES (14)..(14): Hydroxyproline
  MOD_RES (16)..(16): Chloroproline
  MOD_RES (17)..(17): Hydroxyproline
  MOD_RES (19)..(19): Chloroproline
  MOD_RES (20)..(20): Hydroxyproline
PPGCPGPPGPPGPPGPPGPPG

SEQ ID NO: 125 - protein, 21 aa, Artificial Sequence
  Description of Artificial Sequence: Synthetic peptide
  MOD_RES (1)..(1): Chloroproline
  MOD_RES (2)..(2): Hydroxyproline
  MOD_RES (4)..(4): Chloroproline
  MOD_RES (7)..(7): Chloroproline
  MOD_RES (8)..(8): Hydroxyproline
  MOD_RES (10)..(10): Chloroproline
  MOD_RES (11)..(11): Hydroxyproline
  MOD_RES (13)..(13): Chloroproline
  MOD_RES (14)..(14): Hydroxyproline
  MOD_RES (16)..(16): Chloroproline
  MOD_RES (17)..(17): Hydroxyproline
  MOD_RES (19)..(19): Chloroproline
  MOD_RES (20)..(20): Hydroxyproline
PPGPCGPPGPPGPPGPPGPPG

SEQ ID NO: 126 - protein, 21 aa, Artificial Sequence
  Description of Artificial Sequence: Synthetic peptide
  MOD_RES (1)..(1): Chloroproline
  MOD_RES (2)..(2): Hydroxyproline
  MOD_RES (4)..(4): Chloroproline
  MOD_RES (5)..(5): Hydroxyproline
  MOD_RES (8)..(8): Hydroxyproline
  MOD_RES (10)..(10): Chloroproline
  MOD_RES (11)..(11): Hydroxyproline
  MOD_RES (13)..(13): Chloroproline
  MOD_RES (14)..(14): Hydroxyproline
  MOD_RES (16)..(16): Chloroproline
  MOD_RES (17)..(17): Hydroxyproline
  MOD_RES (19)..(19): Chloroproline
  MOD_RES (20)..(20): Hydroxyproline
PPGPPGCPGPPGPPGPPGPPG

SEQ ID NO: 127 - protein, 21 aa, Artificial Sequence
  Description of Artificial Sequence: Synthetic peptide
  MOD_RES (1)..(1): Chloroproline
  MOD_RES (2)..(2): Hydroxyproline
  MOD_RES (4)..(4): Chloroproline
  MOD_RES (5)..(5): Hydroxyproline
  MOD_RES (7)..(7): Chloroproline
  MOD_RES (10)..(10): Chloroproline
  MOD_RES (11)..(11): Hydroxyproline
  MOD_RES (13)..(13): Chloroproline
  MOD_RES (14)..(14): Hydroxyproline
  MOD_RES (16)..(16): Chloroproline
  MOD_RES (17)..(17): Hydroxyproline
  MOD_RES (19)..(19): Chloroproline
  MOD_RES (20)..(20): Hydroxyproline
PPGPPGPCGPPGPPGPPGPPG

SEQ ID NO: 128 - protein, 21 aa, Artificial Sequence
  Description of Artificial Sequence: Synthetic peptide
  MOD_RES (1)..(1): Chloroproline
  MOD_RES (2)..(2): Hydroxyproline
  MOD_RES (4)..(4): Chloroproline
  MOD_RES (5)..(5): Hydroxyproline
  MOD_RES (7)..(7): Chloroproline
  MOD_RES (8)..(8): Hydroxyproline
  MOD_RES (11)..(11): Hydroxyproline
  MOD_RES (13)..(13): Chloroproline
  MOD_RES (14)..(14): Hydroxyproline
  MOD_RES (16)..(16): Chloroproline
  MOD_RES (17)..(17): Hydroxyproline
  MOD_RES (19)..(19): Chloroproline
  MOD_RES (20)..(20): Hydroxyproline
PPGPPGPPGCPGPPGPPGPPG

SEQ ID NO: 129 - protein, 21 aa, Artificial Sequence
  Description of Artificial Sequence: Synthetic peptide
  MOD_RES (1)..(1): Chloroproline
  MOD_RES (2)..(2): Hydroxyproline
  MOD_RES (4)..(4): Chloroproline
  MOD_RES (5)..(5): Hydroxyproline
  MOD_RES (7)..(7): Chloroproline
  MOD_RES (8)..(8): Hydroxyproline
  MOD_RES (10)..(10): Chloroproline
  MOD_RES (13)..(13): Chloroproline
  MOD_RES (14)..(14): Hydroxyproline
  MOD_RES (16)..(16): Chloroproline
  MOD_RES (17)..(17): Hydroxyproline
  MOD_RES (19)..(19): Chloroproline
  MOD_RES (20)..(20): Hydroxyproline
PPGPPGPPGPCGPPGPPGPPG

SEQ ID NO: 130 - protein, 21 aa, Artificial Sequence
  Description of Artificial Sequence: Synthetic peptide
  MOD_RES (1)..(1): Chloroproline
  MOD_RES (2)..(2): Hydroxyproline
  MOD_RES (4)..(4): Chloroproline
  MOD_RES (5)..(5): Hydroxyproline
  MOD_RES (7)..(7): Chloroproline
  MOD_RES (8)..(8): Hydroxyproline
  MOD_RES (10)..(10): Chloroproline
  MOD_RES (11)..(11): Hydroxyproline
  MOD_RES (14)..(14): Hydroxyproline
  MOD_RES (16)..(16): Chloroproline
  MOD_RES (17)..(17): Hydroxyproline
  MOD_RES (19)..(19): Chloroproline
  MOD_RES (20)..(20): Hydroxyproline
PPGPPGPPGPPGCPGPPGPPG

SEQ ID NO: 131 - protein, 21 aa, Artificial Sequence
  Description of Artificial Sequence: Synthetic peptide
  MOD_RES (1)..(1): Chloroproline
  MOD_RES (2)..(2): Hydroxyproline
  MOD_RES (4)..(4): Chloroproline
  MOD_RES (5)..(5): Hydroxyproline
  MOD_RES (7)..(7): Chloroproline
  MOD_RES (8)..(8): Hydroxyproline
  MOD_RES (10)..(10): Chloroproline
  MOD_RES (11)..(11): Hydroxyproline
  MOD_RES (13)..(13): Chloroproline
  MOD_RES (16)..(16): Chloroproline
  MOD_RES (17)..(17): Hydroxyproline
  MOD_RES (19)..(19): Chloroproline
  MOD_RES (20)..(20): Hydroxyproline
PPGPPGPPGPPGPCGPPGPPG

SEQ ID NO: 132 - protein, 21 aa, Artificial Sequence
  Description of Artificial Sequence: Synthetic peptide
  MOD_RES (1)..(1): Chloroproline
  MOD_RES (2)..(2): Hydroxyproline
  MOD_RES (4)..(4): Chloroproline
  MOD_RES (5)..(5): Hydroxyproline
  MOD_RES (7)..(7): Chloroproline
  MOD_RES (8)..(8): Hydroxyproline
  MOD_RES (10)..(10): Chloroproline
  MOD_RES (11)..(11): Hydroxyproline
  MOD_RES (13)..(13): Chloroproline
  MOD_RES (14)..(14): Hydroxyproline
  MOD_RES (17)..(17): Hydroxyproline
  MOD_RES (19)..(19): Chloroproline
  MOD_RES (20)..(20): Hydroxyproline
PPGPPGPPGPPGPPGCPGPPG

SEQ ID NO: 133 - protein, 21 aa, Artificial Sequence
  Description of Artificial Sequence: Synthetic peptide
  MOD_RES (1)..(1): Chloroproline
  MOD_RES (2)..(2): Hydroxyproline
  MOD_RES (4)..(4): Chloroproline
  MOD_RES (5)..(5): Hydroxyproline
  MOD_RES (7)..(7): Chloroproline
  MOD_RES (8)..(8): Hydroxyproline
  MOD_RES (10)..(10): Chloroproline
  MOD_RES (11)..(11): Hydroxyproline
  MOD_RES (13)..(13): Chloroproline
  MOD_RES (14)..(14): Hydroxyproline
  MOD_RES (16)..(16): Chloroproline
  MOD_RES (19)..(19): Chloroproline
  MOD_RES (20)..(20): Hydroxyproline
PPGPPGPPGPPGPPGPCGPPG

SEQ ID NO: 134 - protein, 21 aa, Artificial Sequence
  Description of Artificial Sequence: Synthetic peptide
  MOD_RES (1)..(1): Chloroproline
  MOD_RES (2)..(2): Hydroxyproline
  MOD_RES (4)..(4): Chloroproline
  MOD_RES (5)..(5): Hydroxyproline
  MOD_RES (7)..(7): Chloroproline
  MOD_RES (8)..(8): Hydroxyproline
  MOD_RES (10)..(10): Chloroproline
  MOD_RES (11)..(11): Hydroxyproline
  MOD_RES (13)..(13): Chloroproline
  MOD_RES (14)..(14): Hydroxyproline
  MOD_RES (16)..(16): Chloroproline
  MOD_RES (17)..(17): Hydroxyproline
  MOD_RES (20)..(20): Hydroxyproline
PPGPPGPPGPPGPPGPPGCPG

SEQ ID NO: 135 - protein, 21 aa, Artificial Sequence
  Description of Artificial Sequence: Synthetic peptide
  MOD_RES (1)..(1): Chloroproline
  MOD_RES (2)..(2): Hydroxyproline
  MOD_RES (4)..(4): Chloroproline
  MOD_RES (5)..(5): Hydroxyproline
  MOD_RES (7)..(7): Chloroproline
  MOD_RES (8)..(8): Hydroxyproline
  MOD_RES (10)..(10): Chloroproline
  MOD_RES (11)..(11): Hydroxyproline
  MOD_RES (13)..(13): Chloroproline
  MOD_RES (14)..(14): Hydroxyproline
  MOD_RES (16)..(16): Chloroproline
  MOD_RES (17)..(17): Hydroxyproline
  MOD_RES (19)..(19): Chloroproline
PPGPPGPPGPPGPPGPPGPCG

SEQ ID NO: 136 - protein, 21 aa, Artificial Sequence
  Description of Artificial Sequence: Synthetic peptide
PPGPPGMPGPPGPPGPPGPPG

SEQ ID NO: 137 - protein, 21 aa, Artificial Sequence
  Description of Artificial Sequence: Synthetic peptide
  MOD_RES (1)..(1): Hydroxyproline
  MOD_RES (4)..(4): Hydroxyproline
  MOD_RES (10)..(10): Hydroxyproline
  MOD_RES (13)..(13): Hydroxyproline
  MOD_RES (16)..(16): Hydroxyproline
  MOD_RES (19)..(19): Hydroxyproline
PPGPPGMPGPPGPPGPPGPPG

SEQ ID NO: 138 - protein, 21 aa, Artificial Sequence
  Description of Artificial Sequence: Synthetic peptide
  MOD_RES (2)..(2): Hydroxyproline
  MOD_RES (5)..(5): Hydroxyproline
  MOD_RES (11)..(11): Hydroxyproline
  MOD_RES (14)..(14): Hydroxyproline
  MOD_RES (17)..(17): Hydroxyproline
  MOD_RES (20)..(20): Hydroxyproline
PPGPPGPMGPPGPPGPPGPPG

SEQ ID NO: 139 - protein, 21 aa, Artificial Sequence
  Description of Artificial Sequence: Synthetic peptide
  MOD_RES (2)..(2): Fluoroproline
  MOD_RES (5)..(5): Fluoroproline
  MOD_RES (11)..(11): Fluoroproline
  MOD_RES (14)..(14): Fluoroproline
  MOD_RES (17)..(17): Fluoroproline
  MOD_RES (20)..(20): Fluoroproline
PPGPPGPMGPPGPPGPPGPPG

SEQ ID NO: 140 - protein, 21 aa, Artificial Sequence
  Description of Artificial Sequence: Synthetic peptide
  MOD_RES (2)..(2): Chloroproline
  MOD_RES (5)..(5): Chloroproline
  MOD_RES (11)..(11): Chloroproline
  MOD_RES (14)..(14): Chloroproline
  MOD_RES (17)..(17): Chloroproline
  MOD_RES (20)..(20): Chloroproline
PPGPPGPMGPPGPPGPPGPPG

SEQ ID NO: 141 - protein, 21 aa, Artificial Sequence
  Description of Artificial Sequence: Synthetic peptide
MPGPPGPPGPPGPPGPPGPPG

SEQ ID NO: 142 - protein, 21 aa, Artificial Sequence
  Description of Artificial Sequence: Synthetic peptide
PMGPPGPPGPPGPPGPPGPPG

SEQ ID NO: 143 - protein, 21 aa, Artificial Sequence
  Description of Artificial Sequence: Synthetic peptide
PPGMPGPPGPPGPPGPPGPPG

SEQ ID NO: 144 - protein, 21 aa, Artificial Sequence
  Description of Artificial Sequence: Synthetic peptide
PPGPMGPPGPPGPPGPPGPPG

SEQ ID NO: 145 - protein, 21 aa, Artificial Sequence
  Description of Artificial Sequence: Synthetic peptide
PPGPPGPMGPPGPPGPPGPPG

SEQ ID NO: 146 - protein, 21 aa, Artificial Sequence
  Description of Artificial Sequence: Synthetic peptide
PPGPPGPPGMPGPPGPPGPPG

SEQ ID NO: 147 - protein, 21 aa, Artificial Sequence
  Description of Artificial Sequence: Synthetic peptide
PPGPPGPPGPMGPPGPPGPPG

SEQ ID NO: 148 - protein, 21 aa, Artificial Sequence
  Description of Artificial Sequence: Synthetic peptide
PPGPPGPPGPPGMPGPPGPPG

SEQ ID NO: 149 - protein, 21 aa, Artificial Sequence
  Description of Artificial Sequence: Synthetic peptide
PPGPPGPPGPPGPMGPPGPPG

SEQ ID NO: 150 - protein, 21 aa, Artificial Sequence
  Description of Artificial Sequence: Synthetic peptide
PPGPPGPPGPPGPPGMPGPPG

SEQ ID NO: 151 - protein, 21 aa, Artificial Sequence
  Description of Artificial Sequence: Synthetic peptide
PPGPPGPPGPPGPPGPMGPPG

SEQ ID NO: 152 - protein, 21 aa, Artificial Sequence
  Description of Artificial Sequence: Synthetic peptide
PPGPPGPPGPPGPPGPPGMPG

SEQ ID NO: 153 - protein, 21 aa, Artificial Sequence
  Description of Artificial Sequence: Synthetic peptide
PPGPPGPPGPPGPPGPPGPMG

SEQ ID NO: 154 - protein, 21 aa, Artificial Sequence
  Description of Artificial Sequence: Synthetic peptide
  MOD_RES (4)..(4): Hydroxyproline
  MOD_RES (7)..(7): Hydroxyproline
  MOD_RES (10)..(10): Hydroxyproline
  MOD_RES (13)..(13): Hydroxyproline
  MOD_RES (16)..(16): Hydroxyproline
  MOD_RES (19)..(19): Hydroxyproline
MPGPPGPPGPPGPPGPPGPPG

SEQ ID NO: 155 - protein, 21 aa, Artificial Sequence
  Description of Artificial Sequence: Synthetic peptide
  MOD_RES (1)..(1): Hydroxyproline
  MOD_RES (4)..(4): Hydroxyproline
  MOD_RES (7)..(7): Hydroxyproline
  MOD_RES (10)..(10): Hydroxyproline
  MOD_RES (13)..(13): Hydroxyproline
  MOD_RES (16)..(16): Hydroxyproline
  MOD_RES (19)..(19): Hydroxyproline
PMGPPGPPGPPGPPGPPGPPG

SEQ ID NO: 156 - protein, 21 aa, Artificial Sequence
  Description of Artificial Sequence: Synthetic peptide
  MOD_RES (1)..(1): Hydroxyproline
  MOD_RES (7)..(7): Hydroxyproline
  MOD_RES (10)..(10): Hydroxyproline
  MOD_RES (13)..(13): Hydroxyproline
  MOD_RES (16)..(16): Hydroxyproline
  MOD_RES (19)..(19): Hydroxyproline
PPGMPGPPGPPGPPGPPGPPG

SEQ ID NO: 157 - protein, 21 aa, Artificial Sequence
  Description of Artificial Sequence: Synthetic peptide
  MOD_RES (1)..(1): Hydroxyproline
  MOD_RES (4)..(4): Hydroxyproline
  MOD_RES (7)..(7): Hydroxyproline
  MOD_RES (10)..(10): Hydroxyproline
  MOD_RES (13)..(13): Hydroxyproline
  MOD_RES (16)..(16): Hydroxyproline
  MOD_RES (19)..(19): Hydroxyproline
PPGPMGPPGPPGPPGPPGPPG

SEQ ID NO: 158 - protein, 21 aa, Artificial Sequence
  Description of Artificial Sequence: Synthetic peptide
  MOD_RES (1)..(1): Hydroxyproline
  MOD_RES (4)..(4): Hydroxyproline
  MOD_RES (7)..(7): Hydroxyproline
  MOD_RES (10)..(10): Hydroxyproline
  MOD_RES (13)..(13): Hydroxyproline
  MOD_RES (16)..(16): Hydroxyproline
  MOD_RES (19)..(19): Hydroxyproline
PPGPPGPMGPPGPPGPPGPPG

SEQ ID NO: 159 - protein, 21 aa, Artificial Sequence
  Description of Artificial Sequence: Synthetic peptide
  MOD_RES (1)..(1): Hydroxyproline
  MOD_RES (4)..(4): Hydroxyproline
  MOD_RES (7)..(7): Hydroxyproline
  MOD_RES (13)..(13): Hydroxyproline
  MOD_RES (16)..(16): Hydroxyproline
  MOD_RES (19)..(19): Hydroxyproline
PPGPPGPPGMPGPPGPPGPPG

SEQ ID NO: 160 - protein, 21 aa, Artificial Sequence
  Description of Artificial Sequence: Synthetic peptide
  MOD_RES (1)..(1): Hydroxyproline
  MOD_RES (4)..(4): Hydroxyproline
  MOD_RES (7)..(7): Hydroxyproline
  MOD_RES (10)..(10): Hydroxyproline
  MOD_RES (13)..(13): Hydroxyproline
  MOD_RES (16)..(16): Hydroxyproline
  MOD_RES (19)..(19): Hydroxyproline
PPGPPGPPGPMGPPGPPGPPG

SEQ ID NO: 161 - protein, 21 aa, Artificial Sequence
  Description of Artificial Sequence: Synthetic peptide
  MOD_RES (1)..(1): Hydroxyproline
  MOD_RES (4)..(4): Hydroxyproline
  MOD_RES (7)..(7): Hydroxyproline
  MOD_RES (10)..(10): Hydroxyproline
  MOD_RES (16)..(16): Hydroxyproline
  MOD_RES (19)..(19): Hydroxyproline
PPGPPGPPGPPGMPGPPGPPG

SEQ ID NO: 162 - protein, 21 aa, Artificial Sequence
  Description of Artificial Sequence: Synthetic peptide
  MOD_RES (1)..(1): Hydroxyproline
  MOD_RES (4)..(4): Hydroxyproline
  MOD_RES (7)..(7): Hydroxyproline
  MOD_RES (10)..(10): Hydroxyproline
  MOD_RES (13)..(13): Hydroxyproline
  MOD_RES (16)..(16): Hydroxyproline
  MOD_RES (19)..(19): Hydroxyproline
PPGPPGPPGPPGPMGPPGPPG

SEQ ID NO: 163 - protein, 21 aa, Artificial Sequence
  Description of Artificial Sequence: Synthetic peptide
  MOD_RES (1)..(1): Hydroxyproline
  MOD_RES (4)..(4): Hydroxyproline
  MOD_RES (7)..(7): Hydroxyproline
  MOD_RES (10)..(10): Hydroxyproline
  MOD_RES (13)..(13): Hydroxyproline
  MOD_RES (19)..(19): Hydroxyproline
PPGPPGPPGPPGPPGMPGPPG

SEQ ID NO: 164 - protein, 21 aa, Artificial Sequence
  Description of Artificial Sequence: Synthetic peptide
  MOD_RES (1)..(1): Hydroxyproline
  MOD_RES (4)..(4): Hydroxyproline
  MOD_RES (7)..(7): Hydroxyproline
  MOD_RES (10)..(10): Hydroxyproline
  MOD_RES (13)..(13): Hydroxyproline
  MOD_RES (16)..(16): Hydroxyproline
  MOD_RES (19)..(19): Hydroxyproline
PPGPPGPPGPPGPPGPMGPPG

SEQ ID NO: 165 - protein, 21 aa, Artificial Sequence
  Description of Artificial Sequence: Synthetic peptide
  MOD_RES (1)..(1): Hydroxyproline
  MOD_RES (4)..(4): Hydroxyproline
  MOD_RES (7)..(7): Hydroxyproline
  MOD_RES (10)..(10): Hydroxyproline
  MOD_RES (13)..(13): Hydroxyproline
  MOD_RES (16)..(16): Hydroxyproline
PPGPPGPPGPPGPPGPPGMPG

SEQ ID NO: 166 - protein, 21 aa, Artificial Sequence
  Description of Artificial Sequence: Synthetic peptide
  MOD_RES (1)..(1): Hydroxyproline
  MOD_RES (4)..(4): Hydroxyproline
  MOD_RES (7)..(7): Hydroxyproline
  MOD_RES (10)..(10): Hydroxyproline
  MOD_RES (13)..(13): Hydroxyproline
  MOD_RES (16)..(16): Hydroxyproline
  MOD_RES (19)..(19): Hydroxyproline
PPGPPGPPGPPGPPGPPGPMG

SEQ ID NO: 167 - protein, 21 aa, Artificial Sequence
  Description of Artificial Sequence: Synthetic peptide
  MOD_RES (2)..(2): Hydroxyproline
  MOD_RES (5)..(5): Hydroxyproline
  MOD_RES (8)..(8): Hydroxyproline
  MOD_RES (11)..(11): Hydroxyproline
  MOD_RES (14)..(14): Hydroxyproline
  MOD_RES (17)..(17): Hydroxyproline
  MOD_RES (20)..(20): Hydroxyproline
MPGPPGPPGPPGPPGPPGPPG

SEQ ID NO: 168 - protein, 21 aa, Artificial Sequence
  Description of Artificial Sequence: Synthetic peptide
  MOD_RES (5)..(5): Hydroxyproline
  MOD_RES (8)..(8): Hydroxyproline
  MOD_RES (11)..(11): Hydroxyproline
  MOD_RES (14)..(14): Hydroxyproline
  MOD_RES (17)..(17): Hydroxyproline
  MOD_RES (20)..(20): Hydroxyproline
PMGPPGPPGPPGPPGPPGPPG

SEQ ID NO: 169 - protein, 21 aa, Artificial Sequence
  Description of Artificial Sequence: Synthetic peptide
  MOD_RES (2)..(2): Hydroxyproline
  MOD_RES (5)..(5): Hydroxyproline
  MOD_RES (8)..(8): Hydroxyproline
  MOD_RES (11)..(11): Hydroxyproline
  MOD_RES (14)..(14): Hydroxyproline
  MOD_RES (17)..(17): Hydroxyproline
  MOD_RES (20)..(20): Hydroxyproline
PPGMPGPPGPPGPPGPPGPPG

SEQ ID NO: 170 - protein, 21 aa, Artificial Sequence
  Description of Artificial Sequence: Synthetic peptide
  MOD_RES (2)..(2): Hydroxyproline
  MOD_RES (8)..(8): Hydroxyproline
  MOD_RES (11)..(11): Hydroxyproline
  MOD_RES (14)..(14): Hydroxyproline
  MOD_RES (17)..(17): Hydroxyproline
  MOD_RES (20)..(20): Hydroxyproline
PPGPMGPPGPPGPPGPPGPPG

SEQ ID NO: 171 - protein, 21 aa, Artificial Sequence
  Description of Artificial Sequence: Synthetic peptide
  MOD_RES (2)..(2): Hydroxyproline
  MOD_RES (5)..(5): Hydroxyproline
  MOD_RES (8)..(8): Hydroxyproline
  MOD_RES (11)..(11): Hydroxyproline
  MOD_RES (14)..(14): Hydroxyproline
  MOD_RES (17)..(17): Hydroxyproline
  MOD_RES (20)..(20): Hydroxyproline
PPGPPGMPGPPGPPGPPGPPG

SEQ ID NO: 172 - protein, 21 aa, Artificial Sequence
  Description of Artificial Sequence: Synthetic peptide
  MOD_RES (2)..(2): Hydroxyproline
  MOD_RES (5)..(5): Hydroxyproline
  MOD_RES (8)..(8): Hydroxyproline
  MOD_RES (11)..(11): Hydroxyproline
  MOD_RES (14)..(14): Hydroxyproline
  MOD_RES (17)..(17): Hydroxyproline
  MOD_RES (20)..(20): Hydroxyproline
PPGPPGPPGMPGPPGPPGPPG

SEQ ID NO: 173 - protein, 21 aa, Artificial Sequence
  Description of Artificial Sequence: Synthetic peptide
  MOD_RES (2)..(2): Hydroxyproline
  MOD_RES (5)..(5): Hydroxyproline
  MOD_RES (8)..(8): Hydroxyproline
  MOD_RES (14)..(14): Hydroxyproline
  MOD_RES (17)..(17): Hydroxyproline
  MOD_RES (20)..(20): Hydroxyproline
PPGPPGPPGPMGPPGPPGPPG

SEQ ID NO: 174 - protein, 21 aa, Artificial Sequence
  Description of Artificial Sequence: Synthetic peptide
  MOD_RES (2)..(2): Hydroxyproline
  MOD_RES (5)..(5): Hydroxyproline
  MOD_RES (8)..(8): Hydroxyproline
  MOD_RES (11)..(11): Hydroxyproline
  MOD_RES (14)..(14): Hydroxyproline
  MOD_RES (17)..(17): Hydroxyproline
  MOD_RES (20)..(20): Hydroxyproline
PPGPPGPPGPPGMPGPPGPPG

SEQ ID NO: 175 - protein, 21 aa, Artificial Sequence
  Description of Artificial Sequence: Synthetic peptide
  MOD_RES (2)..(2): Hydroxyproline
  MOD_RES (5)..(5): Hydroxyproline
  MOD_RES (8)..(8): Hydroxyproline
  MOD_RES (11)..(11): Hydroxyproline
  MOD_RES (17)..(17): Hydroxyproline
  MOD_RES (20)..(20): Hydroxyproline
PPGPPGPPGPPGPMGPPGPPG

SEQ ID NO: 176 - protein, 21 aa, Artificial Sequence
  Description of Artificial Sequence: Synthetic peptide
  MOD_RES (2)..(2): Hydroxyproline
  MOD_RES (5)..(5): Hydroxyproline
  MOD_RES (8)..(8): Hydroxyproline
  MOD_RES (11)..(11): Hydroxyproline
  MOD_RES (14)..(14): Hydroxyproline
  MOD_RES (17)..(17): Hydroxyproline
  MOD_RES (20)..(20): Hydroxyproline
PPGPPGPPGPPGPPGMPGPPG

SEQ ID NO: 177 - protein, 21 aa, Artificial Sequence
  Description of Artificial Sequence: Synthetic peptide
  MOD_RES (2)..(2): Hydroxyproline
  MOD_RES (5)..(5): Hydroxyproline
  MOD_RES (8)..(8): Hydroxyproline
  MOD_RES (11)..(11): Hydroxyproline
  MOD_RES (14)..(14): Hydroxyproline
  MOD_RES (20)..(20): Hydroxyproline
PPGPPGPPGPPGPPGPMGPPG

SEQ ID NO: 178 - protein, 21 aa, Artificial Sequence
  Description of Artificial Sequence: Synthetic peptide
  MOD_RES (2)..(2): Hydroxyproline
  MOD_RES (5)..(5): Hydroxyproline
  MOD_RES (8)..(8): Hydroxyproline
  MOD_RES (11)..(11): Hydroxyproline
  MOD_RES (14)..(14): Hydroxyproline
  MOD_RES (17)..(17): Hydroxyproline
  MOD_RES (20)..(20): Hydroxyproline
PPGPPGPPGPPGPPGPPGMPG

SEQ ID NO: 179 - protein, 21 aa, Artificial Sequence
  Description of Artificial Sequence: Synthetic peptide
  MOD_RES (2)..(2): Hydroxyproline
  MOD_RES (5)..(5): Hydroxyproline
  MOD_RES (8)..(8): Hydroxyproline
  MOD_RES (11)..(11): Hydroxyproline
  MOD_RES (14)..(14): Hydroxyproline
  MOD_RES (17)..(17): Hydroxyproline
PPGPPGPPGPPGPPGPPGPMG

SEQ ID NO: 180 - protein, 21 aa, Artificial Sequence
  Description of Artificial Sequence: Synthetic peptide
  MOD_RES (2)..(2): Fluoroproline
  MOD_RES (5)..(5): Fluoroproline
  MOD_RES (8)..(8): Fluoroproline
  MOD_RES (11)..(11): Fluoroproline
  MOD_RES (14)..(14): Fluoroproline
  MOD_RES (17)..(17): Fluoroproline
  MOD_RES (20)..(20): Fluoroproline
MPGPPGPPGPPGPPGPPGPPG

SEQ ID NO: 181 - protein, 21 aa, Artificial Sequence
  Description of Artificial Sequence: Synthetic peptide
  MOD_RES (5)..(5): Fluoroproline
  MOD_RES (8)..(8): Fluoroproline
  MOD_RES (11)..(11): Fluoroproline
  MOD_RES (14)..(14): Fluoroproline
  MOD_RES (17)..(17): Fluoroproline
  MOD_RES (20)..(20): Fluoroproline
PMGPPGPPGPPGPPGPPGPPG

SEQ ID NO: 182 - protein, 21 aa, Artificial Sequence
  Description of Artificial Sequence: Synthetic peptide
  MOD_RES (2)..(2): Fluoroproline
  MOD_RES (5)..(5): Fluoroproline
  MOD_RES (8)..(8): Fluoroproline
  MOD_RES (11)..(11): Fluoroproline
  MOD_RES (14)..(14): Fluoroproline
  MOD_RES (17)..(17): Fluoroproline
  MOD_RES (20)..(20): Fluoroproline
PPGMPGPPGPPGPPGPPGPPG

SEQ ID NO: 183 - protein, 21 aa, Artificial Sequence
  Description of Artificial Sequence: Synthetic peptide
  MOD_RES (2)..(2): Fluoroproline
  MOD_RES (8)..(8): Fluoroproline
  MOD_RES (11)..(11): Fluoroproline
  MOD_RES (14)..(14): Fluoroproline
  MOD_RES (17)..(17): Fluoroproline
  MOD_RES (20)..(20): Fluoroproline
PPGPMGPPGPPGPPGPPGPPG

SEQ ID NO: 184 - protein, 21 aa, Artificial Sequence
  Description of Artificial Sequence: Synthetic peptide
  MOD_RES (2)..(2): Fluoroproline
  MOD_RES (5)..(5): Fluoroproline
  MOD_RES (8)..(8): Fluoroproline
  MOD_RES (11)..(11): Fluoroproline
  MOD_RES (14)..(14): Fluoroproline
  MOD_RES (17)..(17): Fluoroproline
  MOD_RES (20)..(20): Fluoroproline
PPGPPGMPGPPGPPGPPGPPG

SEQ ID NO: 185 - protein, 21 aa, Artificial Sequence
  Description of Artificial Sequence: Synthetic peptide
  MOD_RES (2)..(2): Fluoroproline
  MOD_RES (5)..(5): Fluoroproline
  MOD_RES (8)..(8): Fluoroproline
  MOD_RES (11)..(11): Fluoroproline
  MOD_RES (14)..(14): Fluoroproline
  MOD_RES (17)..(17): Fluoroproline
  MOD_RES (20)..(20): Fluoroproline
PPGPPGPPGMPGPPGPPGPPG

SEQ ID NO: 186 - protein, 21 aa, Artificial Sequence
  Description of Artificial Sequence: Synthetic peptide
  MOD_RES (2)..(2): Fluoroproline
  MOD_RES (5)..(5): Fluoroproline
  MOD_RES (8)..(8): Fluoroproline
  MOD_RES (14)..(14): Fluoroproline
  MOD_RES (17)..(17): Fluoroproline
  MOD_RES (20)..(20): Fluoroproline
PPGPPGPPGPMGPPGPPGPPG

SEQ ID NO: 187 - protein, 21 aa, Artificial Sequence
  Description of Artificial Sequence: Synthetic peptide
  MOD_RES (2)..(2): Fluoroproline
  MOD_RES (5)..(5): Fluoroproline
  MOD_RES (8)..(8): Fluoroproline
  MOD_RES (11)..(11): Fluoroproline
  MOD_RES (14)..(14): Fluoroproline
  MOD_RES (17)..(17): Fluoroproline
  MOD_RES (20)..(20): Fluoroproline
PPGPPGPPGPPGMPGPPGPPG

SEQ ID NO: 188 - protein, 21 aa, Artificial Sequence
  Description of Artificial Sequence: Synthetic peptide
  MOD_RES (2)..(2): Fluoroproline
  MOD_RES (5)..(5): Fluoroproline
  MOD_RES (8)..(8): Fluoroproline
  MOD_RES (11)..(11): Fluoroproline
  MOD_RES (17)..(17): Fluoroproline
  MOD_RES (20)..(20): Fluoroproline
PPGPPGPPGPPGPMGPPGPPG

SEQ ID NO: 189 - protein, 21 aa, Artificial Sequence
  Description of Artificial Sequence: Synthetic peptide
  MOD_RES (2)..(2): Fluoroproline
  MOD_RES (5)..(5): Fluoroproline
  MOD_RES (8)..(8): Fluoroproline
  MOD_RES (11)..(11): Fluoroproline
  MOD_RES (14)..(14): Fluoroproline
  MOD_RES (17)..(17): Fluoroproline
  MOD_RES (20)..(20): Fluoroproline
PPGPPGPPGPPGPPGMPGPPG

SEQ ID NO: 190 - protein, 21 aa, Artificial Sequence
  Description of Artificial Sequence: Synthetic peptide
  MOD_RES (2)..(2): Fluoroproline
  MOD_RES (5)..(5): Fluoroproline
  MOD_RES (8)..(8): Fluoroproline
  MOD_RES (11)..(11): Fluoroproline
  MOD_RES (14)..(14): Fluoroproline
  MOD_RES (20)..(20): Fluoroproline
PPGPPGPPGPPGPPGPMGPPG

SEQ ID NO: 191 - protein, 21 aa, Artificial Sequence
  Description of Artificial Sequence: Synthetic peptide
  MOD_RES (2)..(2): Fluoroproline
  MOD_RES (5)..(5): Fluoroproline
  MOD_RES (8)..(8): Fluoroproline
  MOD_RES (11)..(11): Fluoroproline
  MOD_RES (14)..(14): Fluoroproline
  MOD_RES (17)..(17): Fluoroproline
  MOD_RES (20)..(20): Fluoroproline
PPGPPGPPGPPGPPGPPGMPG

SEQ ID NO: 192 - protein, 21 aa, Artificial Sequence
  Description of Artificial Sequence: Synthetic peptide
  MOD_RES (2)..(2): Fluoroproline
  MOD_RES (5)..(5): Fluoroproline
  MOD_RES (8)..(8): Fluoroproline
  MOD_RES (11)..(11): Fluoroproline
  MOD_RES (14)..(14): Fluoroproline
  MOD_RES (17)..(17): Fluoroproline
PPGPPGPPGPPGPPGPPGPMG

SEQ ID NO: 193 - protein, 21 aa, Artificial Sequence
  Description of Artificial Sequence: Synthetic peptide
  MOD_RES (2)..(2): Fluoroproline
  MOD_RES (5)..(5): Fluoroproline
  MOD_RES (8)..(8): Fluoroproline
  MOD_RES (11)..(11): Fluoroproline
  MOD_RES (14)..(14): Fluoroproline
  MOD_RES (17)..(17): Fluoroproline
  MOD_RES (20)..(20): Fluoroproline
MPGPPGPPGPPGPPGPPGPPG

SEQ ID NO: 194 - protein, 21 aa, Artificial Sequence
  Description of Artificial Sequence: Synthetic peptide
  MOD_RES (5)..(5): Fluoroproline
  MOD_RES (8)..(8): Fluoroproline
  MOD_RES (11)..(11): Fluoroproline
  MOD_RES (14)..(14): Fluoroproline
  MOD_RES (17)..(17): Fluoroproline
  MOD_RES (20)..(20): Fluoroproline
PMGPPGPPGPPGPPGPPGPPG

SEQ ID NO: 195 - protein, 21 aa, Artificial Sequence
  Description of Artificial Sequence: Synthetic peptide
  MOD_RES (2)..(2): Fluoroproline
  MOD_RES (5)..(5): Fluoroproline
  MOD_RES (8)..(8): Fluoroproline
  MOD_RES (11)..(11): Fluoroproline
  MOD_RES (14)..(14): Fluoroproline
  MOD_RES (17)..(17): Fluoroproline
  MOD_RES (20)..(20): Fluoroproline
PPGMPGPPGPPGPPGPPGPPG

SEQ ID NO: 196 - protein, 21 aa, Artificial Sequence
  Description of Artificial Sequence: Synthetic peptide
  MOD_RES (2)..(2): Fluoroproline
  MOD_RES (8)..(8): Fluoroproline
  MOD_RES (11)..(11): Fluoroproline
  MOD_RES (14)..(14): Fluoroproline
  MOD_RES (17)..(17): Fluoroproline
  MOD_RES (20)..(20): Fluoroproline
PPGPMGPPGPPGPPGPPGPPG

SEQ ID NO: 197 - protein, 21 aa, Artificial Sequence
  Description of Artificial Sequence: Synthetic peptide
  MOD_RES (2)..(2): Fluoroproline
  MOD_RES (5)..(5): Fluoroproline
  MOD_RES (8)..(8): Fluoroproline
  MOD_RES (11)..(11): Fluoroproline
  MOD_RES (14)..(14): Fluoroproline
  MOD_RES (17)..(17): Fluoroproline
  MOD_RES (20)..(20): Fluoroproline
PPGPPGMPGPPGPPGPPGPPG

SEQ ID NO: 198 - protein, 21 aa, Artificial Sequence
  Description of Artificial Sequence: Synthetic peptide
  MOD_RES (2)..(2): Fluoroproline
  MOD_RES (5)..(5): Fluoroproline
  MOD_RES (11)..(11): Fluoroproline
  MOD_RES (14)..(14): Fluoroproline
  MOD_RES (17)..(17): Fluoroproline
  MOD_RES (20)..(20): Fluoroproline
PPGPPGPMGPPGPPGPPGPPG

SEQ ID NO: 199 - protein, 21 aa, Artificial Sequence
  Description of Artificial Sequence: Synthetic peptide
  MOD_RES (2)..(2): Fluoroproline
  MOD_RES (5)..(5): Fluoroproline
  MOD_RES (8)..(8): Fluoroproline
  MOD_RES (11)..(11): Fluoroproline
  MOD_RES (14)..(14): Fluoroproline
  MOD_RES (17)..(17): Fluoroproline
  MOD_RES (20)..(20): Fluoroproline
PPGPPGPPGMPGPPGPPGPPG

SEQ ID NO: 200 - protein, 21 aa, Artificial Sequence
  Description of Artificial Sequence: Synthetic peptide
  MOD_RES (2)..(2): Fluoroproline
  MOD_RES (5)..(5): Fluoroproline
  MOD_RES (8)..(8): Fluoroproline
  MOD_RES (14)..(14): Fluoroproline
  MOD_RES (17)..(17): Fluoroproline
  MOD_RES (20)..(20): Fluoroproline
PPGPPGPPGPMGPPGPPGPPG

SEQ ID NO: 201 - protein, 21 aa, Artificial Sequence
  Description of Artificial Sequence: Synthetic peptide
  MOD_RES (2)..(2): Fluoroproline
  MOD_RES (5)..(5): Fluoroproline
  MOD_RES (8)..(8): Fluoroproline
  MOD_RES (11)..(11): Fluoroproline
  MOD_RES (14)..(14): Fluoroproline
  MOD_RES (17)..(17): Fluoroproline
  MOD_RES (20)..(20): Fluoroproline
PPGPPGPPGPPGMPGPPGPPG

SEQ ID NO: 202 - protein, 21 aa, Artificial Sequence
  Description of Artificial Sequence: Synthetic peptide
  MOD_RES (2)..(2): Fluoroproline
  MOD_RES (5)..(5): Fluoroproline
  MOD_RES (8)..(8): Fluoroproline
  MOD_RES (11)..(11): Fluoroproline
  MOD_RES (17)..(17): Fluoroproline
  MOD_RES (20)..(20): Fluoroproline
PPGPPGPPGPPGPMGPPGPPG

SEQ ID NO: 203 - protein, 21 aa, Artificial Sequence
  Description of Artificial Sequence: Synthetic peptide
  MOD_RES (2)..(2): Fluoroproline
  MOD_RES (5)..(5): Fluoroproline
  MOD_RES (8)..(8): Fluoroproline
  MOD_RES (11)..(11): Fluoroproline
  MOD_RES (14)..(14): Fluoroproline
  MOD_RES (17)..(17): Fluoroproline
  MOD_RES (20)..(20): Fluoroproline
PPGPPGPPGPPGPPGMPGPPG

SEQ ID NO: 204 - protein, 21 aa, Artificial Sequence
  Description of Artificial Sequence: Synthetic peptide
  MOD_RES (2)..(2): Fluoroproline
  MOD_RES (5)..(5): Fluoroproline
  MOD_RES (8)..(8): Fluoroproline
  MOD_RES (11)..(11): Fluoroproline
  MOD_RES (14)..(14): Fluoroproline
  MOD_RES (20)..(20): Fluoroproline
PPGPPGPPGPPGPPGPMGPPG

SEQ ID NO: 205 - protein, 21 aa, Artificial Sequence
  Description of Artificial Sequence: Synthetic peptide
  MOD_RES (2)..(2): Fluoroproline
  MOD_RES (5)..(5): Fluoroproline
  MOD_RES (8)..(8): Fluoroproline
  MOD_RES (11)..(11): Fluoroproline
  MOD_RES (14)..(14): Fluoroproline
  MOD_RES (17)..(17): Fluoroproline
  MOD_RES (20)..(20): Fluoroproline
PPGPPGPPGPPGPPGPPGMPG

SEQ ID NO: 206 - protein, 21 aa, Artificial Sequence
  Description of Artificial Sequence: Synthetic peptide
  MOD_RES (2)..(2): Fluoroproline
  MOD_RES (5)..(5): Fluoroproline
  MOD_RES (8)..(8): Fluoroproline
  MOD_RES (11)..(11): Fluoroproline
  MOD_RES (14)..(14): Fluoroproline
  MOD_RES (17)..(17): Fluoroproline
PPGPPGPPGPPGPPGPPGPMG

SEQ ID NO: 207 - protein, 21 aa, Artificial Sequence
  Description of Artificial Sequence: Synthetic peptide
  MOD_RES (2)..(2): Hydroxyproline
  MOD_RES (4)..(4): Fluoroproline
  MOD_RES (5)..(5): Hydroxyproline
  MOD_RES (7)..(7): Fluoroproline
  MOD_RES (8)..(8): Hydroxyproline
  MOD_RES (10)..(10): Fluoroproline
  MOD_RES (11)..(11): Hydroxyproline
  MOD_RES (13)..(13): Fluoroproline
  MOD_RES (14)..(14): Hydroxyproline
  MOD_RES (16)..(16): Fluoroproline
  MOD_RES (17)..(17): Hydroxyproline
  MOD_RES (19)..(19): Fluoroproline
  MOD_RES (20)..(20): Hydroxyproline
MPGPPGPPGPPGPPGPPGPPG

SEQ ID NO: 208 - protein, 21 aa, Artificial Sequence
  Description of Artificial Sequence: Synthetic peptide
  MOD_RES (1)..(1): Fluoroproline
  MOD_RES (4)..(4): Fluoroproline
  MOD_RES (5)..(5): Hydroxyproline
  MOD_RES (7)..(7): Fluoroproline
  MOD_RES (8)..(8): Hydroxyproline
  MOD_RES (10)..(10): Fluoroproline
  MOD_RES (11)..(11): Hydroxyproline
  MOD_RES (13)..(13): Fluoroproline
  MOD_RES (14)..(14): Hydroxyproline
  MOD_RES (16)..(16): Fluoroproline
  MOD_RES (17)..(17): Hydroxyproline
  MOD_RES (19)..(19): Fluoroproline
  MOD_RES (20)..(20): Hydroxyproline
PMGPPGPPGPPGPPGPPGPPG

SEQ ID NO: 209 - protein, 21 aa, Artificial Sequence
  Description of Artificial Sequence: Synthetic peptide
  MOD_RES (1)..(1): Fluoroproline
  MOD_RES (2)..(2): Hydroxyproline
  MOD_RES (5)..(5): Hydroxyproline
  MOD_RES (7)..(7): Fluoroproline
  MOD_RES (8)..(8): Hydroxyproline
  MOD_RES (10)..(10): Fluoroproline
  MOD_RES (11)..(11): Hydroxyproline
  MOD_RES (13)..(13): Fluoroproline
  MOD_RES (14)..(14): Hydroxyproline
  MOD_RES (16)..(16): Fluoroproline
  MOD_RES (17)..(17): Hydroxyproline
  MOD_RES (19)..(19): Fluoroproline
  MOD_RES (20)..(20): Hydroxyproline
PPGMPGPPGPPGPPGPPGPPG

SEQ ID NO: 210 - protein, 21 aa, Artificial Sequence
  Description of Artificial Sequence: Synthetic peptide
  MOD_RES (1)..(1): Fluoroproline
  MOD_RES (2)..(2): Hydroxyproline
  MOD_RES (4)..(4): Fluoroproline
  MOD_RES (7)..(7): Fluoroproline
  MOD_RES (8)..(8): Hydroxyproline
  MOD_RES (10)..(10): Fluoroproline
  MOD_RES (11)..(11): Hydroxyproline
  MOD_RES (13)..(13): Fluoroproline
  MOD_RES (14)..(14): Hydroxyproline
  MOD_RES (16)..(16): Fluoroproline
  MOD_RES (17)..(17): Hydroxyproline
  MOD_RES (19)..(19): Fluoroproline
  MOD_RES (20)..(20): Hydroxyproline
PPGPMGPPGPPGPPGPPGPPG

SEQ ID NO: 211 - protein, 21 aa, Artificial Sequence
  Description of Artificial Sequence: Synthetic peptide
  MOD_RES (1)..(1): Fluoroproline
  MOD_RES (2)..(2): Hydroxyproline
  MOD_RES (4)..(4): Fluoroproline
  MOD_RES (5)..(5): Hydroxyproline
  MOD_RES (8)..(8): Hydroxyproline
  MOD_RES (10)..(10): Fluoroproline
  MOD_RES (11)..(11): Hydroxyproline
  MOD_RES (13)..(13): Fluoroproline
  MOD_RES (14)..(14): Hydroxyproline
  MOD_RES (16)..(16): Fluoroproline
  MOD_RES (17)..(17): Hydroxyproline
  MOD_RES (19)..(19): Fluoroproline
  MOD_RES (20)..(20): Hydroxyproline
PPGPPGMPGPPGPPGPPGPPG

SEQ ID NO: 212 - protein, 21 aa, Artificial Sequence
  Description of Artificial Sequence: Synthetic peptide
  MOD_RES (1)..(1): Fluoroproline
  MOD_RES (2)..(2): Hydroxyproline
  MOD_RES (4)..(4): Fluoroproline
  MOD_RES (5)..(5): Hydroxyproline
  MOD_RES (7)..(7): Fluoroproline
  MOD_RES (10)..(10): Fluoroproline
  MOD_RES (11)..(11): Hydroxyproline
  MOD_RES (13)..(13): Fluoroproline
  MOD_RES (14)..(14): Hydroxyproline
  MOD_RES (16)..(16): Fluoroproline
  MOD_RES (17)..(17): Hydroxyproline
  MOD_RES (19)..(19): Fluoroproline
  MOD_RES (20)..(20): Hydroxyproline
PPGPPGPMGPPGPPGPPGPPG

SEQ ID NO: 213 - protein, 21 aa, Artificial Sequence
  Description of Artificial Sequence: Synthetic peptide
  MOD_RES (1)..(1): Fluoroproline
  MOD_RES (2)..(2): Hydroxyproline
  MOD_RES (4)..(4): Fluoroproline
  MOD_RES (5)..(5): Hydroxyproline
  MOD_RES (7)..(7): Fluoroproline
  MOD_RES (8)..(8): Hydroxyproline
  MOD_RES (11)..(11): Hydroxyproline
  MOD_RES (13)..(13): Fluoroproline
  MOD_RES (14)..(14): Hydroxyproline
  MOD_RES (16)..(16): Fluoroproline
  MOD_RES (17)..(17): Hydroxyproline
  MOD_RES (19)..(19): Fluoroproline
  MOD_RES (20)..(20): Hydroxyproline
PPGPPGPPGMPGPPGPPGPPG

SEQ ID NO: 214 - protein, 21 aa, Artificial Sequence
  Description of Artificial Sequence: Synthetic peptide
  MOD_RES (1)..(1): Fluoroproline
  MOD_RES (2)..(2): Hydroxyproline
  MOD_RES (4)..(4): Fluoroproline
  MOD_RES (5)..(5): Hydroxyproline
  MOD_RES (7)..(7): Fluoroproline
  MOD_RES (8)..(8): Hydroxyproline
  MOD_RES (10)..(10): Fluoroproline
  MOD_RES (13)..(13): Fluoroproline
  MOD_RES (14)..(14): Hydroxyproline
  MOD_RES (16)..(16): Fluoroproline
  MOD_RES (17)..(17): Hydroxyproline
  MOD_RES (19)..(19): Fluoroproline
  MOD_RES (20)..(20): Hydroxyproline
PPGPPGPPGPMGPPGPPGPPG

SEQ ID NO: 215 - protein, 21 aa, Artificial Sequence
  Description of Artificial Sequence: Synthetic peptide
  MOD_RES (1)..(1): Fluoroproline
  MOD_RES (2)..(2): Hydroxyproline
  MOD_RES (4)..(4): Fluoroproline
  MOD_RES (5)..(5): Hydroxyproline
  MOD_RES (7)..(7): Fluoroproline
  MOD_RES (8)..(8): Hydroxyproline
  MOD_RES (10)..(10): Fluoroproline
  MOD_RES (11)..(11): Hydroxyproline
  MOD_RES (14)..(14): Hydroxyproline
  MOD_RES (16)..(16): Fluoroproline
  MOD_RES (17)..(17): Hydroxyproline
  MOD_RES (19)..(19): Fluoroproline
  MOD_RES (20)..(20): Hydroxyproline
PPGPPGPPGPPGMPGPPGPPG

SEQ ID NO: 216 - protein, 21 aa, Artificial Sequence
  Description of Artificial Sequence: Synthetic peptide
  MOD_RES (1)..(1): Fluoroproline
  MOD_RES (2)..(2): Hydroxyproline
  MOD_RES (4)..(4): Fluoroproline
  MOD_RES (5)..(5): Hydroxyproline
  MOD_RES (7)..(7): Fluoroproline
  MOD_RES (8)..(8): Hydroxyproline
  MOD_RES (10)..(10): Fluoroproline
  MOD_RES (11)..(11): Hydroxyproline
  MOD_RES (13)..(13): Fluoroproline
  MOD_RES (16)..(16): Fluoroproline
  MOD_RES (17)..(17): Hydroxyproline
  MOD_RES (19)..(19): Fluoroproline
  MOD_RES (20)..(20): Hydroxyproline
PPGPPGPPGPPGPMGPPGPPG

SEQ ID NO: 217 - protein, 21 aa, Artificial Sequence
  Description of Artificial Sequence: Synthetic peptide
  MOD_RES (1)..(1): Fluoroproline
  MOD_RES (2)..(2): Hydroxyproline
  MOD_RES (4)..(4): Fluoroproline
  MOD_RES (5)..(5): Hydroxyproline
  MOD_RES (7)..(7): Fluoroproline
  MOD_RES (8)..(8): Hydroxyproline
  MOD_RES (10)..(10): Fluoroproline
  MOD_RES (11)..(11): Hydroxyproline
  MOD_RES (13)..(13): Fluoroproline
  MOD_RES (14)..(14): Hydroxyproline
  MOD_RES (17)..(17): Hydroxyproline
  MOD_RES (19)..(19): Fluoroproline
  MOD_RES (20)..(20): Hydroxyproline
PPGPPGPPGPPGPPGMPGPPG

SEQ ID NO: 218 - protein, 21 aa, Artificial Sequence
  Description of Artificial Sequence: Synthetic peptide
  MOD_RES (1)..(1): Fluoroproline
  MOD_RES (2)..(2): Hydroxyproline
  MOD_RES (4)..(4): Fluoroproline
  MOD_RES (5)..(5): Hydroxyproline
  MOD_RES (7)..(7): Fluoroproline
  MOD_RES (8)..(8): Hydroxyproline
  MOD_RES (10)..(10): Fluoroproline
  MOD_RES (11)..(11): Hydroxyproline
  MOD_RES (13)..(13): Fluoroproline
  MOD_RES (14)..(14): Hydroxyproline
  MOD_RES (16)..(16): Fluoroproline
  MOD_RES (19)..(19): Fluoroproline
  MOD_RES (20)..(20): Hydroxyproline
PPGPPGPPGPPGPPGPMGPPG

SEQ ID NO: 219 - protein, 21 aa, Artificial Sequence
  Description of Artificial Sequence: Synthetic peptide
  MOD_RES (1)..(1): Fluoroproline
  MOD_RES (2)..(2): Hydroxyproline
  MOD_RES (4)..(4): Fluoroproline
  MOD_RES (5)..(5): Hydroxyproline
  MOD_RES (7)..(7): Fluoroproline
  MOD_RES (8)..(8): Hydroxyproline
  MOD_RES (10)..(10): Fluoroproline
  MOD_RES (11)..(11): Hydroxyproline
  MOD_RES (13)..(13): Fluoroproline
  MOD_RES (14)..(14): Hydroxyproline
  MOD_RES (16)..(16): Fluoroproline
  MOD_RES (17)..(17): Hydroxyproline
  MOD_RES (20)..(20): Hydroxyproline
PPGPPGPPGPPGPPGPPGMPG

SEQ ID NO: 220 - protein, 21 aa, Artificial Sequence
  Description of Artificial Sequence: Synthetic peptide
  MOD_RES (1)..(1): Fluoroproline
  MOD_RES (2)..(2): Hydroxyproline
  MOD_RES (4)..(4): Fluoroproline
  MOD_RES (5)..(5): Hydroxyproline
  MOD_RES (7)..(7): Fluoroproline
  MOD_RES (8)..(8): Hydroxyproline
  MOD_RES (10)..(10): Fluoroproline
  MOD_RES (11)..(11): Hydroxyproline
  MOD_RES (13)..(13): Fluoroproline
  MOD_RES (14)..(14): Hydroxyproline
  MOD_RES (16)..(16): Fluoroproline
  MOD_RES (17)..(17): Hydroxyproline
  MOD_RES (19)..(19): Fluoroproline
PPGPPGPPGPPGPPGPPGPMG

SEQ ID NO: 221 - protein, 21 aa, Artificial Sequence
  Description of Artificial Sequence: Synthetic peptide
  MOD_RES (2)..(2): Chloroproline
  MOD_RES (5)..(5): Chloroproline
  MOD_RES (8)..(8): Chloroproline
  MOD_RES (11)..(11): Chloroproline
  MOD_RES (14)..(14): Chloroproline
  MOD_RES (17)..(17): Chloroproline
  MOD_RES (20)..(20): Chloroproline
MPGPPGPPGPPGPPGPPGPPG

SEQ ID NO: 222 - protein, 21 aa, Artificial Sequence
  Description of Artificial Sequence: Synthetic peptide
  MOD_RES (5)..(5): Chloroproline
  MOD_RES (8)..(8): Chloroproline
  MOD_RES (11)..(11): Chloroproline
  MOD_RES (14)..(14): Chloroproline
  MOD_RES (17)..(17): Chloroproline
  MOD_RES (20)..(20): Chloroproline
PMGPPGPPGPPGPPGPPGPPG

SEQ ID NO: 223 - protein, 21 aa, Artificial Sequence
  Description of Artificial Sequence: Synthetic peptide
  MOD_RES (2)..(2): Chloroproline
  MOD_RES (5)..(5): Chloroproline
  MOD_RES (8)..(8): Chloroproline
  MOD_RES (11)..(11): Chloroproline
  MOD_RES (14)..(14): Chloroproline
  MOD_RES (17)..(17): Chloroproline
  MOD_RES (20)..(20): Chloroproline
PPGMPGPPGPPGPPGPPGPPG

SEQ ID NO: 224 - protein, 21 aa, Artificial Sequence
  Description of Artificial Sequence: Synthetic peptide
  MOD_RES (2)..(2): Chloroproline
  MOD_RES (8)..(8): Chloroproline
  MOD_RES (11)..(11): Chloroproline
  MOD_RES (14)..(14): Chloroproline
  MOD_RES (17)..(17): Chloroproline
  MOD_RES (20)..(20): Chloroproline
PPGPMGPPGPPGPPGPPGPPG

SEQ ID NO: 225 - protein, 21 aa, Artificial Sequence
  Description of Artificial Sequence: Synthetic peptide
  MOD_RES (2)..(2): Chloroproline
  MOD_RES (5)..(5): Chloroproline
  MOD_RES (8)..(8): Chloroproline
  MOD_RES (11)..(11): Chloroproline
  MOD_RES (14)..(14): Chloroproline
  MOD_RES (17)..(17): Chloroproline
  MOD_RES (20)..(20): Chloroproline
PPGPPGMPGPPGPPGPPGPPG

SEQ ID NO: 226 - protein, 21 aa, Artificial Sequence
  Description of Artificial Sequence: Synthetic peptide
  MOD_RES (2)..(2): Chloroproline
  MOD_RES (5)..(5): Chloroproline
  MOD_RES (8)..(8): Chloroproline
  MOD_RES (11)..(11): Chloroproline
  MOD_RES (14)..(14): Chloroproline
  MOD_RES (17)..(17): Chloroproline
  MOD_RES (20)..(20): Chloroproline
PPGPPGPPGMPGPPGPPGPPG

SEQ ID NO: 227 - protein, 21 aa, Artificial Sequence
  Description of Artificial Sequence: Synthetic peptide
  MOD_RES (2)..(2): Chloroproline
  MOD_RES (5)..(5): Chloroproline
  MOD_RES (8)..(8): Chloroproline
  MOD_RES (14)..(14): Chloroproline
  MOD_RES (17)..(17): Chloroproline
  MOD_RES (20)..(20): Chloroproline
PPGPPGPPGPMGPPGPPGPPG

SEQ ID NO: 228 - protein, 21 aa, Artificial Sequence
  Description of Artificial Sequence: Synthetic peptide
  MOD_RES (2)..(2): Chloroproline
  MOD_RES (5)..(5): Chloroproline
  MOD_RES (8)..(8): Chloroproline
  MOD_RES (11)..(11): Chloroproline
  MOD_RES (14)..(14): Chloroproline
  MOD_RES (17)..(17): Chloroproline
  MOD_RES (20)..(20): Chloroproline
PPGPPGPPGPPGMPGPPGPPG

SEQ ID NO: 229 - protein, 21 aa, Artificial Sequence
  Description of Artificial Sequence: Synthetic peptide
  MOD_RES (2)..(2): Chloroproline
  MOD_RES (5)..(5): Chloroproline
  MOD_RES (8)..(8): Chloroproline
  MOD_RES (11)..(11): Chloroproline
  MOD_RES (17)..(17): Chloroproline
  MOD_RES (20)..(20): Chloroproline
PPGPPGPPGPPGPMGPPGPPG

SEQ ID NO: 230 - protein, 21 aa, Artificial Sequence
  Description of Artificial Sequence: Synthetic peptide
  MOD_RES (2)..(2): Chloroproline
  MOD_RES (5)..(5): Chloroproline
  MOD_RES (8)..(8): Chloroproline
  MOD_RES (11)..(11): Chloroproline
  MOD_RES (14)..(14): Chloroproline
  MOD_RES (17)..(17): Chloroproline
  MOD_RES (20)..(20): Chloroproline
PPGPPGPPGPPGPPGMPGPPG

SEQ ID NO: 231 - protein, 21 aa, Artificial Sequence
  Description of Artificial Sequence: Synthetic peptide
  MOD_RES (2)..(2): Chloroproline
  MOD_RES (5)..(5): Chloroproline
  MOD_RES (8)..(8): Chloroproline
  MOD_RES (11)..(11): Chloroproline
  MOD_RES (14)..(14): Chloroproline
  MOD_RES (20)..(20): Chloroproline
PPGPPGPPGPPGPPGPMGPPG

SEQ ID NO: 232 - protein, 21 aa, Artificial Sequence
  Description of Artificial Sequence: Synthetic peptide
  MOD_RES (2)..(2): Chloroproline
  MOD_RES (5)..(5): Chloroproline
  MOD_RES (8)..(8): Chloroproline
  MOD_RES (11)..(11): Chloroproline
  MOD_RES (14)..(14): Chloroproline
  MOD_RES (17)..(17): Chloroproline
  MOD_RES (20)..(20): Chloroproline
PPGPPGPPGPPGPPGPPGMPG

SEQ ID NO: 233 - protein, 21 aa, Artificial Sequence
  Description of Artificial Sequence: Synthetic peptide
  MOD_RES (2)..(2): Chloroproline
  MOD_RES (5)..(5): Chloroproline
  MOD_RES (8)..(8): Chloroproline
  MOD_RES (11)..(11): Chloroproline
  MOD_RES (14)..(14): Chloroproline
  MOD_RES (17)..(17): Chloroproline
PPGPPGPPGPPGPPGPPGPMG

SEQ ID NO: 234 - protein, 21 aa, Artificial Sequence
  Description of Artificial Sequence: Synthetic peptide
  MOD_RES (2)..(2): Chloroproline
  MOD_RES (5)..(5): Chloroproline
  MOD_RES (8)..(8): Chloroproline
  MOD_RES (11)..(11): Chloroproline
  MOD_RES (14)..(14): Chloroproline
  MOD_RES (17)..(17): Chloroproline
  MOD_RES (20)..(20): Chloroproline
MPGPPGPPGPPGPPGPPGPPG

SEQ ID NO: 235 - protein, 21 aa, Artificial Sequence
  Description of Artificial Sequence: Synthetic peptide
  MOD_RES (5)..(5): Chloroproline
  MOD_RES (8)..(8): Chloroproline
  MOD_RES (11)..(11): Chloroproline
  MOD_RES (14)..(14): Chloroproline
  MOD_RES (17)..(17): Chloroproline
  MOD_RES (20)..(20): Chloroproline
PMGPPGPPGPPGPPGPPGPPG

SEQ ID NO: 236 - protein, 21 aa, Artificial Sequence
  Description of Artificial Sequence: Synthetic peptide
  MOD_RES (2)..(2): Chloroproline
  MOD_RES (5)..(5): Chloroproline
  MOD_RES (8)..(8): Chloroproline
  MOD_RES (11)..(11): Chloroproline
  MOD_RES (14)..(14): Chloroproline
  MOD_RES (17)..(17): Chloroproline
  MOD_RES (20)..(20): Chloroproline
PPGMPGPPGPPGPPGPPGPPG

SEQ ID NO: 237 - protein, 21 aa, Artificial Sequence
  Description of Artificial Sequence: Synthetic peptide
  MOD_RES (2)..(2): Chloroproline
  MOD_RES (8)..(8): Chloroproline
  MOD_RES (11)..(11): Chloroproline
  MOD_RES (14)..(14): Chloroproline
  MOD_RES (17)..(17): Chloroproline
  MOD_RES (20)..(20): Chloroproline
PPGPMGPPGPPGPPGPPGPPG

SEQ ID NO: 238 - protein, 21 aa, Artificial Sequence
  Description of Artificial Sequence: Synthetic peptide
  MOD_RES (2)..(2): Chloroproline
  MOD_RES (5)..(5): Chloroproline
  MOD_RES (8)..(8): Chloroproline
  MOD_RES (11)..(11): Chloroproline
  MOD_RES (14)..(14): Chloroproline
  MOD_RES (17)..(17): Chloroproline
  MOD_RES (20)..(20): Chloroproline
PPGPPGMPGPPGPPGPPGPPG

SEQ ID NO: 239 - protein, 21 aa, Artificial Sequence
  Description of Artificial Sequence: Synthetic peptide
  MOD_RES (2)..(2): Chloroproline
  MOD_RES (5)..(5): Chloroproline
  MOD_RES (11)..(11): Chloroproline
  MOD_RES (14)..(14): Chloroproline
  MOD_RES (17)..(17): Chloroproline
  MOD_RES (20)..(20): Chloroproline
PPGPPGPMGPPGPPGPPGPPG

SEQ ID NO: 240 - protein, 21 aa, Artificial Sequence
  Description of Artificial Sequence: Synthetic peptide
  MOD_RES (2)..(2): Chloroproline
  MOD_RES (5)..(5): Chloroproline
  MOD_RES (8)..(8): Chloroproline
  MOD_RES (11)..(11): Chloroproline
  MOD_RES (14)..(14): Chloroproline
  MOD_RES (17)..(17): Chloroproline
  MOD_RES (20)..(20): Chloroproline
PPGPPGPPGMPGPPGPPGPPG

SEQ ID NO: 241 - protein, 21 aa, Artificial Sequence
  Description of Artificial Sequence: Synthetic peptide
  MOD_RES (2)..(2): Chloroproline
  MOD_RES (5)..(5): Chloroproline
  MOD_RES (8)..(8): Chloroproline
  MOD_RES (14)..(14): Chloroproline
  MOD_RES (17)..(17): Chloroproline
  MOD_RES (20)..(20): Chloroproline
PPGPPGPPGPMGPPGPPGPPG

SEQ ID NO: 242 - protein, 21 aa, Artificial Sequence
  Description of Artificial Sequence: Synthetic peptide
  MOD_RES (2)..(2): Chloroproline
  MOD_RES (5)..(5): Chloroproline
  MOD_RES (8)..(8): Chloroproline
  MOD_RES (11)..(11): Chloroproline
  MOD_RES (14)..(14): Chloroproline
  MOD_RES (17)..(17): Chloroproline
  MOD_RES (20)..(20): Chloroproline
PPGPPGPPGPPGMPGPPGPPG

SEQ ID NO: 243 - protein, 21 aa, Artificial Sequence
  Description of Artificial Sequence: Synthetic peptide
  MOD_RES (2)..(2): Chloroproline
  MOD_RES (5)..(5): Chloroproline
  MOD_RES (8)..(8): Chloroproline
  MOD_RES (11)..(11): Chloroproline
  MOD_RES (17)..(17): Chloroproline
  MOD_RES (20)..(20): Chloroproline
PPGPPGPPGPPGPMGPPGPPG

SEQ ID NO: 244 - protein, 21 aa, Artificial Sequence
  Description of Artificial Sequence: Synthetic peptide
  MOD_RES (2)..(2): Chloroproline
  MOD_RES (5)..(5): Chloroproline
  MOD_RES (8)..(8): Chloroproline
  MOD_RES (11)..(11): Chloroproline
  MOD_RES (14)..(14): Chloroproline
  MOD_RES (17)..(17): Chloroproline
  MOD_RES (20)..(20): Chloroproline
PPGPPGPPGPPGPPGMPGPPG

SEQ ID NO: 245 - protein, 21 aa, Artificial Sequence
  Description of Artificial Sequence: Synthetic peptide
  MOD_RES (2)..(2): Chloroproline
  MOD_RES (5)..(5): Chloroproline
  MOD_RES (8)..(8): Chloroproline
  MOD_RES (11)..(11): Chloroproline
  MOD_RES (14)..(14): Chloroproline
  MOD_RES (20)..(20): Chloroproline
PPGPPGPPGPPGPPGPMGPPG

SEQ ID NO: 246 - protein, 21 aa, Artificial Sequence
  Description of Artificial Sequence: Synthetic peptide
  MOD_RES (2)..(2): Chloroproline
  MOD_RES (5)..(5): Chloroproline
  MOD_RES (8)..(8): Chloroproline
  MOD_RES (11)..(11): Chloroproline
  MOD_RES (14)..(14): Chloroproline
  MOD_RES (17)..(17): Chloroproline
  MOD_RES (20)..(20): Chloroproline
PPGPPGPPGPPGPPGPPGMPG

SEQ ID NO: 247 - protein, 21 aa, Artificial Sequence
  Description of Artificial Sequence: Synthetic peptide
  MOD_RES (2)..(2): Chloroproline
  MOD_RES (5)..(5): Chloroproline
  MOD_RES (8)..(8): Chloroproline
  MOD_RES (11)..(11): Chloroproline
  MOD_RES (14)..(14): Chloroproline
  MOD_RES (17)..(17): Chloroproline
PPGPPGPPGPPGPPGPPGPMG

SEQ ID NO: 248 - protein, 21 aa, Artificial Sequence
  Description of Artificial Sequence: Synthetic peptide
  MOD_RES (2)..(2): Hydroxyproline
  MOD_RES (4)..(4): Chloroproline
  MOD_RES (5)..(5): Hydroxyproline
  MOD_RES (7)..(7): Chloroproline
  MOD_RES (8)..(8): Hydroxyproline
  MOD_RES (10)..(10): Chloroproline
  MOD_RES (11)..(11): Hydroxyproline
  MOD_RES (13)..(13): Chloroproline
  MOD_RES (14)..(14): Hydroxyproline
  MOD_RES (16)..(16): Chloroproline
  MOD_RES (17)..(17): Hydroxyproline
  MOD_RES (19)..(19): Chloroproline
  MOD_RES (20)..(20): Hydroxyproline
MPGPPGPPGPPGPPGPPGPPG

SEQ ID NO: 249 - protein, 21 aa, Artificial Sequence
  Description of Artificial Sequence: Synthetic peptide
  MOD_RES (1)..(1): Chloroproline
  MOD_RES (4)..(4): Chloroproline
  MOD_RES (5)..(5): Hydroxyproline
  MOD_RES (7)..(7): Chloroproline
  MOD_RES (8)..(8): Hydroxyproline
  MOD_RES (10)..(10): Chloroproline
  MOD_RES (11)..(11): Hydroxyproline
  MOD_RES (13)..(13): Chloroproline
  MOD_RES (14)..(14): Hydroxyproline
  MOD_RES (16)..(16): Chloroproline
  MOD_RES (17)..(17): Hydroxyproline
  MOD_RES (19)..(19): Chloroproline
  MOD_RES (20)..(20): Hydroxyproline
PMGPPGPPGPPGPPGPPGPPG

SEQ ID NO: 250 - protein, 21 aa, Artificial Sequence
  Description of Artificial Sequence: Synthetic peptide
  MOD_RES (1)..(1): Chloroproline
  MOD_RES (2)..(2): Hydroxyproline
  MOD_RES (5)..(5): Hydroxyproline
  MOD_RES (7)..(7): Chloroproline
  MOD_RES (8)..(8): Hydroxyproline
  MOD_RES (10)..(10): Chloroproline
  MOD_RES (11)..(11): Hydroxyproline
  MOD_RES (13)..(13): Chloroproline
  MOD_RES (14)..(14): Hydroxyproline
  MOD_RES (16)..(16): Chloroproline
  MOD_RES (17)..(17): Hydroxyproline
  MOD_RES (19)..(19): Chloroproline
  MOD_RES (20)..(20): Hydroxyproline
PPGMPGPPGPPGPPGPPGPPG

SEQ ID NO: 251 - protein, 21 aa, Artificial Sequence
  Description of Artificial Sequence: Synthetic peptide
  MOD_RES (1)..(1): Chloroproline
  MOD_RES (2)..(2): Hydroxyproline
  MOD_RES (4)..(4): Chloroproline
  MOD_RES (7)..(7): Chloroproline
  MOD_RES (8)..(8): Hydroxyproline
  MOD_RES (10)..(10): Chloroproline
  MOD_RES (11)..(11): Hydroxyproline
  MOD_RES (13)..(13): Chloroproline
  MOD_RES (14)..(14): Hydroxyproline
  MOD_RES (16)..(16): Chloroproline
  MOD_RES (17)..(17): Hydroxyproline
  MOD_RES (19)..(19): Chloroproline
  MOD_RES (20)..(20): Hydroxyproline
PPGPMGPPGPPGPPGPPGPPG

SEQ ID NO: 252 - protein, 21 aa, Artificial Sequence
  Description of Artificial Sequence: Synthetic peptide
  MOD_RES (1)..(1): Chloroproline
  MOD_RES (2)..(2): Hydroxyproline
  MOD_RES (4)..(4): Chloroproline
  MOD_RES (5)..(5): Hydroxyproline
  MOD_RES (8)..(8): Hydroxyproline
  MOD_RES (10)..(10): Chloroproline
  MOD_RES (11)..(11): Hydroxyproline
  MOD_RES (13)..(13): Chloroproline
  MOD_RES (14)..(14): Hydroxyproline
  MOD_RES (16)..(16): Chloroproline
  MOD_RES (17)..(17): Hydroxyproline
  MOD_RES (19)..(19): Chloroproline
  MOD_RES (20)..(20): Hydroxyproline
PPGPPGMPGPPGPPGPPGPPG

SEQ ID NO: 253 - protein, 21 aa, Artificial Sequence
  Description of Artificial Sequence: Synthetic peptide
  MOD_RES (1)..(1): Chloroproline
  MOD_RES (2)..(2): Hydroxyproline
  MOD_RES (4)..(4): Chloroproline
  MOD_RES (5)..(5): Hydroxyproline
  MOD_RES (7)..(7): Chloroproline
  MOD_RES (10)..(10): Chloroproline
  MOD_RES (11)..(11): Hydroxyproline
  MOD_RES (13)..(13): Chloroproline
  MOD_RES (14)..(14): Hydroxyproline
  MOD_RES (16)..(16): Chloroproline
  MOD_RES (17)..(17): Hydroxyproline
  MOD_RES (19)..(19): Chloroproline
  MOD_RES (20)..(20): Hydroxyproline
PPGPPGPMGPPGPPGPPGPPG

SEQ ID NO: 254 - protein, 21 aa, Artificial Sequence
  Description of Artificial Sequence: Synthetic peptide
  MOD_RES (1)..(1): Chloroproline
  MOD_RES (2)..(2): Hydroxyproline
  MOD_RES (4)..(4): Chloroproline
  MOD_RES (5)..(5): Hydroxyproline
  MOD_RES (7)..(7): Chloroproline
  MOD_RES (8)..(8): Hydroxyproline
  MOD_RES (11)..(11): Hydroxyproline
  MOD_RES (13)..(13): Chloroproline
  MOD_RES (14)..(14): Hydroxyproline
  MOD_RES (16)..(16): Chloroproline
  MOD_RES (17)..(17): Hydroxyproline
  MOD_RES (19)..(19): Chloroproline
  MOD_RES (20)..(20): Hydroxyproline
PPGPPGPPGMPGPPGPPGPPG

SEQ ID NO: 255 - protein, 21 aa, Artificial Sequence
  Description of Artificial Sequence: Synthetic peptide
  MOD_RES (1)..(1): Chloroproline
  MOD_RES (2)..(2): Hydroxyproline
  MOD_RES (4)..(4): Chloroproline
  MOD_RES (5)..(5): Hydroxyproline
  MOD_RES (7)..(7): Chloroproline
  MOD_RES (8)..(8): Hydroxyproline
  MOD_RES (10)..(10): Chloroproline
  MOD_RES (13)..(13): Chloroproline
  MOD_RES (14)..(14): Hydroxyproline
  MOD_RES (16)..(16): Chloroproline
  MOD_RES (17)..(17): Hydroxyproline
  MOD_RES (19)..(19): Chloroproline
  MOD_RES (20)..(20): Hydroxyproline
PPGPPGPPGPMGPPGPPGPPG

SEQ ID NO: 256 - protein, 21 aa, Artificial Sequence
  Description of Artificial Sequence: Synthetic peptide
  MOD_RES (1)..(1): Chloroproline
  MOD_RES (2)..(2): Hydroxyproline
  MOD_RES (4)..(4): Chloroproline
  MOD_RES (5)..(5): Hydroxyproline
  MOD_RES (7)..(7): Chloroproline
  MOD_RES (8)..(8): Hydroxyproline
  MOD_RES (10)..(10): Chloroproline
  MOD_RES (11)..(11): Hydroxyproline
  MOD_RES (14)..(14): Hydroxyproline
  MOD_RES (16)..(16): Chloroproline
  MOD_RES (17)..(17): Hydroxyproline
  MOD_RES (19)..(19): Chloroproline
  MOD_RES (20)..(20): Hydroxyproline
PPGPPGPPGPPGMPGPPGPPG

SEQ ID NO: 257 - protein, 21 aa, Artificial Sequence
  Description of Artificial Sequence: Synthetic peptide
  MOD_RES (1)..(1): Chloroproline
  MOD_RES (2)..(2): Hydroxyproline
  MOD_RES (4)..(4): Chloroproline
  MOD_RES (5)..(5): Hydroxyproline
  MOD_RES (7)..(7): Chloroproline
  MOD_RES (8)..(8): Hydroxyproline
  MOD_RES (10)..(10): Chloroproline
  MOD_RES (11)..(11): Hydroxyproline
  MOD_RES (13)..(13): Chloroproline
  MOD_RES (16)..(16): Chloroproline
  MOD_RES (17)..(17): Hydroxyproline
  MOD_RES (19)..(19): Chloroproline
  MOD_RES (20)..(20): Hydroxyproline
PPGPPGPPGPPGPMGPPGPPG

SEQ ID NO: 258 - protein, 21 aa, Artificial Sequence
  Description of Artificial Sequence: Synthetic peptide
  MOD_RES (1)..(1): Chloroproline
  MOD_RES (2)..(2): Hydroxyproline
  MOD_RES (4)..(4): Chloroproline
  MOD_RES (5)..(5): Hydroxyproline
  MOD_RES (7)..(7): Chloroproline
  MOD_RES (8)..(8): Hydroxyproline
  MOD_RES (10)..(10): Chloroproline
  MOD_RES (11)..(11): Hydroxyproline
  MOD_RES (13)..(13): Chloroproline
  MOD_RES (14)..(14): Hydroxyproline
  MOD_RES (17)..(17): Hydroxyproline
  MOD_RES (19)..(19): Chloroproline
  MOD_RES (20)..(20): Hydroxyproline
PPGPPGPPGPPGPPGMPGPPG

SEQ ID NO: 259 - protein, 21 aa, Artificial Sequence
  Description of Artificial Sequence: Synthetic peptide
  MOD_RES (1)..(1): Chloroproline
  MOD_RES (2)..(2): Hydroxyproline
  MOD_RES (4)..(4): Chloroproline
  MOD_RES (5)..(5): Hydroxyproline
  MOD_RES (7)..(7): Chloroproline
  MOD_RES (8)..(8): Hydroxyproline
  MOD_RES (10)..(10): Chloroproline
  MOD_RES (11)..(11): Hydroxyproline
  MOD_RES (13)..(13): Chloroproline
  MOD_RES (14)..(14): Hydroxyproline
  MOD_RES (16)..(16): Chloroproline
  MOD_RES (19)..(19): Chloroproline
  MOD_RES (20)..(20): Hydroxyproline
PPGPPGPPGPPGPPGPMGPPG

SEQ ID NO: 260 - protein, 21 aa, Artificial Sequence
  Description of Artificial Sequence: Synthetic peptide
  MOD_RES (1)..(1): Chloroproline
  MOD_RES (2)..(2): Hydroxyproline
  MOD_RES (4)..(4): Chloroproline
  MOD_RES (5)..(5): Hydroxyproline
  MOD_RES (7)..(7): Chloroproline
  MOD_RES (8)..(8): Hydroxyproline
  MOD_RES (10)..(10): Chloroproline
  MOD_RES (11)..(11): Hydroxyproline
  MOD_RES (13)..(13): Chloroproline
  MOD_RES (14)..(14): Hydroxyproline
  MOD_RES (16)..(16): Chloroproline
  MOD_RES (17)..(17): Hydroxyproline
  MOD_RES (20)..(20): Hydroxyproline
PPGPPGPPGPPGPPGPPGMPG

SEQ ID NO: 261 - protein, 21 aa, Artificial Sequence
  Description of Artificial Sequence: Synthetic peptide
  MOD_RES (1)..(1): Chloroproline
  MOD_RES (2)..(2): Hydroxyproline
  MOD_RES (4)..(4): Chloroproline
  MOD_RES (5)..(5): Hydroxyproline
  MOD_RES (7)..(7): Chloroproline
  MOD_RES (8)..(8): Hydroxyproline
  MOD_RES (10)..(10): Chloroproline
  MOD_RES (11)..(11): Hydroxyproline
  MOD_RES (13)..(13): Chloroproline
  MOD_RES (14)..(14): Hydroxyproline
  MOD_RES (16)..(16): Chloroproline
  MOD_RES (17)..(17): Hydroxyproline
  MOD_RES (19)..(19): Chloroproline
PPGPPGPPGPPGPPGPPGPMG

SEQ ID NO: 262 - protein, 21 aa, Artificial Sequence
  Description of Artificial Sequence: Synthetic peptide
PPGPPGKPGPPGPPGPPGPPG

SEQ ID NO: 263 - protein, 21 aa, Artificial Sequence
  Description of Artificial Sequence: Synthetic peptide
  MOD_RES (1)..(1): Hydroxyproline
  MOD_RES (4)..(4): Hydroxyproline
  MOD_RES (10)..(10): Hydroxyproline
  MOD_RES (13)..(13): Hydroxyproline
  MOD_RES (16)..(16): Hydroxyproline
  MOD_RES (19)..(19): Hydroxyproline
PPGPPGKPGPPGPPGPPGPPG

SEQ ID NO: 264 - protein, 21 aa, Artificial Sequence
  Description of Artificial Sequence: Synthetic peptide
  MOD_RES (2)..(2): Hydroxyproline
  MOD_RES (5)..(5): Hydroxyproline
  MOD_RES (11)..(11): Hydroxyproline
  MOD_RES (14)..(14): Hydroxyproline
  MOD_RES (17)..(17): Hydroxyproline
  MOD_RES (20)..(20): Hydroxyproline
PPGPPGPKGPPGPPGPPGPPG

SEQ ID NO: 265 - protein, 21 aa, Artificial Sequence
  Description of Artificial Sequence: Synthetic peptide
  MOD_RES (2)..(2): Fluoroproline
  MOD_RES (5)..(5): Fluoroproline
  MOD_RES (11)..(11): Fluoroproline
  MOD_RES (14)..(14): Fluoroproline
  MOD_RES (17)..(17): Fluoroproline
  MOD_RES (20)..(20): Fluoroproline
PPGPPGPKGPPGPPGPPGPPG

SEQ ID NO: 266 - protein, 21 aa, Artificial Sequence
  Description of Artificial Sequence: Synthetic peptide
  MOD_RES (2)..(2): Chloroproline
  MOD_RES (5)..(5): Chloroproline
  MOD_RES (11)..(11): Chloroproline
  MOD_RES (14)..(14): Chloroproline
  MOD_RES (17)..(17): Chloroproline
  MOD_RES (20)..(20): Chloroproline
PPGPPGPKGPPGPPGPPGPPG

SEQ ID NO: 267 - protein, 21 aa, Artificial Sequence
  Description of Artificial Sequence: Synthetic peptide
KPGPPGPPGPPGPPGPPGPPG

SEQ ID NO: 268 - protein, 21 aa, Artificial Sequence
  Description of Artificial Sequence: Synthetic peptide
PKGPPGPPGPPGPPGPPGPPG

SEQ ID NO: 269 - protein, 21 aa, Artificial Sequence
  Description of Artificial Sequence: Synthetic peptide
PPGKPGPPGPPGPPGPPGPPG

SEQ ID NO: 270 - protein, 21 aa, Artificial Sequence
  Description of Artificial Sequence: Synthetic peptide
PPGPKGPPGPPGPPGPPGPPG

SEQ ID NO: 271 - protein, 21 aa, Artificial Sequence
  Description of Artificial Sequence: Synthetic peptide
PPGPPGPKGPPGPPGPPGPPG

SEQ ID NO: 272 - protein, 21 aa, Artificial Sequence
  Description of Artificial Sequence: Synthetic peptide
PPGPPGPPGKPGPPGPPGPPG

SEQ ID NO: 273 - protein, 21 aa, Artificial Sequence
  Description of Artificial Sequence: Synthetic peptide
PPGPPGPPGPKGPPGPPGPPG

SEQ ID NO: 274 - protein, 21 aa, Artificial Sequence
  Description of Artificial Sequence: Synthetic peptide
PPGPPGPPGPPGKPGPPGPPG

SEQ ID NO: 275 - protein, 21 aa, Artificial Sequence
  Description of Artificial Sequence: Synthetic peptide
PPGPPGPPGPPGPKGPPGPPG

SEQ ID NO: 276 - protein, 21 aa, Artificial Sequence
  Description of Artificial Sequence: Synthetic peptide
PPGPPGPPGPPGPPGKPGPPG

SEQ ID NO: 277 - protein, 21 aa, Artificial Sequence
  Description of Artificial Sequence: Synthetic peptide
PPGPPGPPGPPGPPGPKGPPG

SEQ ID NO: 278 - protein, 21 aa, Artificial Sequence
  Description of Artificial Sequence: Synthetic peptide
PPGPPGPPGPPGPPGPPGKPG

SEQ ID NO: 279 - protein, 21 aa, Artificial Sequence
  Description of Artificial Sequence: Synthetic peptide
PPGPPGPPGPPGPPGPPGPKG

SEQ ID NO: 280 - protein, 21 aa, Artificial Sequence
  Description of Artificial Sequence: Synthetic peptide
  MOD_RES (4)..(4): Hydroxyproline
  MOD_RES (7)..(7): Hydroxyproline
  MOD_RES (10)..(10): Hydroxyproline
  MOD_RES (13)..(13): Hydroxyproline
  MOD_RES (16)..(16): Hydroxyproline
  MOD_RES (19)..(19): Hydroxyproline
KPGPPGPPGPPGPPGPPGPPG

SEQ ID NO: 281 - protein, 21 aa, Artificial Sequence
  Description of Artificial Sequence: Synthetic peptide
  MOD_RES (1)..(1): Hydroxyproline
  MOD_RES (4)..(4): Hydroxyproline
  MOD_RES (7)..(7): Hydroxyproline
  MOD_RES (10)..(10): Hydroxyproline
  MOD_RES (13)..(13): Hydroxyproline
  MOD_RES (16)..(16): Hydroxyproline
  MOD_RES (19)..(19): Hydroxyproline
PKGPPGPPGPPGPPGPPGPPG

SEQ ID NO: 282 - protein, 21 aa, Artificial Sequence
  Description of Artificial Sequence: Synthetic peptide
  MOD_RES (1)..(1): Hydroxyproline
  MOD_RES (7)..(7): Hydroxyproline
  MOD_RES (10)..(10): Hydroxyproline
  MOD_RES (13)..(13): Hydroxyproline
  MOD_RES (16)..(16): Hydroxyproline
  MOD_RES (19)..(19): Hydroxyproline
PPGKPGPPGPPGPPGPPGPPG

SEQ ID NO: 283 - protein, 21 aa, Artificial Sequence
  Description of Artificial Sequence: Synthetic peptide
  MOD_RES (1)..(1): Hydroxyproline
  MOD_RES (4)..(4): Hydroxyproline
  MOD_RES (7)..(7): Hydroxyproline
  MOD_RES (10)..(10): Hydroxyproline
  MOD_RES (13)..(13): Hydroxyproline
  MOD_RES (16)..(16): Hydroxyproline
  MOD_RES (19)..(19): Hydroxyproline
PPGPKGPPGPPGPPGPPGPPG

SEQ ID NO: 284 - protein, 21 aa, Artificial Sequence
  Description of Artificial Sequence: Synthetic peptide
  MOD_RES (1)..(1): Hydroxyproline
  MOD_RES (4)..(4): Hydroxyproline
  MOD_RES (7)..(7): Hydroxyproline
  MOD_RES (10)..(10): Hydroxyproline
  MOD_RES (13)..(13): Hydroxyproline
  MOD_RES (16)..(16): Hydroxyproline
  MOD_RES (19)..(19): Hydroxyproline
PPGPPGPKGPPGPPGPPGPPG

SEQ ID NO: 285 - protein, 21 aa, Artificial Sequence
  Description of Artificial Sequence: Synthetic peptide
  MOD_RES (1)..(1): Hydroxyproline
  MOD_RES (4)..(4): Hydroxyproline
  MOD_RES (7)..(7): Hydroxyproline
  MOD_RES (13)..(13): Hydroxyproline
  MOD_RES (16)..(16): Hydroxyproline
  MOD_RES (19)..(19): Hydroxyproline
PPGPPGPPGKPGPPGPPGPPG

SEQ ID NO: 286 - protein, 21 aa, Artificial Sequence
  Description of Artificial Sequence: Synthetic peptide
  MOD_RES (1)..(1): Hydroxyproline
  MOD_RES (4)..(4): Hydroxyproline
  MOD_RES (7)..(7): Hydroxyproline
  MOD_RES (10)..(10): Hydroxyproline
  MOD_RES (13)..(13): Hydroxyproline
  MOD_RES (16)..(16): Hydroxyproline
  MOD_RES (19)..(19): Hydroxyproline
PPGPPGPPGPKGPPGPPGPPG

SEQ ID NO: 287 - protein, 21 aa, Artificial Sequence
  Description of Artificial Sequence: Synthetic peptide
  MOD_RES (1)..(1): Hydroxyproline
  MOD_RES (4)..(4): Hydroxyproline
  MOD_RES (7)..(7): Hydroxyproline
  MOD_RES (10)..(10): Hydroxyproline
  MOD_RES (16)..(16): Hydroxyproline
  MOD_RES (19)..(19): Hydroxyproline
PPGPPGPPGPPGKPGPPGPPG

SEQ ID NO: 288 - protein, 21 aa, Artificial Sequence
  Description of Artificial Sequence: Synthetic peptide
  MOD_RES (1)..(1): Hydroxyproline
  MOD_RES (4)..(4): Hydroxyproline
  MOD_RES (7)..(7): Hydroxyproline
  MOD_RES (10)..(10): Hydroxyproline
  MOD_RES (13)..(13): Hydroxyproline
  MOD_RES (16)..(16): Hydroxyproline
  MOD_RES (19)..(19): Hydroxyproline
PPGPPGPPGPPGPKGPPGPPG

SEQ ID NO: 289 - protein, 21 aa, Artificial Sequence
  Description of Artificial Sequence: Synthetic peptide
  MOD_RES (1)..(1): Hydroxyproline
  MOD_RES (4)..(4): Hydroxyproline
  MOD_RES (7)..(7): Hydroxyproline
  MOD_RES (10)..(10): Hydroxyproline
  MOD_RES (13)..(13): Hydroxyproline
  MOD_RES (19)..(19): Hydroxyproline
PPGPPGPPGPPGPPGKPGPPG

SEQ ID NO: 290 - protein, 21 aa, Artificial Sequence
  Description of Artificial Sequence: Synthetic peptide
  MOD_RES (1)..(1): Hydroxyproline
  MOD_RES (4)..(4): Hydroxyproline
  MOD_RES (7)..(7): Hydroxyproline
  MOD_RES (10)..(10): Hydroxyproline
  MOD_RES (13)..(13): Hydroxyproline
  MOD_RES (16)..(16): Hydroxyproline
  MOD_RES (19)..(19): Hydroxyproline
PPGPPGPPGPPGPPGPKGPPG

SEQ ID NO: 291 - protein, 21 aa, Artificial Sequence
  Description of Artificial Sequence: Synthetic peptide
  MOD_RES (1)..(1): Hydroxyproline
  MOD_RES (4)..(4): Hydroxyproline
  MOD_RES (7)..(7): Hydroxyproline
  MOD_RES (10)..(10): Hydroxyproline
  MOD_RES (13)..(13): Hydroxyproline
  MOD_RES (16)..(16): Hydroxyproline
PPGPPGPPGPPGPPGPPGKPG

SEQ ID NO: 292 - protein, 21 aa, Artificial Sequence
  Description of Artificial Sequence: Synthetic peptide
  MOD_RES (1)..(1): Hydroxyproline
  MOD_RES (4)..(4): Hydroxyproline
  MOD_RES (7)..(7): Hydroxyproline
  MOD_RES (10)..(10): Hydroxyproline
  MOD_RES (13)..(13): Hydroxyproline
  MOD_RES (16)..(16): Hydroxyproline
  MOD_RES (19)..(19): Hydroxyproline
PPGPPGPPGPPGPPGPPGPKG

SEQ ID NO: 293 - protein, 21 aa, Artificial Sequence
  Description of Artificial Sequence: Synthetic peptide
  MOD_RES (2)..(2): Hydroxyproline
  MOD_RES (5)..(5): Hydroxyproline
  MOD_RES (8)..(8): Hydroxyproline
  MOD_RES (11)..(11): Hydroxyproline
  MOD_RES (14)..(14): Hydroxyproline
  MOD_RES (17)..(17): Hydroxyproline
  MOD_RES (20)..(20): Hydroxyproline
KPGPPGPPGPPGPPGPPGPPG

SEQ ID NO: 294 - protein, 21 aa, Artificial Sequence
  Description of Artificial Sequence: Synthetic peptide
  MOD_RES (5)..(5): Hydroxyproline
  MOD_RES (8)..(8): Hydroxyproline
  MOD_RES (11)..(11): Hydroxyproline
  MOD_RES (14)..(14): Hydroxyproline
  MOD_RES (17)..(17): Hydroxyproline
  MOD_RES (20)..(20): Hydroxyproline
PKGPPGPPGPPGPPGPPGPPG

SEQ ID NO: 295 - protein, 21 aa, Artificial Sequence
  Description of Artificial Sequence: Synthetic peptide
  MOD_RES (2)..(2): Hydroxyproline
  MOD_RES (5)..(5): Hydroxyproline
  MOD_RES (8)..(8): Hydroxyproline
  MOD_RES (11)..(11): Hydroxyproline
  MOD_RES (14)..(14): Hydroxyproline
  MOD_RES (17)..(17): Hydroxyproline
  MOD_RES (20)..(20): Hydroxyproline
PPGKPGPPGPPGPPGPPGPPG

SEQ ID NO: 296 - protein, 21 aa, Artificial Sequence
  Description of Artificial Sequence: Synthetic peptide
  MOD_RES (2)..(2): Hydroxyproline
  MOD_RES (8)..(8): Hydroxyproline
  MOD_RES (11)..(11): Hydroxyproline
  MOD_RES (14)..(14): Hydroxyproline
  MOD_RES (17)..(17): Hydroxyproline
  MOD_RES (20)..(20): Hydroxyproline
PPGPKGPPGPPGPPGPPGPPG

SEQ ID NO: 297 - protein, 21 aa, Artificial Sequence
  Description of Artificial Sequence: Synthetic peptide
  MOD_RES (2)..(2): Hydroxyproline
  MOD_RES (5)..(5): Hydroxyproline
  MOD_RES (8)..(8): Hydroxyproline
  MOD_RES (11)..(11): Hydroxyproline
  MOD_RES (14)..(14): Hydroxyproline
  MOD_RES (17)..(17): Hydroxyproline
  MOD_RES (20)..(20): Hydroxyproline
PPGPPGKPGPPGPPGPPGPPG

SEQ ID NO: 298 - protein, 21 aa, Artificial Sequence
  Description of Artificial Sequence: Synthetic peptide
  MOD_RES (2)..(2): Hydroxyproline
  MOD_RES (5)..(5): Hydroxyproline
  MOD_RES (8)..(8): Hydroxyproline
  MOD_RES (11)..(11): Hydroxyproline
  MOD_RES (14)..(14): Hydroxyproline
  MOD_RES (17)..(17): Hydroxyproline
  MOD_RES (20)..(20): Hydroxyproline
PPGPPGPPGKPGPPGPPGPPG

SEQ ID NO: 299 - protein, 21 aa, Artificial Sequence
  Description of Artificial Sequence: Synthetic peptide
  MOD_RES (2)..(2): Hydroxyproline
  MOD_RES (5)..(5): Hydroxyproline
  MOD_RES (8)..(8): Hydroxyproline
  MOD_RES (14)..(14): Hydroxyproline
  MOD_RES (17)..(17): Hydroxyproline
  MOD_RES (20)..(20): Hydroxyproline
PPGPPGPPGPKGPPGPPGPPG

SEQ ID NO: 300 - protein, 21 aa, Artificial Sequence
  Description of Artificial Sequence: Synthetic peptide
  MOD_RES (2)..(2): Hydroxyproline
  MOD_RES (5)..(5): Hydroxyproline
  MOD_RES (8)..(8): Hydroxyproline
  MOD_RES (11)..(11): Hydroxyproline
  MOD_RES (14)..(14): Hydroxyproline
  MOD_RES (17)..(17): Hydroxyproline
  MOD_RES (20)..(20): Hydroxyproline
PPGPPGPPGPPGKPGPPGPPG

SEQ ID NO: 301 - protein, 21 aa, Artificial Sequence
  Description of Artificial Sequence: Synthetic peptide
  MOD_RES (2)..(2): Hydroxyproline
  MOD_RES (5)..(5): Hydroxyproline
  MOD_RES (8)..(8): Hydroxyproline
  MOD_RES (11)..(11): Hydroxyproline
  MOD_RES (17)..(17): Hydroxyproline
  MOD_RES (20)..(20): Hydroxyproline
PPGPPGPPGPPGPKGPPGPPG

SEQ ID NO: 302 - protein, 21 aa, Artificial Sequence
  Description of Artificial Sequence: Synthetic peptide
  MOD_RES (2)..(2): Hydroxyproline
  MOD_RES (5)..(5): Hydroxyproline
  MOD_RES (8)..(8): Hydroxyproline
  MOD_RES (11)..(11): Hydroxyproline
  MOD_RES (14)..(14): Hydroxyproline
  MOD_RES (17)..(17): Hydroxyproline
  MOD_RES (20)..(20): Hydroxyproline
PPGPPGPPGPPGPPGKPGPPG

SEQ ID NO: 303 - protein, 21 aa, Artificial Sequence
  Description of Artificial Sequence: Synthetic peptide
  MOD_RES (2)..(2): Hydroxyproline
  MOD_RES (5)..(5): Hydroxyproline
  MOD_RES (8)..(8): Hydroxyproline
  MOD_RES (11)..(11): Hydroxyproline
  MOD_RES (14)..(14): Hydroxyproline
  MOD_RES (20)..(20): Hydroxyproline
PPGPPGPPGPPGPPGPKGPPG

SEQ ID NO: 304 - protein, 21 aa, Artificial Sequence
  Description of Artificial Sequence: Synthetic peptide
  MOD_RES (2)..(2): Hydroxyproline
  MOD_RES (5)..(5): Hydroxyproline
  MOD_RES (8)..(8): Hydroxyproline
  MOD_RES (11)..(11): Hydroxyproline
  MOD_RES (14)..(14): Hydroxyproline
  MOD_RES (17)..(17): Hydroxyproline
  MOD_RES (20)..(20): Hydroxyproline
PPGPPGPPGPPGPPGPPGKPG

SEQ ID NO: 305 - protein, 21 aa, Artificial Sequence
  Description of Artificial Sequence: Synthetic peptide
  MOD_RES (2)..(2): Hydroxyproline
  MOD_RES (5)..(5): Hydroxyproline
  MOD_RES (8)..(8): Hydroxyproline
  MOD_RES (11)..(11): Hydroxyproline
  MOD_RES (14)..(14): Hydroxyproline
  MOD_RES (17)..(17): Hydroxyproline
PPGPPGPPGPPGPPGPPGPKG

SEQ ID NO: 306 - protein, 21 aa, Artificial Sequence
  Description of Artificial Sequence: Synthetic peptide
  MOD_RES (2)..(2): Fluoroproline
  MOD_RES (5)..(5): Fluoroproline
  MOD_RES (8)..(8): Fluoroproline
  MOD_RES (11)..(11): Fluoroproline
  MOD_RES (14)..(14): Fluoroproline
  MOD_RES (17)..(17): Fluoroproline
  MOD_RES (20)..(20): Fluoroproline
KPGPPGPPGPPGPPGPPGPPG

SEQ ID NO: 307 - protein, 21 aa, Artificial Sequence
  Description of Artificial Sequence: Synthetic peptide
  MOD_RES (5)..(5): Fluoroproline
  MOD_RES (8)..(8): Fluoroproline
  MOD_RES (11)..(11): Fluoroproline
  MOD_RES (14)..(14): Fluoroproline
  MOD_RES (17)..(17): Fluoroproline
  MOD_RES (20)..(20): Fluoroproline
PKGPPGPPGPPGPPGPPGPPG

SEQ ID NO: 308 - protein, 21 aa, Artificial Sequence
  Description of Artificial Sequence: Synthetic peptide
  MOD_RES (2)..(2): Fluoroproline
  MOD_RES (5)..(5): Fluoroproline
  MOD_RES (8)..(8): Fluoroproline
  MOD_RES (11)..(11): Fluoroproline
  MOD_RES (14)..(14): Fluoroproline
  MOD_RES (17)..(17): Fluoroproline
  MOD_RES (20)..(20): Fluoroproline
PPGKPGPPGPPGPPGPPGPPG

SEQ ID NO: 309 - protein, 21 aa, Artificial Sequence
  Description of Artificial Sequence: Synthetic peptide
  MOD_RES (2)..(2): Fluoroproline
  MOD_RES (8)..(8): Fluoroproline
  MOD_RES (11)..(11): Fluoroproline
  MOD_RES (14)..(14): Fluoroproline
  MOD_RES (17)..(17): Fluoroproline
  MOD_RES (20)..(20): Fluoroproline
PPGPKGPPGPPGPPGPPGPPG

SEQ ID NO: 310 - protein, 21 aa, Artificial Sequence
  Description of Artificial Sequence: Synthetic peptide
  MOD_RES (2)..(2): Fluoroproline
  MOD_RES (5)..(5): Fluoroproline
  MOD_RES (8)..(8): Fluoroproline
  MOD_RES (11)..(11): Fluoroproline
  MOD_RES (14)..(14): Fluoroproline
  MOD_RES (17)..(17): Fluoroproline
  MOD_RES (20)..(20): Fluoroproline
PPGPPGKPGPPGPPGPPGPPG

SEQ ID NO: 311 - protein, 21 aa, Artificial Sequence
  Description of Artificial Sequence: Synthetic peptide
  MOD_RES (2)..(2): Fluoroproline
  MOD_RES (5)..(5): Fluoroproline
  MOD_RES (8)..(8): Fluoroproline
  MOD_RES (11)..(11): Fluoroproline
  MOD_RES (14)..(14): Fluoroproline
  MOD_RES (17)..(17): Fluoroproline
  MOD_RES (20)..(20): Fluoroproline
PPGPPGPPGKPGPPGPPGPPG

SEQ ID NO: 312 - protein, 21 aa, Artificial Sequence
  Description of Artificial Sequence: Synthetic peptide
  MOD_RES (2)..(2): Fluoroproline
  MOD_RES (5)..(5): Fluoroproline
  MOD_RES (8)..(8): Fluoroproline
  MOD_RES (14)..(14): Fluoroproline
  MOD_RES (17)..(17): Fluoroproline
  MOD_RES (20)..(20): Fluoroproline
PPGPPGPPGPKGPPGPPGPPG

SEQ ID NO: 313 - protein, 21 aa, Artificial Sequence
  Description of Artificial Sequence: Synthetic peptide
  MOD_RES (2)..(2): Fluoroproline
  MOD_RES (5)..(5): Fluoroproline
  MOD_RES (8)..(8): Fluoroproline
  MOD_RES (11)..(11): Fluoroproline
  MOD_RES (14)..(14): Fluoroproline
  MOD_RES (17)..(17): Fluoroproline
  MOD_RES (20)..(20): Fluoroproline
PPGPPGPPGPPGKPGPPGPPG

SEQ ID NO: 314 - protein, 21 aa, Artificial Sequence
  Description of Artificial Sequence: Synthetic peptide
  MOD_RES (2)..(2): Fluoroproline
  MOD_RES (5)..(5): Fluoroproline
  MOD_RES (8)..(8): Fluoroproline
  MOD_RES (11)..(11): Fluoroproline
  MOD_RES (17)..(17): Fluoroproline
  MOD_RES (20)..(20): Fluoroproline
PPGPPGPPGPPGPKGPPGPPG

SEQ ID NO: 315 - protein, 21 aa, Artificial Sequence
  Description of Artificial Sequence: Synthetic peptide
  MOD_RES (2)..(2): Fluoroproline
  MOD_RES (5)..(5): Fluoroproline
  MOD_RES (8)..(8): Fluoroproline
  MOD_RES (11)..(11): Fluoroproline
  MOD_RES (14)..(14): Fluoroproline
  MOD_RES (17)..(17): Fluoroproline
  MOD_RES (20)..(20): Fluoroproline
PPGPPGPPGPPGPPGKPGPPG

SEQ ID NO: 316 - protein, 21 aa, Artificial Sequence
  Description of Artificial Sequence: Synthetic peptide
  MOD_RES (2)..(2): Fluoroproline
  MOD_RES (5)..(5): Fluoroproline
  MOD_RES (8)..(8): Fluoroproline
  MOD_RES (11)..(11): Fluoroproline
  MOD_RES (14)..(14): Fluoroproline
  MOD_RES (20)..(20): Fluoroproline
PPGPPGPPGPPGPPGPKGPPG

SEQ ID NO: 317 - protein, 21 aa, Artificial Sequence
  Description of Artificial Sequence: Synthetic peptide
  MOD_RES (2)..(2): Fluoroproline
  MOD_RES (5)..(5): Fluoroproline
  MOD_RES (8)..(8): Fluoroproline
  MOD_RES (11)..(11): Fluoroproline
  MOD_RES (14)..(14): Fluoroproline
  MOD_RES (17)..(17): Fluoroproline
  MOD_RES (20)..(20): Fluoroproline
PPGPPGPPGPPGPPGPPGKPG

SEQ ID NO: 318 - protein, 21 aa, Artificial Sequence
  Description of Artificial Sequence: Synthetic peptide
  MOD_RES (2)..(2): Fluoroproline
  MOD_RES (5)..(5): Fluoroproline
  MOD_RES (8)..(8): Fluoroproline
  MOD_RES (11)..(11): Fluoroproline
  MOD_RES (14)..(14): Fluoroproline
  MOD_RES (17)..(17): Fluoroproline
PPGPPGPPGPPGPPGPPGPKG

SEQ ID NO: 319 - protein, 21 aa, Artificial Sequence
  Description of Artificial Sequence: Synthetic peptide
  MOD_RES (2)..(2): Fluoroproline
  MOD_RES (5)..(5): Fluoroproline
  MOD_RES (8)..(8): Fluoroproline
  MOD_RES (11)..(11): Fluoroproline
  MOD_RES (14)..(14): Fluoroproline
  MOD_RES (17)..(17): Fluoroproline
  MOD_RES (20)..(20): Fluoroproline
KPGPPGPPGPPGPPGPPGPPG

SEQ ID NO: 320 - protein, 21 aa, Artificial Sequence
  Description of Artificial Sequence: Synthetic peptide
  MOD_RES (5)..(5): Fluoroproline
  MOD_RES (8)..(8): Fluoroproline
  MOD_RES (11)..(11): Fluoroproline
  MOD_RES (14)..(14): Fluoroproline
  MOD_RES (17)..(17): Fluoroproline
  MOD_RES (20)..(20): Fluoroproline
PKGPPGPPGPPGPPGPPGPPG

SEQ ID NO: 321 - protein, 21 aa, Artificial Sequence
  Description of Artificial Sequence: Synthetic peptide
  MOD_RES (2)..(2): Fluoroproline
  MOD_RES (5)..(5): Fluoroproline
  MOD_RES (8)..(8): Fluoroproline
  MOD_RES (11)..(11): Fluoroproline
  MOD_RES (14)..(14): Fluoroproline
  MOD_RES (17)..(17): Fluoroproline
  MOD_RES (20)..(20): Fluoroproline
PPGKPGPPGPPGPPGPPGPPG

SEQ ID NO: 322 - protein, 21 aa, Artificial Sequence
  Description of Artificial Sequence: Synthetic peptide
  MOD_RES (2)..(2): Fluoroproline
  MOD_RES (8)..(8): Fluoroproline
  MOD_RES (11)..(11): Fluoroproline
  MOD_RES (14)..(14): Fluoroproline
  MOD_RES (17)..(17): Fluoroproline
  MOD_RES (20)..(20): Fluoroproline
PPGPKGPPGPPGPPGPPGPPG

SEQ ID NO: 323 - protein, 21 aa, Artificial Sequence
  Description of Artificial Sequence: Synthetic peptide
  MOD_RES (2)..(2): Fluoroproline
  MOD_RES (5)..(5): Fluoroproline
  MOD_RES (8)..(8): Fluoroproline
  MOD_RES (11)..(11): Fluoroproline
  MOD_RES (14)..(14): Fluoroproline
  MOD_RES (17)..(17): Fluoroproline
  MOD_RES (20)..(20): Fluoroproline
PPGPPGKPGPPGPPGPPGPPG

SEQ ID NO: 324 - protein, 21 aa, Artificial Sequence
  Description of Artificial Sequence: Synthetic peptide
  MOD_RES (2)..(2): Fluoroproline
  MOD_RES (5)..(5): Fluoroproline
  MOD_RES (11)..(11): Fluoroproline
  MOD_RES (14)..(14): Fluoroproline
  MOD_RES (17)..(17): Fluoroproline
  MOD_RES (20)..(20): Fluoroproline
PPGPPGPKGPPGPPGPPGPPG

SEQ ID NO: 325 - protein, 21 aa, Artificial Sequence
  Description of Artificial Sequence: Synthetic peptide
  MOD_RES (2)..(2): Fluoroproline
  MOD_RES (5)..(5): Fluoroproline
  MOD_RES (8)..(8): Fluoroproline
  MOD_RES (11)..(11): Fluoroproline
  MOD_RES (14)..(14): Fluoroproline
  MOD_RES (17)..(17): Fluoroproline
  MOD_RES (20)..(20): Fluoroproline
PPGPPGPPGKPGPPGPPGPPG

SEQ ID NO: 326 - protein, 21 aa, Artificial Sequence
  Description of Artificial Sequence: Synthetic peptide
  MOD_RES (2)..(2): Fluoroproline
  MOD_RES (5)..(5): Fluoroproline
  MOD_RES (8)..(8): Fluoroproline
  MOD_RES (14)..(14): Fluoroproline
  MOD_RES (17)..(17): Fluoroproline
  MOD_RES (20)..(20): Fluoroproline
PPGPPGPPGPKGPPGPPGPPG

SEQ ID NO: 327 - protein, 21 aa, Artificial Sequence
  Description of Artificial Sequence: Synthetic peptide
  MOD_RES (2)..(2): Fluoroproline
  MOD_RES (5)..(5): Fluoroproline
  MOD_RES (8)..(8): Fluoroproline
  MOD_RES (11)..(11): Fluoroproline
  MOD_RES (14)..(14): Fluoroproline
  MOD_RES (17)..(17): Fluoroproline
  MOD_RES (20)..(20): Fluoroproline
PPGPPGPPGPPGKPGPPGPPG

SEQ ID NO: 328 - protein, 21 aa, Artificial Sequence
  Description of Artificial Sequence: Synthetic peptide
  MOD_RES (2)..(2): Fluoroproline
  MOD_RES (5)..(5): Fluoroproline
  MOD_RES (8)..(8): Fluoroproline
  MOD_RES (11)..(11): Fluoroproline
  MOD_RES (17)..(17): Fluoroproline
  MOD_RES (20)..(20): Fluoroproline
PPGPPGPPGPPGPKGPPGPPG

SEQ ID NO: 329 - protein, 21 aa, Artificial Sequence
  Description of Artificial Sequence: Synthetic peptide
  MOD_RES (2)..(2): Fluoroproline
  MOD_RES (5)..(5): Fluoroproline
  MOD_RES (8)..(8): Fluoroproline
  MOD_RES (11)..(11): Fluoroproline
  MOD_RES (14)..(14): Fluoroproline
  MOD_RES (17)..(17): Fluoroproline
  MOD_RES (20)..(20): Fluoroproline
PPGPPGPPGPPGPPGKPGPPG

SEQ ID NO: 330 - protein, 21 aa, Artificial Sequence
  Description of Artificial Sequence: Synthetic peptide
  MOD_RES (2)..(2): Fluoroproline
  MOD_RES (5)..(5): Fluoroproline
  MOD_RES (8)..(8): Fluoroproline
  MOD_RES (11)..(11): Fluoroproline
  MOD_RES (14)..(14): Fluoroproline
  MOD_RES (20)..(20): Fluoroproline
PPGPPGPPGPPGPPGPKGPPG

SEQ ID NO: 331 - protein, 21 aa, Artificial Sequence
  Description of Artificial Sequence: Synthetic peptide
  MOD_RES (2)..(2): Fluoroproline
  MOD_RES (5)..(5): Fluoroproline
  MOD_RES (8)..(8): Fluoroproline
  MOD_RES (11)..(11): Fluoroproline
  MOD_RES (14)..(14): Fluoroproline
  MOD_RES (17)..(17): Fluoroproline
  MOD_RES (20)..(20): Fluoroproline
PPGPPGPPGPPGPPGPPGKPG

SEQ ID NO: 332 - protein, 21 aa, Artificial Sequence
  Description of Artificial Sequence: Synthetic peptide
  MOD_RES (2)..(2): Fluoroproline
  MOD_RES (5)..(5): Fluoroproline
  MOD_RES (8)..(8): Fluoroproline
  MOD_RES (11)..(11): Fluoroproline
  MOD_RES (14)..(14): Fluoroproline
  MOD_RES (17)..(17): Fluoroproline
PPGPPGPPGPPGPPGPPGPKG

SEQ ID NO: 333 - protein, 21 aa, Artificial Sequence
  Description of Artificial Sequence: Synthetic peptide
  MOD_RES (2)..(2): Hydroxyproline
  MOD_RES (4)..(4): Fluoroproline
  MOD_RES (5)..(5): Hydroxyproline
  MOD_RES (7)..(7): Fluoroproline
  MOD_RES (8)..(8): Hydroxyproline
  MOD_RES (10)..(10): Fluoroproline
  MOD_RES (11)..(11): Hydroxyproline
  MOD_RES (13)..(13): Fluoroproline
  MOD_RES (14)..(14): Hydroxyproline
  MOD_RES (16)..(16): Fluoroproline
  MOD_RES (17)..(17): Hydroxyproline
  MOD_RES (19)..(19): Fluoroproline
  MOD_RES (20)..(20): Hydroxyproline
KPGPPGPPGPPGPPGPPGPPG

SEQ ID NO: 334 - protein, 21 aa, Artificial Sequence
  Description of Artificial Sequence: Synthetic peptide
  MOD_RES (1)..(1): Fluoroproline
  MOD_RES (4)..(4): Fluoroproline
  MOD_RES (5)..(5): Hydroxyproline
  MOD_RES (7)..(7): Fluoroproline
  MOD_RES (8)..(8): Hydroxyproline
  MOD_RES (10)..(10): Fluoroproline
  MOD_RES (11)..(11): Hydroxyproline
  MOD_RES (13)..(13): Fluoroproline
  MOD_RES (14)..(14): Hydroxyproline
  MOD_RES (16)..(16): Fluoroproline
  MOD_RES (17)..(17): Hydroxyproline
  MOD_RES (19)..(19): Fluoroproline
  MOD_RES (20)..(20): Hydroxyproline
PKGPPGPPGPPGPPGPPGPPG

SEQ ID NO: 335 - protein, 21 aa, Artificial Sequence
  Description of Artificial Sequence: Synthetic peptide
  MOD_RES (1)..(1): Fluoroproline
  MOD_RES (2)..(2): Hydroxyproline
  MOD_RES (5)..(5): Hydroxyproline
  MOD_RES (7)..(7): Fluoroproline
  MOD_RES (8)..(8): Hydroxyproline
  MOD_RES (10)..(10): Fluoroproline
  MOD_RES (11)..(11): Hydroxyproline
  MOD_RES (13)..(13): Fluoroproline
  MOD_RES (14)..(14): Hydroxyproline
  MOD_RES (16)..(16): Fluoroproline
  MOD_RES (17)..(17): Hydroxyproline
  MOD_RES (19)..(19): Fluoroproline
  MOD_RES (20)..(20): Hydroxyproline
PPGKPGPPGPPGPPGPPGPPG

SEQ ID NO: 336 - protein, 21 aa, Artificial Sequence
  Description of Artificial Sequence: Synthetic peptide
  MOD_RES (1)..(1): Fluoroproline
  MOD_RES (2)..(2): Hydroxyproline
  MOD_RES (4)..(4): Fluoroproline
  MOD_RES (7)..(7): Fluoroproline
  MOD_RES (8)..(8): Hydroxyproline
  MOD_RES (10)..(10): Fluoroproline
  MOD_RES (11)..(11): Hydroxyproline
  MOD_RES (13)..(13): Fluoroproline
  MOD_RES (14)..(14): Hydroxyproline
  MOD_RES (16)..(16): Fluoroproline
  MOD_RES (17)..(17): Hydroxyproline
  MOD_RES (19)..(19): Fluoroproline
  MOD_RES (20)..(20): Hydroxyproline
PPGPKGPPGPPGPPGPPGPPG

SEQ ID NO: 337 - protein, 21 aa, Artificial Sequence
  Description of Artificial Sequence: Synthetic peptide
  MOD_RES (1)..(1): Fluoroproline
  MOD_RES (2)..(2): Hydroxyproline
  MOD_RES (4)..(4): Fluoroproline
  MOD_RES (5)..(5): Hydroxyproline
  MOD_RES (8)..(8): Hydroxyproline
  MOD_RES (10)..(10): Fluoroproline
  MOD_RES (11)..(11): Hydroxyproline
  MOD_RES (13)..(13): Fluoroproline
  MOD_RES (14)..(14): Hydroxyproline
  MOD_RES (16)..(16): Fluoroproline
  MOD_RES (17)..(17): Hydroxyproline
  MOD_RES (19)..(19): Fluoroproline
  MOD_RES (20)..(20): Hydroxyproline
PPGPPGKPGPPGPPGPPGPPG

SEQ ID NO: 338 - protein, 21 aa, Artificial Sequence
  Description of Artificial Sequence: Synthetic peptide
  MOD_RES (1)..(1): Fluoroproline
  MOD_RES (2)..(2): Hydroxyproline
  MOD_RES (4)..(4): Fluoroproline
  MOD_RES (5)..(5): Hydroxyproline
  MOD_RES (7)..(7): Fluoroproline
  MOD_RES (10)..(10): Fluoroproline
  MOD_RES (11)..(11): Hydroxyproline
  MOD_RES (13)..(13): Fluoroproline
  MOD_RES (14)..(14): Hydroxyproline
  MOD_RES (16)..(16): Fluoroproline
  MOD_RES (17)..(17): Hydroxyproline
  MOD_RES (19)..(19): Fluoroproline
  MOD_RES (20)..(20): Hydroxyproline
PPGPPGPKGPPGPPGPPGPPG

SEQ ID NO: 339 - protein, 21 aa, Artificial Sequence
  Description of Artificial Sequence: Synthetic peptide
  MOD_RES (1)..(1): Fluoroproline
  MOD_RES (2)..(2): Hydroxyproline
  MOD_RES (4)..(4): Fluoroproline
  MOD_RES (5)..(5): Hydroxyproline
  MOD_RES (7)..(7): Fluoroproline
  MOD_RES (8)..(8): Hydroxyproline
  MOD_RES (11)..(11): Hydroxyproline
  MOD_RES (13)..(13): Fluoroproline
  MOD_RES (14)..(14): Hydroxyproline
  MOD_RES (16)..(16): Fluoroproline
  MOD_RES (17)..(17): Hydroxyproline
  MOD_RES (19)..(19): Fluoroproline
  MOD_RES (20)..(20): Hydroxyproline
PPGPPGPPGKPGPPGPPGPPG

SEQ ID NO: 340 - protein, 21 aa, Artificial Sequence
  Description of Artificial Sequence: Synthetic peptide
  MOD_RES (1)..(1): Fluoroproline
  MOD_RES (2)..(2): Hydroxyproline
  MOD_RES (4)..(4): Fluoroproline
  MOD_RES (5)..(5): Hydroxyproline
  MOD_RES (7)..(7): Fluoroproline
  MOD_RES (8)..(8): Hydroxyproline
  MOD_RES (10)..(10): Fluoroproline
  MOD_RES (13)..(13): Fluoroproline
  MOD_RES (14)..(14): Hydroxyproline
  MOD_RES (16)..(16): Fluoroproline
  MOD_RES (17)..(17): Hydroxyproline
  MOD_RES (19)..(19): Fluoroproline
  MOD_RES (20)..(20): Hydroxyproline
PPGPPGPPGPKGPPGPPGPPG

SEQ ID NO: 341 - protein, 21 aa, Artificial Sequence
  Description of Artificial Sequence: Synthetic peptide
  MOD_RES (1)..(1): Fluoroproline
  MOD_RES (2)..(2): Hydroxyproline
  MOD_RES (4)..(4): Fluoroproline
  MOD_RES (5)..(5): Hydroxyproline
  MOD_RES (7)..(7): Fluoroproline
  MOD_RES (8)..(8): Hydroxyproline
  MOD_RES (10)..(10): Fluoroproline
  MOD_RES (11)..(11): Hydroxyproline
  MOD_RES (14)..(14): Hydroxyproline
  MOD_RES (16)..(16): Fluoroproline
  MOD_RES (17)..(17): Hydroxyproline
  MOD_RES (19)..(19): Fluoroproline
  MOD_RES (20)..(20): Hydroxyproline
PPGPPGPPGPPGKPGPPGPPG

SEQ ID NO: 342 - protein, 21 aa, Artificial Sequence
  Description of Artificial Sequence: Synthetic peptide
  MOD_RES (1)..(1): Fluoroproline
  MOD_RES (2)..(2): Hydroxyproline
  MOD_RES (4)..(4): Fluoroproline
  MOD_RES (5)..(5): Hydroxyproline
  MOD_RES (7)..(7): Fluoroproline
  MOD_RES (8)..(8): Hydroxyproline
  MOD_RES (10)..(10): Fluoroproline
  MOD_RES (11)..(11): Hydroxyproline
  MOD_RES (13)..(13): Fluoroproline
  MOD_RES (16)..(16): Fluoroproline
  MOD_RES (17)..(17): Hydroxyproline
  MOD_RES (19)..(19): Fluoroproline
  MOD_RES (20)..(20): Hydroxyproline
PPGPPGPPGPPGPKGPPGPPG

SEQ ID NO: 343 - protein, 21 aa, Artificial Sequence
  Description of Artificial Sequence: Synthetic peptide
  MOD_RES (1)..(1): Fluoroproline
  MOD_RES (2)..(2): Hydroxyproline
  MOD_RES (4)..(4): Fluoroproline
  MOD_RES (5)..(5): Hydroxyproline
  MOD_RES (7)..(7): Fluoroproline
  MOD_RES (8)..(8): Hydroxyproline
  MOD_RES (10)..(10): Fluoroproline
  MOD_RES (11)..(11): Hydroxyproline
  MOD_RES (13)..(13): Fluoroproline
  MOD_RES (14)..(14): Hydroxyproline
  MOD_RES (17)..(17): Hydroxyproline
  MOD_RES (19)..(19): Fluoroproline
  MOD_RES (20)..(20): Hydroxyproline
PPGPPGPPGPPGPPGKPGPPG

SEQ ID NO: 344 - protein, 21 aa, Artificial Sequence
  Description of Artificial Sequence: Synthetic peptide
  MOD_RES (1)..(1): Fluoroproline
  MOD_RES (2)..(2): Hydroxyproline
  MOD_RES (4)..(4): Fluoroproline
  MOD_RES (5)..(5): Hydroxyproline
  MOD_RES (7)..(7): Fluoroproline
  MOD_RES (8)..(8): Hydroxyproline
  MOD_RES (10)..(10): Fluoroproline
  MOD_RES (11)..(11): Hydroxyproline
  MOD_RES (13)..(13): Fluoroproline
  MOD_RES (14)..(14): Hydroxyproline
  MOD_RES (16)..(16): Fluoroproline
  MOD_RES (19)..(19): Fluoroproline
  MOD_RES (20)..(20): Hydroxyproline
PPGPPGPPGPPGPPGPKGPPG

SEQ ID NO: 345 - protein, 21 aa, Artificial Sequence
  Description of Artificial Sequence: Synthetic peptide
  MOD_RES (1)..(1): Fluoroproline
  MOD_RES (2)..(2): Hydroxyproline
  MOD_RES (4)..(4): Fluoroproline
  MOD_RES (5)..(5): Hydroxyproline
  MOD_RES (7)..(7): Fluoroproline
  MOD_RES (8)..(8): Hydroxyproline
  MOD_RES (10)..(10): Fluoroproline
  MOD_RES (11)..(11): Hydroxyproline
  MOD_RES (13)..(13): Fluoroproline
  MOD_RES (14)..(14): Hydroxyproline
  MOD_RES (16)..(16): Fluoroproline
  MOD_RES (17)..(17): Hydroxyproline
  MOD_RES (20)..(20): Hydroxyproline
PPGPPGPPGPPGPPGPPGKPG

SEQ ID NO: 346 - protein, 21 aa, Artificial Sequence
  Description of Artificial Sequence: Synthetic peptide
  MOD_RES (1)..(1): Fluoroproline
  MOD_RES (2)..(2): Hydroxyproline
  MOD_RES (4)..(4): Fluoroproline
  MOD_RES (5)..(5): Hydroxyproline
  MOD_RES (7)..(7): Fluoroproline
  MOD_RES (8)..(8): Hydroxyproline
  MOD_RES (10)..(10): Fluoroproline
  MOD_RES (11)..(11): Hydroxyproline
  MOD_RES (13)..(13): Fluoroproline
  MOD_RES (14)..(14): Hydroxyproline
  MOD_RES (16)..(16): Fluoroproline
  MOD_RES (17)..(17): Hydroxyproline
  MOD_RES (19)..(19): Fluoroproline
PPGPPGPPGPPGPPGPPGPKG

SEQ ID NO: 347 - protein, 21 aa, Artificial Sequence
  Description of Artificial Sequence: Synthetic peptide
  MOD_RES (2)..(2): Chloroproline
  MOD_RES (5)..(5): Chloroproline
  MOD_RES (8)..(8): Chloroproline
  MOD_RES (11)..(11): Chloroproline
  MOD_RES (14)..(14): Chloroproline
  MOD_RES (17)..(17): Chloroproline
  MOD_RES (20)..(20): Chloroproline
KPGPPGPPGPPGPPGPPGPPG

SEQ ID NO: 348 - protein, 21 aa, Artificial Sequence
  Description of Artificial Sequence: Synthetic peptide
  MOD_RES (5)..(5): Chloroproline
  MOD_RES (8)..(8): Chloroproline
  MOD_RES (11)..(11): Chloroproline
  MOD_RES (14)..(14): Chloroproline
  MOD_RES (17)..(17): Chloroproline
  MOD_RES (20)..(20): Chloroproline
PKGPPGPPGPPGPPGPPGPPG

SEQ ID NO: 349 - protein, 21 aa, Artificial Sequence
  Description of Artificial Sequence: Synthetic peptide
  MOD_RES (2)..(2): Chloroproline
  MOD_RES (5)..(5): Chloroproline
  MOD_RES (8)..(8): Chloroproline
  MOD_RES (11)..(11): Chloroproline
  MOD_RES (14)..(14): Chloroproline
  MOD_RES (17)..(17): Chloroproline
  MOD_RES (20)..(20): Chloroproline
PPGKPGPPGPPGPPGPPGPPG

SEQ ID NO: 350 - protein, 21 aa, Artificial Sequence
  Description of Artificial Sequence: Synthetic peptide
  MOD_RES (2)..(2): Chloroproline
  MOD_RES (8)..(8): Chloroproline
  MOD_RES (11)..(11): Chloroproline
  MOD_RES (14)..(14): Chloroproline
  MOD_RES (17)..(17): Chloroproline
  MOD_RES (20)..(20): Chloroproline
PPGPKGPPGPPGPPGPPGPPG

SEQ ID NO: 351 - protein, 21 aa, Artificial Sequence
  Description of Artificial Sequence: Synthetic peptide
  MOD_RES (2)..(2): Chloroproline
  MOD_RES (5)..(5): Chloroproline
  MOD_RES (8)..(8): Chloroproline
  MOD_RES (11)..(11): Chloroproline
  MOD_RES (14)..(14): Chloroproline
  MOD_RES (17)..(17): Chloroproline
  MOD_RES (20)..(20): Chloroproline
PPGPPGKPGPPGPPGPPGPPG

SEQ ID NO: 352 - protein, 21 aa, Artificial Sequence
  Description of Artificial Sequence: Synthetic peptide
  MOD_RES (2)..(2): Chloroproline
  MOD_RES (5)..(5): Chloroproline
  MOD_RES (8)..(8): Chloroproline
  MOD_RES (11)..(11): Chloroproline
  MOD_RES (14)..(14): Chloroproline
  MOD_RES (17)..(17): Chloroproline
  MOD_RES (20)..(20): Chloroproline
PPGPPGPPGKPGPPGPPGPPG

SEQ ID NO: 353 - protein, 21 aa, Artificial Sequence
  Description of Artificial Sequence: Synthetic peptide
  MOD_RES (2)..(2): Chloroproline
  MOD_RES (5)..(5): Chloroproline
  MOD_RES (8)..(8): Chloroproline
  MOD_RES (14)..(14): Chloroproline
  MOD_RES (17)..(17): Chloroproline
  MOD_RES (20)..(20): Chloroproline
PPGPPGPPGPKGPPGPPGPPG

SEQ ID NO: 354 - protein, 21 aa, Artificial Sequence
  Description of Artificial Sequence: Synthetic peptide
  MOD_RES (2)..(2): Chloroproline
  MOD_RES (5)..(5): Chloroproline
  MOD_RES (8)..(8): Chloroproline
  MOD_RES (11)..(11): Chloroproline
  MOD_RES (14)..(14): Chloroproline
  MOD_RES (17)..(17): Chloroproline
  MOD_RES (20)..(20): Chloroproline
PPGPPGPPGPPGKPGPPGPPG

SEQ ID NO: 355 - protein, 21 aa, Artificial Sequence
  Description of Artificial Sequence: Synthetic peptide
  MOD_RES (2)..(2): Chloroproline
  MOD_RES (5)..(5): Chloroproline
  MOD_RES (8)..(8): Chloroproline
  MOD_RES (11)..(11): Chloroproline
  MOD_RES (17)..(17): Chloroproline
  MOD_RES (20)..(20): Chloroproline
PPGPPGPPGPPGPKGPPGPPG

SEQ ID NO: 356 - protein, 21 aa, Artificial Sequence
  Description of Artificial Sequence: Synthetic peptide
  MOD_RES (2)..(2): Chloroproline
  MOD_RES (5)..(5): Chloroproline
  MOD_RES (8)..(8): Chloroproline
  MOD_RES (11)..(11): Chloroproline
  MOD_RES (14)..(14): Chloroproline
  MOD_RES (17)..(17): Chloroproline
  MOD_RES (20)..(20): Chloroproline
PPGPPGPPGPPGPPGKPGPPG

SEQ ID NO: 357 - protein, 21 aa, Artificial Sequence
  Description of Artificial Sequence: Synthetic peptide
  MOD_RES (2)..(2): Chloroproline
  MOD_RES (5)..(5): Chloroproline
  MOD_RES (8)..(8): Chloroproline
  MOD_RES (11)..(11): Chloroproline
  MOD_RES (14)..(14): Chloroproline
  MOD_RES (20)..(20): Chloroproline
PPGPPGPPGPPGPPGPKGPPG

SEQ ID NO: 358 - protein, 21 aa, Artificial Sequence
  Description of Artificial Sequence: Synthetic peptide
  MOD_RES (2)..(2): Chloroproline
  MOD_RES (5)..(5): Chloroproline
  MOD_RES (8)..(8): Chloroproline
  MOD_RES (11)..(11): Chloroproline
  MOD_RES (14)..(14): Chloroproline
  MOD_RES (17)..(17): Chloroproline
  MOD_RES (20)..(20): Chloroproline
PPGPPGPPGPPGPPGPPGKPG

SEQ ID NO: 359 - protein, 21 aa, Artificial Sequence
  Description of Artificial Sequence: Synthetic peptide
  MOD_RES (2)..(2): Chloroproline
  MOD_RES (5)..(5): Chloroproline
  MOD_RES (8)..(8): Chloroproline
  MOD_RES (11)..(11): Chloroproline
  MOD_RES (14)..(14): Chloroproline
  MOD_RES (17)..(17): Chloroproline
PPGPPGPPGPPGPPGPPGPKG

SEQ ID NO: 360 - protein, 21 aa, Artificial Sequence
  Description of Artificial Sequence: Synthetic peptide
  MOD_RES (2)..(2): Chloroproline
  MOD_RES (5)..(5): Chloroproline
  MOD_RES (8)..(8): Chloroproline
  MOD_RES (11)..(11): Chloroproline
  MOD_RES (14)..(14): Chloroproline
  MOD_RES (17)..(17): Chloroproline
  MOD_RES (20)..(20): Chloroproline
KPGPPGPPGPPGPPGPPGPPG

SEQ ID NO: 361 - protein, 21 aa, Artificial Sequence
  Description of Artificial Sequence: Synthetic peptide
  MOD_RES (5)..(5): Chloroproline
  MOD_RES (8)..(8): Chloroproline
  MOD_RES (11)..(11): Chloroproline
  MOD_RES (14)..(14): Chloroproline
  MOD_RES (17)..(17): Chloroproline
  MOD_RES (20)..(20): Chloroproline
PKGPPGPPGPPGPPGPPGPPG

SEQ ID NO: 362 - protein, 21 aa, Artificial Sequence
  Description of Artificial Sequence: Synthetic peptide
  MOD_RES (2)..(2): Chloroproline
  MOD_RES (5)..(5): Chloroproline
  MOD_RES (8)..(8): Chloroproline
  MOD_RES (11)..(11): Chloroproline
  MOD_RES (14)..(14): Chloroproline
  MOD_RES (17)..(17): Chloroproline
  MOD_RES (20)..(20): Chloroproline
PPGKPGPPGPPGPPGPPGPPG

SEQ ID NO: 363 - protein, 21 aa, Artificial Sequence
  Description of Artificial Sequence: Synthetic peptide
  MOD_RES (2)..(2): Chloroproline
  MOD_RES (8)..(8): Chloroproline
  MOD_RES (11)..(11): Chloroproline
  MOD_RES (14)..(14): Chloroproline
  MOD_RES (17)..(17): Chloroproline
  MOD_RES (20)..(20): Chloroproline
PPGPKGPPGPPGPPGPPGPPG

SEQ ID NO: 364 - protein, 21 aa, Artificial Sequence
  Description of Artificial Sequence: Synthetic peptide
  MOD_RES (2)..(2): Chloroproline
  MOD_RES (5)..(5): Chloroproline
  MOD_RES (8)..(8): Chloroproline
  MOD_RES (11)..(11): Chloroproline
  MOD_RES (14)..(14): Chloroproline
  MOD_RES (17)..(17): Chloroproline
  MOD_RES (20)..(20): Chloroproline
PPGPPGKPGPPGPPGPPGPPG

SEQ ID NO: 365 - protein, 21 aa, Artificial Sequence
  Description of Artificial Sequence: Synthetic peptide
  MOD_RES (2)..(2): Chloroproline
  MOD_RES (5)..(5): Chloroproline
  MOD_RES (11)..(11): Chloroproline
  MOD_RES (14)..(14): Chloroproline
  MOD_RES (17)..(17): Chloroproline
  MOD_RES (20)..(20): Chloroproline
PPGPPGPKGPPGPPGPPGPPG

SEQ ID NO: 366 - protein, 21 aa, Artificial Sequence
  Description of Artificial Sequence: Synthetic peptide
  MOD_RES (2)..(2): Chloroproline
  MOD_RES (5)..(5): Chloroproline
  MOD_RES (8)..(8): Chloroproline
  MOD_RES (11)..(11): Chloroproline
  MOD_RES (14)..(14): Chloroproline
  MOD_RES (17)..(17): Chloroproline
  MOD_RES (20)..(20): Chloroproline
PPGPPGPPGKPGPPGPPGPPG

SEQ ID NO: 367 - protein, 21 aa, Artificial Sequence
  Description of Artificial Sequence: Synthetic peptide
  MOD_RES (2)..(2): Chloroproline
  MOD_RES (5)..(5): Chloroproline
  MOD_RES (8)..(8): Chloroproline
  MOD_RES (14)..(14): Chloroproline
  MOD_RES (17)..(17): Chloroproline
  MOD_RES (20)..(20): Chloroproline
PPGPPGPPGPKGPPGPPGPPG

SEQ ID NO: 368 - protein, 21 aa, Artificial Sequence
  Description of Artificial Sequence: Synthetic peptide
  MOD_RES (2)..(2): Chloroproline
  MOD_RES (5)..(5): Chloroproline
  MOD_RES (8)..(8): Chloroproline
  MOD_RES (11)..(11): Chloroproline
  MOD_RES (14)..(14): Chloroproline
  MOD_RES (17)..(17): Chloroproline
  MOD_RES (20)..(20): Chloroproline
PPGPPGPPGPPGKPGPPGPPG

SEQ ID NO: 369 - protein, 21 aa, Artificial Sequence
  Description of Artificial Sequence: Synthetic peptide
  MOD_RES (2)..(2): Chloroproline
  MOD_RES (5)..(5): Chloroproline
  MOD_RES (8)..(8): Chloroproline
  MOD_RES (11)..(11): Chloroproline
  MOD_RES (17)..(17): Chloroproline
  MOD_RES (20)..(20): Chloroproline
PPGPPGPPGPPGPKGPPGPPG

SEQ ID NO: 370 - protein, 21 aa, Artificial Sequence
  Description of Artificial Sequence: Synthetic peptide
  MOD_RES (2)..(2): Chloroproline
  MOD_RES (5)..(5): Chloroproline
  MOD_RES (8)..(8): Chloroproline
  MOD_RES (11)..(11): Chloroproline
  MOD_RES (14)..(14): Chloroproline
  MOD_RES (17)..(17): Chloroproline
  MOD_RES (20)..(20): Chloroproline
PPGPPGPPGPPGPPGKPGPPG

SEQ ID NO: 371 - protein, 21 aa, Artificial Sequence
  Description of Artificial Sequence: Synthetic peptide
  MOD_RES (2)..(2): Chloroproline
  MOD_RES (5)..(5): Chloroproline
  MOD_RES (8)..(8): Chloroproline
  MOD_RES (11)..(11): Chloroproline
  MOD_RES (14)..(14): Chloroproline
  MOD_RES (20)..(20): Chloroproline
PPGPPGPPGPPGPPGPKGPPG

SEQ ID NO: 372 - protein, 21 aa, Artificial Sequence
  Description of Artificial Sequence: Synthetic peptide
  MOD_RES (2)..(2): Chloroproline
  MOD_RES (5)..(5): Chloroproline
  MOD_RES (8)..(8): Chloroproline
  MOD_RES (11)..(11): Chloroproline
  MOD_RES (14)..(14): Chloroproline
  MOD_RES (17)..(17): Chloroproline
  MOD_RES (20)..(20): Chloroproline
PPGPPGPPGPPGPPGPPGKPG

SEQ ID NO: 373 - protein, 21 aa, Artificial Sequence
  Description of Artificial Sequence: Synthetic peptide
  MOD_RES (2)..(2): Chloroproline
  MOD_RES (5)..(5): Chloroproline
  MOD_RES (8)..(8): Chloroproline
  MOD_RES (11)..(11): Chloroproline
  MOD_RES (14)..(14): Chloroproline
  MOD_RES (17)..(17): Chloroproline
PPGPPGPPGPPGPPGPPGPKG

SEQ ID NO: 374 - protein, 21 aa, Artificial Sequence
  Description of Artificial Sequence: Synthetic peptide
  MOD_RES (2)..(2): Hydroxyproline
  MOD_RES (4)..(4): Chloroproline
  MOD_RES (5)..(5): Hydroxyproline
  MOD_RES (7)..(7): Chloroproline
  MOD_RES (8)..(8): Hydroxyproline
  MOD_RES (10)..(10): Chloroproline
  MOD_RES (11)..(11): Hydroxyproline
  MOD_RES (13)..(13): Chloroproline
  MOD_RES (14)..(14): Hydroxyproline
  MOD_RES (16)..(16): Chloroproline
  MOD_RES (17)..(17): Hydroxyproline
  MOD_RES (19)..(19): Chloroproline
  MOD_RES (20)..(20): Hydroxyproline
KPGPPGPPGPPGPPGPPGPPG

SEQ ID NO: 375 - protein, 21 aa, Artificial Sequence
  Description of Artificial Sequence: Synthetic peptide
  MOD_RES (1)..(1): Chloroproline
  MOD_RES (4)..(4): Chloroproline
  MOD_RES (5)..(5): Hydroxyproline
  MOD_RES (7)..(7): Chloroproline
  MOD_RES (8)..(8): Hydroxyproline
  MOD_RES (10)..(10): Chloroproline
  MOD_RES (11)..(11): Hydroxyproline
  MOD_RES (13)..(13): Chloroproline
  MOD_RES (14)..(14): Hydroxyproline
  MOD_RES (16)..(16): Chloroproline
  MOD_RES (17)..(17): Hydroxyproline
  MOD_RES (19)..(19): Chloroproline
  MOD_RES (20)..(20): Hydroxyproline
PKGPPGPPGPPGPPGPPGPPG

SEQ ID NO: 376 - protein, 21 aa, Artificial Sequence
  Description of Artificial Sequence: Synthetic peptide
  MOD_RES (1)..(1): Chloroproline
  MOD_RES (2)..(2): Hydroxyproline
  MOD_RES (5)..(5): Hydroxyproline
  MOD_RES (7)..(7): Chloroproline
  MOD_RES (8)..(8): Hydroxyproline
  MOD_RES (10)..(10): Chloroproline
  MOD_RES (11)..(11): Hydroxyproline
  MOD_RES (13)..(13): Chloroproline
  MOD_RES (14)..(14): Hydroxyproline
  MOD_RES (16)..(16): Chloroproline
  MOD_RES (17)..(17): Hydroxyproline
  MOD_RES (19)..(19): Chloroproline
  MOD_RES (20)..(20): Hydroxyproline
PPGKPGPPGPPGPPGPPGPPG

SEQ ID NO: 377 - protein, 21 aa, Artificial Sequence
  Description of Artificial Sequence: Synthetic peptide
  MOD_RES (1)..(1): Chloroproline
  MOD_RES (2)..(2): Hydroxyproline
  MOD_RES (4)..(4): Chloroproline
  MOD_RES (7)..(7): Chloroproline
  MOD_RES (8)..(8): Hydroxyproline
  MOD_RES (10)..(10): Chloroproline
  MOD_RES (11)..(11): Hydroxyproline
  MOD_RES (13)..(13): Chloroproline
  MOD_RES (14)..(14): Hydroxyproline
  MOD_RES (16)..(16): Chloroproline
  MOD_RES (17)..(17): Hydroxyproline
  MOD_RES (19)..(19): Chloroproline
  MOD_RES (20)..(20): Hydroxyproline
PPGPKGPPGPPGPPGPPGPPG

SEQ ID NO: 378 - protein, 21 aa, Artificial Sequence
  Description of Artificial Sequence: Synthetic peptide
  MOD_RES (1)..(1): Chloroproline
  MOD_RES (2)..(2): Hydroxyproline
  MOD_RES (4)..(4): Chloroproline
  MOD_RES (5)..(5): Hydroxyproline
  MOD_RES (8)..(8): Hydroxyproline
  MOD_RES (10)..(10): Chloroproline
  MOD_RES (11)..(11): Hydroxyproline
  MOD_RES (13)..(13): Chloroproline
  MOD_RES (14)..(14): Hydroxyproline
  MOD_RES (16)..(16): Chloroproline
  MOD_RES (17)..(17): Hydroxyproline
  MOD_RES (19)..(19): Chloroproline
  MOD_RES (20)..(20): Hydroxyproline
PPGPPGKPGPPGPPGPPGPPG

SEQ ID NO: 379 - protein, 21 aa, Artificial Sequence
  Description of Artificial Sequence: Synthetic peptide
  MOD_RES (1)..(1): Chloroproline
  MOD_RES (2)..(2): Hydroxyproline
  MOD_RES (4)..(4): Chloroproline
  MOD_RES (5)..(5): Hydroxyproline
  MOD_RES (7)..(7): Chloroproline
  MOD_RES (10)..(10): Chloroproline
  MOD_RES (11)..(11): Hydroxyproline
  MOD_RES (13)..(13): Chloroproline
  MOD_RES (14)..(14): Hydroxyproline
  MOD_RES (16)..(16): Chloroproline
  MOD_RES (17)..(17): Hydroxyproline
  MOD_RES (19)..(19): Chloroproline
  MOD_RES (20)..(20): Hydroxyproline
PPGPPGPKGPPGPPGPPGPPG

SEQ ID NO: 380 - protein, 21 aa, Artificial Sequence
  Description of Artificial Sequence: Synthetic peptide
  MOD_RES (1)..(1): Chloroproline
  MOD_RES (2)..(2): Hydroxyproline
  MOD_RES (4)..(4): Chloroproline
  MOD_RES (5)..(5): Hydroxyproline
  MOD_RES (7)..(7): Chloroproline
  MOD_RES (8)..(8): Hydroxyproline
  MOD_RES (11)..(11): Hydroxyproline
  MOD_RES (13)..(13): Chloroproline
  MOD_RES (14)..(14): Hydroxyproline
  MOD_RES (16)..(16): Chloroproline
  MOD_RES (17)..(17): Hydroxyproline
  MOD_RES (19)..(19): Chloroproline
  MOD_RES (20)..(20): Hydroxyproline
PPGPPGPPGKPGPPGPPGPPG

SEQ ID NO: 381 - protein, 21 aa, Artificial Sequence
  Description of Artificial Sequence: Synthetic peptide
  MOD_RES (1)..(1): Chloroproline
  MOD_RES (2)..(2): Hydroxyproline
  MOD_RES (4)..(4): Chloroproline
  MOD_RES (5)..(5): Hydroxyproline
  MOD_RES (7)..(7): Chloroproline
  MOD_RES (8)..(8): Hydroxyproline
  MOD_RES (10)..(10): Chloroproline
  MOD_RES (13)..(13): Chloroproline
  MOD_RES (14)..(14): Hydroxyproline
  MOD_RES (16)..(16): Chloroproline
  MOD_RES (17)..(17): Hydroxyproline
  MOD_RES (19)..(19): Chloroproline
  MOD_RES (20)..(20): Hydroxyproline
PPGPPGPPGPKGPPGPPGPPG

SEQ ID NO: 382 - protein, 21 aa, Artificial Sequence
  Description of Artificial Sequence: Synthetic peptide
  MOD_RES (1)..(1): Chloroproline
  MOD_RES (2)..(2): Hydroxyproline
  MOD_RES (4)..(4): Chloroproline
  MOD_RES (5)..(5): Hydroxyproline
  MOD_RES (7)..(7): Chloroproline
  MOD_RES (8)..(8): Hydroxyproline
  MOD_RES (10)..(10): Chloroproline
  MOD_RES (11)..(11): Hydroxyproline
  MOD_RES (14)..(14): Hydroxyproline
  MOD_RES (16)..(16): Chloroproline
  MOD_RES (17)..(17): Hydroxyproline
  MOD_RES (19)..(19): Chloroproline
  MOD_RES (20)..(20): Hydroxyproline
PPGPPGPPGPPGKPGPPGPPG

SEQ ID NO: 383 - protein, 21 aa, Artificial Sequence
  Description of Artificial Sequence: Synthetic peptide
  MOD_RES (1)..(1): Chloroproline
  MOD_RES (2)..(2): Hydroxyproline
  MOD_RES (4)..(4): Chloroproline
  MOD_RES (5)..(5): Hydroxyproline
  MOD_RES (7)..(7): Chloroproline
  MOD_RES (8)..(8): Hydroxyproline
  MOD_RES (10)..(10): Chloroproline
  MOD_RES (11)..(11): Hydroxyproline
  MOD_RES (13)..(13): Chloroproline
  MOD_RES (16)..(16): Chloroproline
  MOD_RES (17)..(17): Hydroxyproline
  MOD_RES (19)..(19): Chloroproline
  MOD_RES (20)..(20): Hydroxyproline
PPGPPGPPGPPGPKGPPGPPG

SEQ ID NO: 384 - protein, 21 aa, Artificial Sequence
  Description of Artificial Sequence: Synthetic peptide
  MOD_RES (1)..(1): Chloroproline
  MOD_RES (2)..(2): Hydroxyproline
  MOD_RES (4)..(4): Chloroproline
  MOD_RES (5)..(5): Hydroxyproline
  MOD_RES (7)..(7): Chloroproline
  MOD_RES (8)..(8): Hydroxyproline
  MOD_RES (10)..(10): Chloroproline
  MOD_RES (11)..(11): Hydroxyproline
  MOD_RES (13)..(13): Chloroproline
  MOD_RES (14)..(14): Hydroxyproline
  MOD_RES (17)..(17): Hydroxyproline
  MOD_RES (19)..(19): Chloroproline
  MOD_RES (20)..(20): Hydroxyproline
PPGPPGPPGPPGPPGKPGPPG

SEQ ID NO: 385 - protein, 21 aa, Artificial Sequence
  Description of Artificial Sequence: Synthetic peptide
  MOD_RES (1)..(1): Chloroproline
  MOD_RES (2)..(2): Hydroxyproline
  MOD_RES (4)..(4): Chloroproline
  MOD_RES (5)..(5): Hydroxyproline
  MOD_RES (7)..(7): Chloroproline
  MOD_RES (8)..(8): Hydroxyproline
  MOD_RES (10)..(10): Chloroproline
  MOD_RES (11)..(11): Hydroxyproline
  MOD_RES (13)..(13): Chloroproline
  MOD_RES (14)..(14): Hydroxyproline
  MOD_RES (16)..(16): Chloroproline
  MOD_RES (19)..(19): Chloroproline
  MOD_RES (20)..(20): Hydroxyproline
PPGPPGPPGPPGPPGPKGPPG

SEQ ID NO: 386 - protein, 21 aa, Artificial Sequence
  Description of Artificial Sequence: Synthetic peptide
  MOD_RES (1)..(1): Chloroproline
  MOD_RES (2)..(2): Hydroxyproline
  MOD_RES (4)..(4): Chloroproline
  MOD_RES (5)..(5): Hydroxyproline
  MOD_RES (7)..(7): Chloroproline
  MOD_RES (8)..(8): Hydroxyproline
  MOD_RES (10)..(10): Chloroproline
  MOD_RES (11)..(11): Hydroxyproline
  MOD_RES (13)..(13): Chloroproline
  MOD_RES (14)..(14): Hydroxyproline
  MOD_RES (16)..(16): Chloroproline
  MOD_RES (17)..(17): Hydroxyproline
  MOD_RES (20)..(20): Hydroxyproline
PPGPPGPPGPPGPPGPPGKPG

SEQ ID NO: 387 - protein, 21 aa, Artificial Sequence
  Description of Artificial Sequence: Synthetic peptide
  MOD_RES (1)..(1): Chloroproline
  MOD_RES (2)..(2): Hydroxyproline
  MOD_RES (4)..(4): Chloroproline
  MOD_RES (5)..(5): Hydroxyproline
  MOD_RES (7)..(7): Chloroproline
  MOD_RES (8)..(8): Hydroxyproline
  MOD_RES (10)..(10): Chloroproline
  MOD_RES (11)..(11): Hydroxyproline
  MOD_RES (13)..(13): Chloroproline
  MOD_RES (14)..(14): Hydroxyproline
  MOD_RES (16)..(16): Chloroproline
  MOD_RES (17)..(17): Hydroxyproline
  MOD_RES (19)..(19): Chloroproline
PPGPPGPPGPPGPPGPPGPKG

SEQ ID NO: 388 - protein, 11 aa, Artificial Sequence
  Description of Artificial Sequence: Synthetic peptide
RPKPQQFFGLM

SEQ ID NO: 389 - protein, 32 aa, Artificial Sequence
  Description of Artificial Sequence: Synthetic polypeptide
PPGPPGPPGPPGPPGPPGPPGRPKPQQFFGLM

SEQ ID NO: 390 - protein, 32 aa, Artificial Sequence; identical to SEQ ID NO: 389
  Description of Artificial Sequence: Synthetic polypeptide
  MOD_RES (1)..(1): Hydroxyproline
  MOD_RES (4)..(4): Hydroxyproline
  MOD_RES (7)..(7): Hydroxyproline
  MOD_RES (10)..(10): Hydroxyproline
  MOD_RES (13)..(13): Hydroxyproline
  MOD_RES (16)..(16): Hydroxyproline
  MOD_RES (19)..(19): Hydroxyproline

SEQ ID NO: 391 - protein, 32 aa, Artificial Sequence; identical to SEQ ID NO: 389
  Description of Artificial Sequence: Synthetic polypeptide
  MOD_RES (2)..(2): Hydroxyproline
  MOD_RES (5)..(5): Hydroxyproline
  MOD_RES (8)..(8): Hydroxyproline
  MOD_RES (11)..(11): Hydroxyproline
  MOD_RES (14)..(14): Hydroxyproline
  MOD_RES (17)..(17): Hydroxyproline
  MOD_RES (20)..(20): Hydroxyproline

SEQ ID NO: 392 - protein, 32 aa, Artificial Sequence; identical to SEQ ID NO: 389
  Description of Artificial Sequence: Synthetic polypeptide
  MOD_RES (1)..(1): Fluoroproline
  MOD_RES (2)..(2): Hydroxyproline
  MOD_RES (4)..(4): Fluoroproline
  MOD_RES (5)..(5): Hydroxyproline
  MOD_RES (7)..(7): Fluoroproline
  MOD_RES (8)..(8): Hydroxyproline
  MOD_RES (10)..(10): Fluoroproline
  MOD_RES (11)..(11): Hydroxyproline
  MOD_RES (13)..(13): Fluoroproline
  MOD_RES (14)..(14): Hydroxyproline
  MOD_RES (16)..(16): Fluoroproline
  MOD_RES (17)..(17): Hydroxyproline
  MOD_RES (19)..(19): Fluoroproline
  MOD_RES (20)..(20): Hydroxyproline

SEQ ID NO: 393 - protein, 32 aa, Artificial Sequence; identical to SEQ ID NO: 389
  Description of Artificial Sequence: Synthetic polypeptide
  MOD_RES (1)..(1): Chloroproline
  MOD_RES (2)..(2): Hydroxyproline
  MOD_RES (4)..(4): Chloroproline
  MOD_RES (5)..(5): Hydroxyproline
  MOD_RES (7)..(7): Chloroproline
  MOD_RES (8)..(8): Hydroxyproline
  MOD_RES (10)..(10): Chloroproline
  MOD_RES (11)..(11): Hydroxyproline
  MOD_RES (13)..(13): Chloroproline
  MOD_RES (14)..(14): Hydroxyproline
  MOD_RES (16)..(16): Chloroproline
  MOD_RES (17)..(17): Hydroxyproline
  MOD_RES (19)..(19): Chloroproline
  MOD_RES (20)..(20): Hydroxyproline

SEQ ID NO: 394 - protein, 32 aa, Artificial Sequence; identical to SEQ ID NO: 389
  Description of Artificial Sequence: Synthetic polypeptide
  MOD_RES (2)..(2): Fluoroproline
  MOD_RES (5)..(5): Fluoroproline
  MOD_RES (8)..(8): Fluoroproline
  MOD_RES (11)..(11): Fluoroproline
  MOD_RES (14)..(14): Fluoroproline
  MOD_RES (17)..(17): Fluoroproline
  MOD_RES (20)..(20): Fluoroproline

SEQ ID NO: 395 - protein, 32 aa, Artificial Sequence; identical to SEQ ID NO: 389
  Description of Artificial Sequence: Synthetic polypeptide
  MOD_RES (2)..(2): Chloroproline
  MOD_RES (5)..(5): Chloroproline
  MOD_RES (8)..(8): Chloroproline
  MOD_RES (11)..(11): Chloroproline
  MOD_RES (14)..(14): Chloroproline
  MOD_RES (17)..(17): Chloroproline
  MOD_RES (20)..(20): Chloroproline

SEQ ID NO: 396 - protein, 30 aa, Artificial Sequence
  Description of Artificial Sequence: Synthetic polypeptide
  MOD_RES (2)..(2): Hydroxyproline
  MOD_RES (5)..(5): Hydroxyproline
  MOD_RES (8)..(8): Hydroxyproline
  MOD_RES (11)..(11): Hydroxyproline
  MOD_RES (14)..(14): Hydroxyproline
  MOD_RES (17)..(17): Hydroxyproline
  MOD_RES (20)..(20): Hydroxyproline
  MOD_RES (23)..(23): Hydroxyproline
  MOD_RES (26)..(26): Hydroxyproline
  MOD_RES (29)..(29): Hydroxyproline
PPGPPGPPGPPGPPGPPGPPGPPGPPGPPG

SEQ ID NO: 397 - protein, 30 aa, Artificial Sequence; identical to SEQ ID NO: 396
  Description of Artificial Sequence: Synthetic polypeptide

SEQ ID NO: 398 - protein, 60 aa, Artificial Sequence
  Description of Artificial Sequence: Synthetic polypeptide
  MOD_RES (1)..(1): Pro, 4S-hydroxyproline, fluoroproline, chloroproline, Lys, Cys or Met
  MOD_RES (2)..(2): Pro, 4R-hydroxyproline, fluoroproline, chloroproline, Lys, Cys or Met
  MOD_RES (4)..(4): Pro, 4S-hydroxyproline, fluoroproline, chloroproline, Lys, Cys or Met
  MOD_RES (5)..(5): Pro, 4R-hydroxyproline, fluoroproline, chloroproline, Lys, Cys or Met
  MOD_RES (7)..(7): Pro, 4S-hydroxyproline, fluoroproline, chloroproline, Lys, Cys or Met
  MOD_RES (8)..(8): Pro, 4R-hydroxyproline, fluoroproline, chloroproline, Lys, Cys or Met
  MOD_RES (10)..(10): Pro, 4S-hydroxyproline, fluoroproline, chloroproline, Lys, Cys or Met
  MOD_RES (11)..(11): Pro, 4R-hydroxyproline, fluoroproline, chloroproline, Lys, Cys or Met
  MOD_RES (13)..(13): Pro, 4S-hydroxyproline, fluoroproline, chloroproline, Lys, Cys or Met
  MOD_RES (14)..(14): Pro, 4R-hydroxyproline, fluoroproline, chloroproline, Lys, Cys or Met
  MOD_RES (16)..(16): Pro, 4S-hydroxyproline, fluoroproline, chloroproline, Lys, Cys or Met
  MOD_RES (17)..(17): Pro, 4R-hydroxyproline, fluoroproline, chloroproline, Lys, Cys or Met
  MOD_RES (19)..(19): Pro, 4S-hydroxyproline, fluoroproline, chloroproline, Lys, Cys or Met
  MOD_RES (20)..(20): Pro, 4R-hydroxyproline, fluoroproline, chloroproline, Lys, Cys or Met
  MOD_RES (22)..(22): Pro, 4S-hydroxyproline, fluoroproline, chloroproline, Lys, Cys or Met
  MOD_RES (23)..(23): Pro, 4R-hydroxyproline, fluoroproline, chloroproline, Lys, Cys or Met
  MOD_RES (25)..(25): Pro, 4S-hydroxyproline, fluoroproline, chloroproline, Lys, Cys or Met
  MOD_RES (26)..(26): Pro, 4R-hydroxyproline, fluoroproline, chloroproline, Lys, Cys or Met
  MOD_RES (28)..(28): Pro, 4S-hydroxyproline, fluoroproline, chloroproline, Lys, Cys or Met
  MOD_RES (29)..(29): Pro, 4R-hydroxyproline, fluoroproline, chloroproline, Lys, Cys or Met
  MOD_RES (31)..(31): Pro, 4S-hydroxyproline, fluoroproline, chloroproline, Lys, Cys or Met
  MOD_RES (32)..(32): Pro, 4R-hydroxyproline, fluoroproline, chloroproline, Lys, Cys or Met
  MOD_RES (34)..(34): Pro, 4S-hydroxyproline, fluoroproline, chloroproline, Lys, Cys or Met
  MOD_RES (35)..(35): Pro, 4R-hydroxyproline, fluoroproline, chloroproline, Lys, Cys or Met
  MOD_RES (37)..(37): Pro, 4S-hydroxyproline, fluoroproline, chloroproline, Lys, Cys or Met
  MOD_RES (38)..(38): Pro, 4R-hydroxyproline, fluoroproline, chloroproline, Lys, Cys or Met
  MOD_RES (40)..(40): Pro, 4S-hydroxyproline, fluoroproline, chloroproline, Lys, Cys or Met
  MOD_RES (41)..(41): Pro, 4R-hydroxyproline, fluoroproline, chloroproline, Lys, Cys or Met
  MOD_RES (43)..(43): Pro, 4S-hydroxyproline, fluoroproline, chloroproline, Lys, Cys or Met
  MOD_RES (44)..(44): Pro, 4R-hydroxyproline, fluoroproline, chloroproline, Lys, Cys or Met
  MOD_RES (46)..(46): Pro, 4S-hydroxyproline, fluoroproline, chloroproline, Lys, Cys or Met
  MOD_RES (47)..(47): Pro, 4R-hydroxyproline, fluoroproline, chloroproline, Lys, Cys or Met
  MOD_RES (49)..(49): Pro, 4S-hydroxyproline, fluoroproline, chloroproline, Lys, Cys or Met
  MOD_RES (50)..(50): Pro, 4R-hydroxyproline, fluoroproline, chloroproline, Lys, Cys or Met
  MOD_RES (52)..(52): Pro, 4S-hydroxyproline, fluoroproline, chloroproline, Lys, Cys or Met
  MOD_RES (53)..(53): Pro, 4R-hydroxyproline, fluoroproline, chloroproline, Lys, Cys or Met
  MOD_RES (55)..(55): Pro, 4S-hydroxyproline, fluoroproline, chloroproline, Lys, Cys or Met
  MOD_RES (56)..(56): Pro, 4R-hydroxyproline, fluoroproline, chloroproline, Lys, Cys or Met
  MOD_RES (58)..(58): Pro, 4S-hydroxyproline, fluoroproline, chloroproline, Lys, Cys or Met
  MOD_RES (59)..(59): Pro, 4R-hydroxyproline, fluoroproline, chloroproline, Lys, Cys or Met
  MISC_FEATURE (1)..(60): This sequence may encompass 1-20 "Xaa Xaa Gly" repeating units wherein Xaa is Pro, 4S-hydroxyproline, 4R-hydroxyproline, fluoroproline, chloroproline, Lys, Cys or Met
  See specification as filed for detailed description of substitutions and preferred embodiments
XXGXXGXXGXXGXXGXXGXXGXXGXXGXXGXXGXXGXXGXXGXXGXXGXXGXXGXXGXXG